European Patent Specification EP 3 536 780 B1, published May 14, 2025. Title: Proline hydroxylase and uses thereof. Applicant: ASYMCHEM LABORATORIES (TIANJIN) CO.,LTD ASYMCHEM LIFE SCIENCE (TIANJIN) CO.,LTD TIANJIN ASYMCHEM PHARMACEUTICAL CO.,LTD ASYMCHEM LABORATORIES (FUXIN) CO.,LTD JILIN ASYMCHEM LABORATORIES CO.,LTD. The sequence listing filed with the application follows.

SEQUENCE LISTING (292 sequences)

SEQ ID NO: 1 - DNA, 831 bp, Kordia jejudonensis
atggaatcaaaaataataggcaaagtaaattttgaagaacacttactggacaaagagctgaaattgatagatactttcgaattcaatgattcgtacagtgaatatgcatcaggaatttggaaaacatgcatgctttggaatcgctccggacagaaagatgatcatttatctatagaacatgatacgtatgtaaaaccgacagaatatggtaaacaacttgcatatgtcaatgaaattatagcaaatactttcaaaaaagagcatataaaaacggttcgactttttatgtgtattaacggattaattattccacataaagactatttagaatttaaaaaaggatttacacgaattcacattccgcttaaaattaacgaacatgcgcttacttccgaagaagatgttgtgtacaatatgcaaaaaggcgaaatatggtttatagaaggaagaaaaattcacagtgccgccaacttttcaaaagtaaagcggatcaatttagtgattgactttgctcctgatattccgtttgaagaattatttctaaactcggaaaattaccaaccaaatttgattccaaaaattagccaacgaacacagctaaaagaagaagaattaggctatataaaaggattatctaagatcattaatgaaatgaactttgacgatattttatcaatactctccaaaatacatttttatagaaatgtgtctagcgaactggttttcggttggttagatgaaattgcaactgcttctaacaattataacattcaacgaaaagcacaagaagtgaccgatttattaataagaaaaggaccaataaataattaa

SEQ ID NO: 2 - protein, 276 aa, Kordia jejudonensis
MESKIIGKVNFEEHLLDKELKLIDTFEFNDSYSEYASGIWKTCMLWNRSGQKDDHLSIEHDTYVKPTEYGKQLAYVNEIIANTFKKEHIKTVRLFMCINGLIIPHKDYLEFKKGFTRIHIPLKINEHALTSEEDVVYNMQKGEIWFIEGRKIHSAANFSKVKRINLVIDFAPDIPFEELFLNSENYQPNLIPKISQRTQLKEEELGYIKGLSKIINEMNFDDILSILSKIHFYRNVSSELVFGWLDEIATASNNYNIQRKAQEVTDLLIRKGPINN

SEQ ID NO: 3 - DNA, 831 bp, Artificial Sequence
  condon-optimizated DNA sequence
atggaatccaagatcatcggtaaagtcaacttcgaggagcatctgctggataaagagctgaaactgatcgacactttcgagttcaacgacagctacagcgaatacgcttctggtatttggaagacttgcatgctgtggaaccgttctggtcagaaagatgaccatctgtctattgaacatgatacctacgtgaaacctactgaatacggcaaacagctggcatacgtaaacgaaatcatcgctaacacctttaagaaagaacacatcaagacggtgcgtctgttcatgtgtatcaacggcctgatcatcccacacaaagactacctggaattcaagaaaggcttcacccgtatccacatcccgctgaaaatcaacgaacacgcactgacctctgaagaagatgttgtttacaacatgcagaaaggtgaaatttggttcatcgaaggccgtaaaatccacagcgctgccaatttcagcaaagtgaaacgtatcaacctggtcatcgacttcgcgccggatattccgtttgaagaactgttcctgaattctgagaactatcaaccgaacctgatcccgaaaatctctcaacgtacccagctgaaagaagaagagctgggttatatcaaaggtctgtctaaaattatcaatgaaatgaactttgacgacatcctgtccattctgagcaaaattcacttctatcgcaacgtttcctccgaactggtttttggctggctggacgaaattgccacggcgtccaacaactataacattcagcgcaaagcgcaggaagtaaccgatctgctgattcgcaaaggcccgattaataactaa

SEQ ID NO: 4 - protein, 276 aa, Artificial Sequence; identical to SEQ ID NO: 2
  condon-optimizated sequence drived from Kordia jejudonensis

SEQ ID NO: 5 - DNA, 831 bp, Artificial Sequence
  gene sequence of H14R mutant
atggaatccaagatcatcggtaaagtcaacttcgaggagcgtctgctggataaagagctgaaactgatcgacactttcgagttcaacgacagctacagcgaatacgcttctggtatttggaagacttgcatgctgtggaaccgttctggtcagaaagatgaccatctgtctattgaacatgatacctacgtgaaacctactgaatacggcaaacagctggcatacgtaaacgaaatcatcgctaacacctttaagaaagaacacatcaagacggtgcgtctgttcatgtgtatcaacggcctgatcatcccacacaaagactacctggaattcaagaaaggcttcacccgtatccacatcccgctgaaaatcaacgaacacgcactgacctctgaagaagatgttgtttacaacatgcagaaaggtgaaatttggttcatcgaaggccgtaaaatccacagcgctgccaatttcagcaaagtgaaacgtatcaacctggtcatcgacttcgcgccggatattccgtttgaagaactgttcctgaattctgagaactatcaaccgaacctgatcccgaaaatctctcaacgtacccagctgaaagaagaagagctgggttatatcaaaggtctgtctaaaattatcaatgaaatgaactttgacgacatcctgtccattctgagcaaaattcacttctatcgcaacgtttcctccgaactggtttttggctggctggacgaaattgccacggcgtccaacaactataacattcagcgcaaagcgcaggaagtaaccgatctgctgattcgcaaaggcccgattaataactaa

SEQ ID NO: 6 - protein, 276 aa, Artificial Sequence
  amino acid sequence of H14R mutant
MESKIIGKVNFEERLLDKELKLIDTFEFNDSYSEYASGIWKTCMLWNRSGQKDDHLSIEHDTYVKPTEYGKQLAYVNEIIANTFKKEHIKTVRLFMCINGLIIPHKDYLEFKKGFTRIHIPLKINEHALTSEEDVVYNMQKGEIWFIEGRKIHSAANFSKVKRINLVIDFAPDIPFEELFLNSENYQPNLIPKISQRTQLKEEELGYIKGLSKIINEMNFDDILSILSKIHFYRNVSSELVFGWLDEIATASNNYNIQRKAQEVTDLLIRKGPINN

SEQ ID NO: 7 - DNA, 831 bp, Artificial Sequence
  gene sequence of S16N mutant
atggaatccaagatcatcggtaaagtcaacttcgaggagcatctgaatgataaagagctgaaactgatcgacactttcgagttcaacgacagctacagcgaatacgcttctggtatttggaagacttgcatgctgtggaaccgttctggtcagaaagatgaccatctgtctattgaacatgatacctacgtgaaacctactgaatacggcaaacagctggcatacgtaaacgaaatcatcgctaacacctttaagaaagaacacatcaagacggtgcgtctgttcatgtgtatcaacggcctgatcatcccacacaaagactacctggaattcaagaaaggcttcacccgtatccacatcccgctgaaaatcaacgaacacgcactgacctctgaagaagatgttgtttacaacatgcagaaaggtgaaatttggttcatcgaaggccgtaaaatccacagcgctgccaatttcagcaaagtgaaacgtatcaacctggtcatcgacttcgcgccggatattccgtttgaagaactgttcctgaattctgagaactatcaaccgaacctgatcccgaaaatctctcaacgtacccagctgaaagaagaagagctgggttatatcaaaggtctgtctaaaattatcaatgaaatgaactttgacgacatcctgtccattctgagcaaaattcacttctatcgcaacgtttcctccgaactggtttttggctggctggacgaaattgccacggcgtccaacaactataacattcagcgcaaagcgcaggaagtaaccgatctgctgattcgcaaaggcccgattaataactaa

SEQ ID NO: 8 - protein, 276 aa, Artificial Sequence
  amino acid of S16N mutant
MESKIIGKVNFEEHLNDKELKLIDTFEFNDSYSEYASGIWKTCMLWNRSGQKDDHLSIEHDTYVKPTEYGKQLAYVNEIIANTFKKEHIKTVRLFMCINGLIIPHKDYLEFKKGFTRIHIPLKINEHALTSEEDVVYNMQKGEIWFIEGRKIHSAANFSKVKRINLVIDFAPDIPFEELFLNSENYQPNLIPKISQRTQLKEEELGYIKGLSKIINEMNFDDILSILSKIHFYRNVSSELVFGWLDEIATASNNYNIQRKAQEVTDLLIRKGPINN

SEQ ID NO: 9 - DNA, 831 bp, Artificial Sequence
  gene sequence of T25G mutant
atggaatccaagatcatcggtaaagtcaacttcgaggagcatctgctggataaagagctgaaactgatcgacggtttcgagttcaacgacagctacagcgaatacgcttctggtatttggaagacttgcatgctgtggaaccgttctggtcagaaagatgaccatctgtctattgaacatgatacctacgtgaaacctactgaatacggcaaacagctggcatacgtaaacgaaatcatcgctaacacctttaagaaagaacacatcaagacggtgcgtctgttcatgtgtatcaacggcctgatcatcccacacaaagactacctggaattcaagaaaggcttcacccgtatccacatcccgctgaaaatcaacgaacacgcactgacctctgaagaagatgttgtttacaacatgcagaaaggtgaaatttggttcatcgaaggccgtaaaatccacagcgctgccaatttcagcaaagtgaaacgtatcaacctggtcatcgacttcgcgccggatattccgtttgaagaactgttcctgaattctgagaactatcaaccgaacctgatcccgaaaatctctcaacgtacccagctgaaagaagaagagctgggttatatcaaaggtctgtctaaaattatcaatgaaatgaactttgacgacatcctgtccattctgagcaaaattcacttctatcgcaacgtttcctccgaactggtttttggctggctggacgaaattgccacggcgtccaacaactataacattcagcgcaaagcgcaggaagtaaccgatctgctgattcgcaaaggcccgattaataactaa

SEQ ID NO: 10 - protein, 276 aa, Artificial Sequence
  amino acid sequence of T25G mutant
MESKIIGKVNFEEHLLDKELKLIDGFEFNDSYSEYASGIWKTCMLWNRSGQKDDHLSIEHDTYVKPTEYGKQLAYVNEIIANTFKKEHIKTVRLFMCINGLIIPHKDYLEFKKGFTRIHIPLKINEHALTSEEDVVYNMQKGEIWFIEGRKIHSAANFSKVKRINLVIDFAPDIPFEELFLNSENYQPNLIPKISQRTQLKEEELGYIKGLSKIINEMNFDDILSILSKIHFYRNVSSELVFGWLDEIATASNNYNIQRKAQEVTDLLIRKGPINN

SEQ ID NO: 11 - DNA, 831 bp, Artificial Sequence
  gene sequence of T25R mutant
atggaatccaagatcatcggtaaagtcaacttcgaggagcatctgctggataaagagctgaaactgatcgaccgtttcgagttcaacgacagctacagcgaatacgcttctggtatttggaagacttgcatgctgtggaaccgttctggtcagaaagatgaccatctgtctattgaacatgatacctacgtgaaacctactgaatacggcaaacagctggcatacgtaaacgaaatcatcgctaacacctttaagaaagaacacatcaagacggtgcgtctgttcatgtgtatcaacggcctgatcatcccacacaaagactacctggaattcaagaaaggcttcacccgtatccacatcccgctgaaaatcaacgaacacgcactgacctctgaagaagatgttgtttacaacatgcagaaaggtgaaatttggttcatcgaaggccgtaaaatccacagcgctgccaatttcagcaaagtgaaacgtatcaacctggtcatcgacttcgcgccggatattccgtttgaagaactgttcctgaattctgagaactatcaaccgaacctgatcccgaaaatctctcaacgtacccagctgaaagaagaagagctgggttatatcaaaggtctgtctaaaattatcaatgaaatgaactttgacgacatcctgtccattctgagcaaaattcacttctatcgcaacgtttcctccgaactggtttttggctggctggacgaaattgccacggcgtccaacaactataacattcagcgcaaagcgcaggaagtaaccgatctgctgattcgcaaaggcccgattaataactaa

SEQ ID NO: 12 - protein, 276 aa, Artificial Sequence
  amino acid sequence of T25R mutant
MESKIIGKVNFEEHLLDKELKLIDRFEFNDSYSEYASGIWKTCMLWNRSGQKDDHLSIEHDTYVKPTEYGKQLAYVNEIIANTFKKEHIKTVRLFMCINGLIIPHKDYLEFKKGFTRIHIPLKINEHALTSEEDVVYNMQKGEIWFIEGRKIHSAANFSKVKRINLVIDFAPDIPFEELFLNSENYQPNLIPKISQRTQLKEEELGYIKGLSKIINEMNFDDILSILSKIHFYRNVSSELVFGWLDEIATASNNYNIQRKAQEVTDLLIRKGPINN

SEQ ID NO: 13 - DNA, 831 bp, Artificial Sequence
  genge sequence of F26L mutant
atggaatccaagatcatcggtaaagtcaacttcgaggagcatctgctggataaagagctgaaactgatcgacactctggagttcaacgacagctacagcgaatacgcttctggtatttggaagacttgcatgctgtggaaccgttctggtcagaaagatgaccatctgtctattgaacatgatacctacgtgaaacctactgaatacggcaaacagctggcatacgtaaacgaaatcatcgctaacacctttaagaaagaacacatcaagacggtgcgtctgttcatgtgtatcaacggcctgatcatcccacacaaagactacctggaattcaagaaaggcttcacccgtatccacatcccgctgaaaatcaacgaacacgcactgacctctgaagaagatgttgtttacaacatgcagaaaggtgaaatttggttcatcgaaggccgtaaaatccacagcgctgccaatttcagcaaagtgaaacgtatcaacctggtcatcgacttcgcgccggatattccgtttgaagaactgttcctgaattctgagaactatcaaccgaacctgatcccgaaaatctctcaacgtacccagctgaaagaagaagagctgggttatatcaaaggtctgtctaaaattatcaatgaaatgaactttgacgacatcctgtccattctgagcaaaattcacttctatcgcaacgtttcctccgaactggtttttggctggctggacgaaattgccacggcgtccaacaactataacattcagcgcaaagcgcaggaagtaaccgatctgctgattcgcaaaggcccgattaataactaa

SEQ ID NO: 14 - protein, 276 aa, Artificial Sequence
  amino acid sequence of F26L mutant
MESKIIGKVNFEEHLLDKELKLIDTLEFNDSYSEYASGIWKTCMLWNRSGQKDDHLSIEHDTYVKPTEYGKQLAYVNEIIANTFKKEHIKTVRLFMCINGLIIPHKDYLEFKKGFTRIHIPLKINEHALTSEEDVVYNMQKGEIWFIEGRKIHSAANFSKVKRINLVIDFAPDIPFEELFLNSENYQPNLIPKISQRTQLKEEELGYIKGLSKIINEMNFDDILSILSKIHFYRNVSSELVFGWLDEIATASNNYNIQRKAQEVTDLLIRKGPINN

SEQ ID NO: 15 - DNA, 831 bp, Artificial Sequence
  gene sequence of E27K mutant
atggaatccaagatcatcggtaaagtcaacttcgaggagcatctgctggataaagagctgaaactgatcgacactttcaaattcaacgacagctacagcgaatacgcttctggtatttggaagacttgcatgctgtggaaccgttctggtcagaaagatgaccatctgtctattgaacatgatacctacgtgaaacctactgaatacggcaaacagctggcatacgtaaacgaaatcatcgctaacacctttaagaaagaacacatcaagacggtgcgtctgttcatgtgtatcaacggcctgatcatcccacacaaagactacctggaattcaagaaaggcttcacccgtatccacatcccgctgaaaatcaacgaacacgcactgacctctgaagaagatgttgtttacaacatgcagaaaggtgaaatttggttcatcgaaggccgtaaaatccacagcgctgccaatttcagcaaagtgaaacgtatcaacctggtcatcgacttcgcgccggatattccgtttgaagaactgttcctgaattctgagaactatcaaccgaacctgatcccgaaaatctctcaacgtacccagctgaaagaagaagagctgggttatatcaaaggtctgtctaaaattatcaatgaaatgaactttgacgacatcctgtccattctgagcaaaattcacttctatcgcaacgtttcctccgaactggtttttggctggctggacgaaattgccacggcgtccaacaactataacattcagcgcaaagcgcaggaagtaaccgatctgctgattcgcaaaggcccgattaataactaa

SEQ ID NO: 16 - protein, 276 aa, Artificial Sequence
  amino acid sequence of E27K mutant
MESKIIGKVNFEEHLLDKELKLIDTFKFNDSYSEYASGIWKTCMLWNRSGQKDDHLSIEHDTYVKPTEYGKQLAYVNEIIANTFKKEHIKTVRLFMCINGLIIPHKDYLEFKKGFTRIHIPLKINEHALTSEEDVVYNMQKGEIWFIEGRKIHSAANFSKVKRINLVIDFAPDIPFEELFLNSENYQPNLIPKISQRTQLKEEELGYIKGLSKIINEMNFDDILSILSKIHFYRNVSSELVFGWLDEIATASNNYNIQRKAQEVTDLLIRKGPINN

SEQ ID NO: 17 - DNA, 831 bp, Artificial Sequence
  gene sequence of D30S mutant
atggaatccaagatcatcggtaaagtcaacttcgaggagcatctgctggataaagagctgaaactgatcgacactttcgagttcaacagcagctacagcgaatacgcttctggtatttggaagacttgcatgctgtggaaccgttctggtcagaaagatgaccatctgtctattgaacatgatacctacgtgaaacctactgaatacggcaaacagctggcatacgtaaacgaaatcatcgctaacacctttaagaaagaacacatcaagacggtgcgtctgttcatgtgtatcaacggcctgatcatcccacacaaagactacctggaattcaagaaaggcttcacccgtatccacatcccgctgaaaatcaacgaacacgcactgacctctgaagaagatgttgtttacaacatgcagaaaggtgaaatttggttcatcgaaggccgtaaaatccacagcgctgccaatttcagcaaagtgaaacgtatcaacctggtcatcgacttcgcgccggatattccgtttgaagaactgttcctgaattctgagaactatcaaccgaacctgatcccgaaaatctctcaacgtacccagctgaaagaagaagagctgggttatatcaaaggtctgtctaaaattatcaatgaaatgaactttgacgacatcctgtccattctgagcaaaattcacttctatcgcaacgtttcctccgaactggtttttggctggctggacgaaattgccacggcgtccaacaactataacattcagcgcaaagcgcaggaagtaaccgatctgctgattcgcaaaggcccgattaataactaa

SEQ ID NO: 18 - protein, 276 aa, Artificial Sequence
  amino acid sequence of D30S mutant
MESKIIGKVNFEEHLLDKELKLIDTFEFNSSYSEYASGIWKTCMLWNRSGQKDDHLSIEHDTYVKPTEYGKQLAYVNEIIANTFKKEHIKTVRLFMCINGLIIPHKDYLEFKKGFTRIHIPLKINEHALTSEEDVVYNMQKGEIWFIEGRKIHSAANFSKVKRINLVIDFAPDIPFEELFLNSENYQPNLIPKISQRTQLKEEELGYIKGLSKIINEMNFDDILSILSKIHFYRNVSSELVFGWLDEIATASNNYNIQRKAQEVTDLLIRKGPINN

SEQ ID NO: 19 - DNA, 831 bp, Artificial Sequence
  gene sequence of S33N mutant
atggaatccaagatcatcggtaaagtcaacttcgaggagcatctgctggataaagagctgaaactgatcgacactttcgagttcaacgacagctacaatgaatacgcttctggtatttggaagacttgcatgctgtggaaccgttctggtcagaaagatgaccatctgtctattgaacatgatacctacgtgaaacctactgaatacggcaaacagctggcatacgtaaacgaaatcatcgctaacacctttaagaaagaacacatcaagacggtgcgtctgttcatgtgtatcaacggcctgatcatcccacacaaagactacctggaattcaagaaaggcttcacccgtatccacatcccgctgaaaatcaacgaacacgcactgacctctgaagaagatgttgtttacaacatgcagaaaggtgaaatttggttcatcgaaggccgtaaaatccacagcgctgccaatttcagcaaagtgaaacgtatcaacctggtcatcgacttcgcgccggatattccgtttgaagaactgttcctgaattctgagaactatcaaccgaacctgatcccgaaaatctctcaacgtacccagctgaaagaagaagagctgggttatatcaaaggtctgtctaaaattatcaatgaaatgaactttgacgacatcctgtccattctgagcaaaattcacttctatcgcaacgtttcctccgaactggtttttggctggctggacgaaattgccacggcgtccaacaactataacattcagcgcaaagcgcaggaagtaaccgatctgctgattcgcaaaggcccgattaataactaa

SEQ ID NO: 20 - protein, 276 aa, Artificial Sequence
  amino acid sequence of S33N mutant
MESKIIGKVNFEEHLLDKELKLIDTFEFNDSYNEYASGIWKTCMLWNRSGQKDDHLSIEHDTYVKPTEYGKQLAYVNEIIANTFKKEHIKTVRLFMCINGLIIPHKDYLEFKKGFTRIHIPLKINEHALTSEEDVVYNMQKGEIWFIEGRKIHSAANFSKVKRINLVIDFAPDIPFEELFLNSENYQPNLIPKISQRTQLKEEELGYIKGLSKIINEMNFDDILSILSKIHFYRNVSSELVFGWLDEIATASNNYNIQRKAQEVTDLLIRKGPINN

SEQ ID NO: 21 - DNA, 831 bp, Artificial Sequence
  gene sequence of E34N mutant
atggaatccaagatcatcggtaaagtcaacttcgaggagcatctgctggataaagagctgaaactgatcgacactttcgagttcaacgacagctacagcaattacgcttctggtatttggaagacttgcatgctgtggaaccgttctggtcagaaagatgaccatctgtctattgaacatgatacctacgtgaaacctactgaatacggcaaacagctggcatacgtaaacgaaatcatcgctaacacctttaagaaagaacacatcaagacggtgcgtctgttcatgtgtatcaacggcctgatcatcccacacaaagactacctggaattcaagaaaggcttcacccgtatccacatcccgctgaaaatcaacgaacacgcactgacctctgaagaagatgttgtttacaacatgcagaaaggtgaaatttggttcatcgaaggccgtaaaatccacagcgctgccaatttcagcaaagtgaaacgtatcaacctggtcatcgacttcgcgccggatattccgtttgaagaactgttcctgaattctgagaactatcaaccgaacctgatcccgaaaatctctcaacgtacccagctgaaagaagaagagctgggttatatcaaaggtctgtctaaaattatcaatgaaatgaactttgacgacatcctgtccattctgagcaaaattcacttctatcgcaacgtttcctccgaactggtttttggctggctggacgaaattgccacggcgtccaacaactataacattcagcgcaaagcgcaggaagtaaccgatctgctgattcgcaaaggcccgattaataactaa

SEQ ID NO: 22 - protein, 276 aa, Artificial Sequence
  amino acid sequence of E34N mutant
MESKIIGKVNFEEHLLDKELKLIDTFEFNDSYSNYASGIWKTCMLWNRSGQKDDHLSIEHDTYVKPTEYGKQLAYVNEIIANTFKKEHIKTVRLFMCINGLIIPHKDYLEFKKGFTRIHIPLKINEHALTSEEDVVYNMQKGEIWFIEGRKIHSAANFSKVKRINLVIDFAPDIPFEELFLNSENYQPNLIPKISQRTQLKEEELGYIKGLSKIINEMNFDDILSILSKIHFYRNVSSELVFGWLDEIATASNNYNIQRKAQEVTDLLIRKGPINN

SEQ ID NO: 23 - DNA, 831 bp, Artificial Sequence
  gene sequence of E34G mutant
atggaatccaagatcatcggtaaagtcaacttcgaggagcatctgctggataaagagctgaaactgatcgacactttcgagttcaacgacagctacagcggttacgcttctggtatttggaagacttgcatgctgtggaaccgttctggtcagaaagatgaccatctgtctattgaacatgatacctacgtgaaacctactgaatacggcaaacagctggcatacgtaaacgaaatcatcgctaacacctttaagaaagaacacatcaagacggtgcgtctgttcatgtgtatcaacggcctgatcatcccacacaaagactacctggaattcaagaaaggcttcacccgtatccacatcccgctgaaaatcaacgaacacgcactgacctctgaagaagatgttgtttacaacatgcagaaaggtgaaatttggttcatcgaaggccgtaaaatccacagcgctgccaatttcagcaaagtgaaacgtatcaacctggtcatcgacttcgcgccggatattccgtttgaagaactgttcctgaattctgagaactatcaaccgaacctgatcccgaaaatctctcaacgtacccagctgaaagaagaagagctgggttatatcaaaggtctgtctaaaattatcaatgaaatgaactttgacgacatcctgtccattctgagcaaaattcacttctatcgcaacgtttcctccgaactggtttttggctggctggacgaaattgccacggcgtccaacaactataacattcagcgcaaagcgcaggaagtaaccgatctgctgattcgcaaaggcccgattaataactaa

SEQ ID NO: 24 - protein, 276 aa, Artificial Sequence
  amino acid sequence of E34G mutant
MESKIIGKVNFEEHLLDKELKLIDTFEFNDSYSGYASGIWKTCMLWNRSGQKDDHLSIEHDTYVKPTEYGKQLAYVNEIIANTFKKEHIKTVRLFMCINGLIIPHKDYLEFKKGFTRIHIPLKINEHALTSEEDVVYNMQKGEIWFIEGRKIHSAANFSKVKRINLVIDFAPDIPFEELFLNSENYQPNLIPKISQRTQLKEEELGYIKGLSKIINEMNFDDILSILSKIHFYRNVSSELVFGWLDEIATASNNYNIQRKAQEVTDLLIRKGPINN

SEQ ID NO: 25 - DNA, 831 bp, Artificial Sequence
  gene sequence of E34L mutant
atggaatccaagatcatcggtaaagtcaacttcgaggagcatctgctggataaagagctgaaactgatcgacactttcgagttcaacgacagctacagcctgtacgcttctggtatttggaagacttgcatgctgtggaaccgttctggtcagaaagatgaccatctgtctattgaacatgatacctacgtgaaacctactgaatacggcaaacagctggcatacgtaaacgaaatcatcgctaacacctttaagaaagaacacatcaagacggtgcgtctgttcatgtgtatcaacggcctgatcatcccacacaaagactacctggaattcaagaaaggcttcacccgtatccacatcccgctgaaaatcaacgaacacgcactgacctctgaagaagatgttgtttacaacatgcagaaaggtgaaatttggttcatcgaaggccgtaaaatccacagcgctgccaatttcagcaaagtgaaacgtatcaacctggtcatcgacttcgcgccggatattccgtttgaagaactgttcctgaattctgagaactatcaaccgaacctgatcccgaaaatctctcaacgtacccagctgaaagaagaagagctgggttatatcaaaggtctgtctaaaattatcaatgaaatgaactttgacgacatcctgtccattctgagcaaaattcacttctatcgcaacgtttcctccgaactggtttttggctggctggacgaaattgccacggcgtccaacaactataacattcagcgcaaagcgcaggaagtaaccgatctgctgattcgcaaaggcccgattaataactaa

SEQ ID NO: 26 - protein, 276 aa, Artificial Sequence
  amino acid sequence of E34L mutant
MESKIIGKVNFEEHLLDKELKLIDTFEFNDSYSLYASGIWKTCMLWNRSGQKDDHLSIEHDTYVKPTEYGKQLAYVNEIIANTFKKEHIKTVRLFMCINGLIIPHKDYLEFKKGFTRIHIPLKINEHALTSEEDVVYNMQKGEIWFIEGRKIHSAANFSKVKRINLVIDFAPDIPFEELFLNSENYQPNLIPKISQRTQLKEEELGYIKGLSKIINEMNFDDILSILSKIHFYRNVSSELVFGWLDEIATASNNYNIQRKAQEVTDLLIRKGPINN

SEQ ID NO: 27 - DNA, 831 bp, Artificial Sequence
  gene sequence of E34D mutant
atggaatccaagatcatcggtaaagtcaacttcgaggagcatctgctggataaagagctgaaactgatcgacactttcgagttcaacgacagctacagcgattacgcttctggtatttggaagacttgcatgctgtggaaccgttctggtcagaaagatgaccatctgtctattgaacatgatacctacgtgaaacctactgaatacggcaaacagctggcatacgtaaacgaaatcatcgctaacacctttaagaaagaacacatcaagacggtgcgtctgttcatgtgtatcaacggcctgatcatcccacacaaagactacctggaattcaagaaaggcttcacccgtatccacatcccgctgaaaatcaacgaacacgcactgacctctgaagaagatgttgtttacaacatgcagaaaggtgaaatttggttcatcgaaggccgtaaaatccacagcgctgccaatttcagcaaagtgaaacgtatcaacctggtcatcgacttcgcgccggatattccgtttgaagaactgttcctgaattctgagaactatcaaccgaacctgatcccgaaaatctctcaacgtacccagctgaaagaagaagagctgggttatatcaaaggtctgtctaaaattatcaatgaaatgaactttgacgacatcctgtccattctgagcaaaattcacttctatcgcaacgtttcctccgaactggtttttggctggctggacgaaattgccacggcgtccaacaactataacattcagcgcaaagcgcaggaagtaaccgatctgctgattcgcaaaggcccgattaataactaa

SEQ ID NO: 28 - protein, 276 aa, Artificial Sequence
  amino acid sequence of E34D mutant
MESKIIGKVNFEEHLLDKELKLIDTFEFNDSYSDYASGIWKTCMLWNRSGQKDDHLSIEHDTYVKPTEYGKQLAYVNEIIANTFKKEHIKTVRLFMCINGLIIPHKDYLEFKKGFTRIHIPLKINEHALTSEEDVVYNMQKGEIWFIEGRKIHSAANFSKVKRINLVIDFAPDIPFEELFLNSENYQPNLIPKISQRTQLKEEELGYIKGLSKIINEMNFDDILSILSKIHFYRNVSSELVFGWLDEIATASNNYNIQRKAQEVTDLLIRKGPINN

SEQ ID NO: 29 - DNA, 831 bp, Artificial Sequence
  gene sequence of E34S mutant
atggaatccaagatcatcggtaaagtcaacttcgaggagcatctgctggataaagagctgaaactgatcgacactttcgagttcaacgacagctacagcagctacgcttctggtatttggaagacttgcatgctgtggaaccgttctggtcagaaagatgaccatctgtctattgaacatgatacctacgtgaaacctactgaatacggcaaacagctggcatacgtaaacgaaatcatcgctaacacctttaagaaagaacacatcaagacggtgcgtctgttcatgtgtatcaacggcctgatcatcccacacaaagactacctggaattcaagaaaggcttcacccgtatccacatcccgctgaaaatcaacgaacacgcactgacctctgaagaagatgttgtttacaacatgcagaaaggtgaaatttggttcatcgaaggccgtaaaatccacagcgctgccaatttcagcaaagtgaaacgtatcaacctggtcatcgacttcgcgccggatattccgtttgaagaactgttcctgaattctgagaactatcaaccgaacctgatcccgaaaatctctcaacgtacccagctgaaagaagaagagctgggttatatcaaaggtctgtctaaaattatcaatgaaatgaactttgacgacatcctgtccattctgagcaaaattcacttctatcgcaacgtttcctccgaactggtttttggctggctggacgaaattgccacggcgtccaacaactataacattcagcgcaaagcgcaggaagtaaccgatctgctgattcgcaaaggcccgattaataactaa

SEQ ID NO: 30 - protein, 276 aa, Artificial Sequence
  amino acid sequence of E34S mutant
MESKIIGKVNFEEHLLDKELKLIDTFEFNDSYSSYASGIWKTCMLWNRSGQKDDHLSIEHDTYVKPTEYGKQLAYVNEIIANTFKKEHIKTVRLFMCINGLIIPHKDYLEFKKGFTRIHIPLKINEHALTSEEDVVYNMQKGEIWFIEGRKIHSAANFSKVKRINLVIDFAPDIPFEELFLNSENYQPNLIPKISQRTQLKEEELGYIKGLSKIINEMNFDDILSILSKIHFYRNVSSELVFGWLDEIATASNNYNIQRKAQEVTDLLIRKGPINN

SEQ ID NO: 31 - DNA, 831 bp, Artificial Sequence
  gene sequence of Y35W mutant
atggaatccaagatcatcggtaaagtcaacttcgaggagcatctgctggataaagagctgaaactgatcgacactttcgagttcaacgacagctacagcgaatgggcttctggtatttggaagacttgcatgctgtggaaccgttctggtcagaaagatgaccatctgtctattgaacatgatacctacgtgaaacctactgaatacggcaaacagctggcatacgtaaacgaaatcatcgctaacacctttaagaaagaacacatcaagacggtgcgtctgttcatgtgtatcaacggcctgatcatcccacacaaagactacctggaattcaagaaaggcttcacccgtatccacatcccgctgaaaatcaacgaacacgcactgacctctgaagaagatgttgtttacaacatgcagaaaggtgaaatttggttcatcgaaggccgtaaaatccacagcgctgccaatttcagcaaagtgaaacgtatcaacctggtcatcgacttcgcgccggatattccgtttgaagaactgttcctgaattctgagaactatcaaccgaacctgatcccgaaaatctctcaacgtacccagctgaaagaagaagagctgggttatatcaaaggtctgtctaaaattatcaatgaaatgaactttgacgacatcctgtccattctgagcaaaattcacttctatcgcaacgtttcctccgaactggtttttggctggctggacgaaattgccacggcgtccaacaactataacattcagcgcaaagcgcaggaagtaaccgatctgctgattcgcaaaggcccgattaataactaa

SEQ ID NO: 32 - protein, 276 aa, Artificial Sequence
  amino acid sequence of Y35W mutant
MESKIIGKVNFEEHLLDKELKLIDTFEFNDSYSEWASGIWKTCMLWNRSGQKDDHLSIEHDTYVKPTEYGKQLAYVNEIIANTFKKEHIKTVRLFMCINGLIIPHKDYLEFKKGFTRIHIPLKINEHALTSEEDVVYNMQKGEIWFIEGRKIHSAANFSKVKRINLVIDFAPDIPFEELFLNSENYQPNLIPKISQRTQLKEEELGYIKGLSKIINEMNFDDILSILSKIHFYRNVSSELVFGWLDEIATASNNYNIQRKAQEVTDLLIRKGPINN

SEQ ID NO: 33 - DNA, 831 bp, Artificial Sequence
  gene sequence of Y35K mutant
atggaatccaagatcatcggtaaagtcaacttcgaggagcatctgctggataaagagctgaaactgatcgacactttcgagttcaacgacagctacagcgaaaaagcttctggtatttggaagacttgcatgctgtggaaccgttctggtcagaaagatgaccatctgtctattgaacatgatacctacgtgaaacctactgaatacggcaaacagctggcatacgtaaacgaaatcatcgctaacacctttaagaaagaacacatcaagacggtgcgtctgttcatgtgtatcaacggcctgatcatcccacacaaagactacctggaattcaagaaaggcttcacccgtatccacatcccgctgaaaatcaacgaacacgcactgacctctgaagaagatgttgtttacaacatgcagaaaggtgaaatttggttcatcgaaggccgtaaaatccacagcgctgccaatttcagcaaagtgaaacgtatcaacctggtcatcgacttcgcgccggatattccgtttgaagaactgttcctgaattctgagaactatcaaccgaacctgatcccgaaaatctctcaacgtacccagctgaaagaagaagagctgggttatatcaaaggtctgtctaaaattatcaatgaaatgaactttgacgacatcctgtccattctgagcaaaattcacttctatcgcaacgtttcctccgaactggtttttggctggctggacgaaattgccacggcgtccaacaactataacattcagcgcaaagcgcaggaagtaaccgatctgctgattcgcaaaggcccgattaataactaa

SEQ ID NO: 34 - protein, 276 aa, Artificial Sequence
  amino acid sequence of Y35K mutant
MESKIIGKVNFEEHLLDKELKLIDTFEFNDSYSEKASGIWKTCMLWNRSGQKDDHLSIEHDTYVKPTEYGKQLAYVNEIIANTFKKEHIKTVRLFMCINGLIIPHKDYLEFKKGFTRIHIPLKINEHALTSEEDVVYNMQKGEIWFIEGRKIHSAANFSKVKRINLVIDFAPDIPFEELFLNSENYQPNLIPKISQRTQLKEEELGYIKGLSKIINEMNFDDILSILSKIHFYRNVSSELVFGWLDEIATASNNYNIQRKAQEVTDLLIRKGPINN

SEQ ID NO: 35 - DNA, 831 bp, Artificial Sequence
  gene sequence of S37W mutant
atggaatccaagatcatcggtaaagtcaacttcgaggagcatctgctggataaagagctgaaactgatcgacactttcgagttcaacgacagctacagcgaatacgcttggggtatttggaagacttgcatgctgtggaaccgttctggtcagaaagatgaccatctgtctattgaacatgatacctacgtgaaacctactgaatacggcaaacagctggcatacgtaaacgaaatcatcgctaacacctttaagaaagaacacatcaagacggtgcgtctgttcatgtgtatcaacggcctgatcatcccacacaaagactacctggaattcaagaaaggcttcacccgtatccacatcccgctgaaaatcaacgaacacgcactgacctctgaagaagatgttgtttacaacatgcagaaaggtgaaatttggttcatcgaaggccgtaaaatccacagcgctgccaatttcagcaaagtgaaacgtatcaacctggtcatcgacttcgcgccggatattccgtttgaagaactgttcctgaattctgagaactatcaaccgaacctgatcccgaaaatctctcaacgtacccagctgaaagaagaagagctgggttatatcaaaggtctgtctaaaattatcaatgaaatgaactttgacgacatcctgtccattctgagcaaaattcacttctatcgcaacgtttcctccgaactggtttttggctggctggacgaaattgccacggcgtccaacaactataacattcagcgcaaagcgcaggaagtaaccgatctgctgattcgcaaaggcccgattaataactaa

SEQ ID NO: 36 - protein, 276 aa, Artificial Sequence
  amino acid sequence of S37W mutant
MESKIIGKVNFEEHLLDKELKLIDTFEFNDSYSEYAWGIWKTCMLWNRSGQKDDHLSIEHDTYVKPTEYGKQLAYVNEIIANTFKKEHIKTVRLFMCINGLIIPHKDYLEFKKGFTRIHIPLKINEHALTSEEDVVYNMQKGEIWFIEGRKIHSAANFSKVKRINLVIDFAPDIPFEELFLNSENYQPNLIPKISQRTQLKEEELGYIKGLSKIINEMNFDDILSILSKIHFYRNVSSELVFGWLDEIATASNNYNIQRKAQEVTDLLIRKGPINN

SEQ ID NO: 37 - DNA, 831 bp, Artificial Sequence
  gene sequence of S37F mutant
atggaatccaagatcatcggtaaagtcaacttcgaggagcatctgctggataaagagctgaaactgatcgacactttcgagttcaacgacagctacagcgaatacgcttttggtatttggaagacttgcatgctgtggaaccgttctggtcagaaagatgaccatctgtctattgaacatgatacctacgtgaaacctactgaatacggcaaacagctggcatacgtaaacgaaatcatcgctaacacctttaagaaagaacacatcaagacggtgcgtctgttcatgtgtatcaacggcctgatcatcccacacaaagactacctggaattcaagaaaggcttcacccgtatccacatcccgctgaaaatcaacgaacacgcactgacctctgaagaagatgttgtttacaacatgcagaaaggtgaaatttggttcatcgaaggccgtaaaatccacagcgctgccaatttcagcaaagtgaaacgtatcaacctggtcatcgacttcgcgccggatattccgtttgaagaactgttcctgaattctgagaactatcaaccgaacctgatcccgaaaatctctcaacgtacccagctgaaagaagaagagctgggttatatcaaaggtctgtctaaaattatcaatgaaatgaactttgacgacatcctgtccattctgagcaaaattcacttctatcgcaacgtttcctccgaactggtttttggctggctggacgaaattgccacggcgtccaacaactataacattcagcgcaaagcgcaggaagtaaccgatctgctgattcgcaaaggcccgattaataactaa

SEQ ID NO: 38 - protein, 276 aa, Artificial Sequence
  amino acid sequence of S37F mutant
MESKIIGKVNFEEHLLDKELKLIDTFEFNDSYSEYAFGIWKTCMLWNRSGQKDDHLSIEHDTYVKPTEYGKQLAYVNEIIANTFKKEHIKTVRLFMCINGLIIPHKDYLEFKKGFTRIHIPLKINEHALTSEEDVVYNMQKGEIWFIEGRKIHSAANFSKVKRINLVIDFAPDIPFEELFLNSENYQPNLIPKISQRTQLKEEELGYIKGLSKIINEMNFDDILSILSKIHFYRNVSSELVFGWLDEIATASNNYNIQRKAQEVTDLLIRKGPINN

SEQ ID NO: 39 - DNA, 831 bp, Artificial Sequence
  gene sequence of S37E mutant
atggaatccaagatcatcggtaaagtcaacttcgaggagcatctgctggataaagagctgaaactgatcgacactttcgagttcaacgacagctacagcgaatacgctgaaggtatttggaagacttgcatgctgtggaaccgttctggtcagaaagatgaccatctgtctattgaacatgatacctacgtgaaacctactgaatacggcaaacagctggcatacgtaaacgaaatcatcgctaacacctttaagaaagaacacatcaagacggtgcgtctgttcatgtgtatcaacggcctgatcatcccacacaaagactacctggaattcaagaaaggcttcacccgtatccacatcccgctgaaaatcaacgaacacgcactgacctctgaagaagatgttgtttacaacatgcagaaaggtgaaatttggttcatcgaaggccgtaaaatccacagcgctgccaatttcagcaaagtgaaacgtatcaacctggtcatcgacttcgcgccggatattccgtttgaagaactgttcctgaattctgagaactatcaaccgaacctgatcccgaaaatctctcaacgtacccagctgaaagaagaagagctgggttatatcaaaggtctgtctaaaattatcaatgaaatgaactttgacgacatcctgtccattctgagcaaaattcacttctatcgcaacgtttcctccgaactggtttttggctggctggacgaaattgccacggcgtccaacaactataacattcagcgcaaagcgcaggaagtaaccgatctgctgattcgcaaaggcccgattaataactaa

SEQ ID NO: 40 - protein, 276 aa, Artificial Sequence
  amino acid sequence of S37E mutant
MESKIIGKVNFEEHLLDKELKLIDTFEFNDSYSEYAEGIWKTCMLWNRSGQKDDHLSIEHDTYVKPTEYGKQLAYVNEIIANTFKKEHIKTVRLFMCINGLIIPHKDYLEFKKGFTRIHIPLKINEHALTSEEDVVYNMQKGEIWFIEGRKIHSAANFSKVKRINLVIDFAPDIPFEELFLNSENYQPNLIPKISQRTQLKEEELGYIKGLSKIINEMNFDDILSILSKIHFYRNVSSELVFGWLDEIATASNNYNIQRKAQEVTDLLIRKGPINN

SEQ ID NO: 41 - DNA, 831 bp, Artificial Sequence
  gene sequence of S37N mutant
atggaatccaagatcatcggtaaagtcaacttcgaggagcatctgctggataaagagctgaaactgatcgacactttcgagttcaacgacagctacagcgaatacgctaatggtatttggaagacttgcatgctgtggaaccgttctggtcagaaagatgaccatctgtctattgaacatgatacctacgtgaaacctactgaatacggcaaacagctggcatacgtaaacgaaatcatcgctaacacctttaagaaagaacacatcaagacggtgcgtctgttcatgtgtatcaacggcctgatcatcccacacaaagactacctggaattcaagaaaggcttcacccgtatccacatcccgctgaaaatcaacgaacacgcactgacctctgaagaagatgttgtttacaacatgcagaaaggtgaaatttggttcatcgaaggccgtaaaatccacagcgctgccaatttcagcaaagtgaaacgtatcaacctggtcatcgacttcgcgccggatattccgtttgaagaactgttcctgaattctgagaactatcaaccgaacctgatcccgaaaatctctcaacgtacccagctgaaagaagaagagctgggttatatcaaaggtctgtctaaaattatcaatgaaatgaactttgacgacatcctgtccattctgagcaaaattcacttctatcgcaacgtttcctccgaactggtttttggctggctggacgaaattgccacggcgtccaacaactataacattcagcgcaaagcgcaggaagtaaccgatctgctgattcgcaaaggcccgattaataactaa

SEQ ID NO: 42 - protein, 276 aa, Artificial Sequence
  amino acid sequence of S37N mutant
MESKIIGKVNFEEHLLDKELKLIDTFEFNDSYSEYANGIWKTCMLWNRSGQKDDHLSIEHDTYVKPTEYGKQLAYVNEIIANTFKKEHIKTVRLFMCINGLIIPHKDYLEFKKGFTRIHIPLKINEHALTSEEDVVYNMQKGEIWFIEGRKIHSAANFSKVKRINLVIDFAPDIPFEELFLNSENYQPNLIPKISQRTQLKEEELGYIKGLSKIINEMNFDDILSILSKIHFYRNVSSELVFGWLDEIATASNNYNIQRKAQEVTDLLIRKGPINN

SEQ ID NO: 43 - DNA, 831 bp, Artificial Sequence
  gene sequence of S37T mutant
atggaatccaagatcatcggtaaagtcaacttcgaggagcatctgctggataaagagctgaaactgatcgacactttcgagttcaacgacagctacagcgaatacgctaccggtatttggaagacttgcatgctgtggaaccgttctggtcagaaagatgaccatctgtctattgaacatgatacctacgtgaaacctactgaatacggcaaacagctggcatacgtaaacgaaatcatcgctaacacctttaagaaagaacacatcaagacggtgcgtctgttcatgtgtatcaacggcctgatcatcccacacaaagactacctggaattcaagaaaggcttcacccgtatccacatcccgctgaaaatcaacgaacacgcactgacctctgaagaagatgttgtttacaacatgcagaaaggtgaaatttggttcatcgaaggccgtaaaatccacagcgctgccaatttcagcaaagtgaaacgtatcaacctggtcatcgacttcgcgccggatattccgtttgaagaactgttcctgaattctgagaactatcaaccgaacctgatcccgaaaatctctcaacgtacccagctgaaagaagaagagctgggttatatcaaaggtctgtctaaaattatcaatgaaatgaactttgacgacatcctgtccattctgagcaaaattcacttctatcgcaacgtttcctccgaactggtttttggctggctggacgaaattgccacggcgtccaacaactataacattcagcgcaaagcgcaggaagtaaccgatctgctgattcgcaaaggcccgattaataactaa

SEQ ID NO: 44 - protein, 276 aa, Artificial Sequence
  amino acid sequence of S37T mutant
MESKIIGKVNFEEHLLDKELKLIDTFEFNDSYSEYATGIWKTCMLWNRSGQKDDHLSIEHDTYVKPTEYGKQLAYVNEIIANTFKKEHIKTVRLFMCINGLIIPHKDYLEFKKGFTRIHIPLKINEHALTSEEDVVYNMQKGEIWFIEGRKIHSAANFSKVKRINLVIDFAPDIPFEELFLNSENYQPNLIPKISQRTQLKEEELGYIKGLSKIINEMNFDDILSILSKIHFYRNVSSELVFGWLDEIATASNNYNIQRKAQEVTDLLIRKGPINN

SEQ ID NO: 45 - DNA, 831 bp, Artificial Sequence
  gene sequence of S37C mutant
atggaatccaagatcatcggtaaagtcaacttcgaggagcatctgctggataaagagctgaaactgatcgacactttcgagttcaacgacagctacagcgaatacgcttgtggtatttggaagacttgcatgctgtggaaccgttctggtcagaaagatgaccatctgtctattgaacatgatacctacgtgaaacctactgaatacggcaaacagctggcatacgtaaacgaaatcatcgctaacacctttaagaaagaacacatcaagacggtgcgtctgttcatgtgtatcaacggcctgatcatcccacacaaagactacctggaattcaagaaaggcttcacccgtatccacatcccgctgaaaatcaacgaacacgcactgacctctgaagaagatgttgtttacaacatgcagaaaggtgaaatttggttcatcgaaggccgtaaaatccacagcgctgccaatttcagcaaagtgaaacgtatcaacctggtcatcgacttcgcgccggatattccgtttgaagaactgttcctgaattctgagaactatcaaccgaacctgatcccgaaaatctctcaacgtacccagctgaaagaagaagagctgggttatatcaaaggtctgtctaaaattatcaatgaaatgaactttgacgacatcctgtccattctgagcaaaattcacttctatcgcaacgtttcctccgaactggtttttggctggctggacgaaattgccacggcgtccaacaactataacattcagcgcaaagcgcaggaagtaaccgatctgctgattcgcaaaggcccgattaataactaa

SEQ ID NO: 46 - protein, 276 aa, Artificial Sequence
  amino acid sequence of S37C mutant
MESKIIGKVNFEEHLLDKELKLIDTFEFNDSYSEYACGIWKTCMLWNRSGQKDDHLSIEHDTYVKPTEYGKQLAYVNEIIANTFKKEHIKTVRLFMCINGLIIPHKDYLEFKKGFTRIHIPLKINEHALTSEEDVVYNMQKGEIWFIEGRKIHSAANFSKVKRINLVIDFAPDIPFEELFLNSENYQPNLIPKISQRTQLKEEELGYIKGLSKIINEMNFDDILSILSKIHFYRNVSSELVFGWLDEIATASNNYNIQRKAQEVTDLLIRKGPINN

SEQ ID NO: 47 - DNA, 831 bp, Artificial Sequence
  gene sequence of I39K mutant
atggaatccaagatcatcggtaaagtcaacttcgaggagcatctgctggataaagagctgaaactgatcgacactttcgagttcaacgacagctacagcgaatacgcttctggtaaatggaagacttgcatgctgtggaaccgttctggtcagaaagatgaccatctgtctattgaacatgatacctacgtgaaacctactgaatacggcaaacagctggcatacgtaaacgaaatcatcgctaacacctttaagaaagaacacatcaagacggtgcgtctgttcatgtgtatcaacggcctgatcatcccacacaaagactacctggaattcaagaaaggcttcacccgtatccacatcccgctgaaaatcaacgaacacgcactgacctctgaagaagatgttgtttacaacatgcagaaaggtgaaatttggttcatcgaaggccgtaaaatccacagcgctgccaatttcagcaaagtgaaacgtatcaacctggtcatcgacttcgcgccggatattccgtttgaagaactgttcctgaattctgagaactatcaaccgaacctgatcccgaaaatctctcaacgtacccagctgaaagaagaagagctgggttatatcaaaggtctgtctaaaattatcaatgaaatgaactttgacgacatcctgtccattctgagcaaaattcacttctatcgcaacgtttcctccgaactggtttttggctggctggacgaaattgccacggcgtccaacaactataacattcagcgcaaagcgcaggaagtaaccgatctgctgattcgcaaaggcccgattaataactaa

SEQ ID NO: 48 - protein, 276 aa, Artificial Sequence
  amino acid sequence of I39K mutant
MESKIIGKVNFEEHLLDKELKLIDTFEFNDSYSEYASGKWKTCMLWNRSGQKDDHLSIEHDTYVKPTEYGKQLAYVNEIIANTFKKEHIKTVRLFMCINGLIIPHKDYLEFKKGFTRIHIPLKINEHALTSEEDVVYNMQKGEIWFIEGRKIHSAANFSKVKRINLVIDFAPDIPFEELFLNSENYQPNLIPKISQRTQLKEEELGYIKGLSKIINEMNFDDILSILSKIHFYRNVSSELVFGWLDEIATASNNYNIQRKAQEVTDLLIRKGPINN

SEQ ID NO: 49 - DNA, 831 bp, Artificial Sequence
  gene sequence of I39R mutant
atggaatccaagatcatcggtaaagtcaacttcgaggagcatctgctggataaagagctgaaactgatcgacactttcgagttcaacgacagctacagcgaatacgcttctggtcgttggaagacttgcatgctgtggaaccgttctggtcagaaagatgaccatctgtctattgaacatgatacctacgtgaaacctactgaatacggcaaacagctggcatacgtaaacgaaatcatcgctaacacctttaagaaagaacacatcaagacggtgcgtctgttcatgtgtatcaacggcctgatcatcccacacaaagactacctggaattcaagaaaggcttcacccgtatccacatcccgctgaaaatcaacgaacacgcactgacctctgaagaagatgttgtttacaacatgcagaaaggtgaaatttggttcatcgaaggccgtaaaatccacagcgctgccaatttcagcaaagtgaaacgtatcaacctggtcatcgacttcgcgccggatattccgtttgaagaactgttcctgaattctgagaactatcaaccgaacctgatcccgaaaatctctcaacgtacccagctgaaagaagaagagctgggttatatcaaaggtctgtctaaaattatcaatgaaatgaactttgacgacatcctgtccattctgagcaaaattcacttctatcgcaacgtttcctccgaactggtttttggctggctggacgaaattgccacggcgtccaacaactataacattcagcgcaaagcgcaggaagtaaccgatctgctgattcgcaaaggcccgattaataactaa

SEQ ID NO: 50 - protein, 276 aa, Artificial Sequence
  amino acid sequence of I39R mutant
MESKIIGKVNFEEHLLDKELKLIDTFEFNDSYSEYASGRWKTCMLWNRSGQKDDHLSIEHDTYVKPTEYGKQLAYVNEIIANTFKKEHIKTVRLFMCINGLIIPHKDYLEFKKGFTRIHIPLKINEHALTSEEDVVYNMQKGEIWFIEGRKIHSAANFSKVKRINLVIDFAPDIPFEELFLNSENYQPNLIPKISQRTQLKEEELGYIKGLSKIINEMNFDDILSILSKIHFYRNVSSELVFGWLDEIATASNNYNIQRKAQEVTDLLIRKGPINN

SEQ ID NO: 51 - DNA, 831 bp, Artificial Sequence
  gene sequence of W40F mutant
atggaatccaagatcatcggtaaagtcaacttcgaggagcatctgctggataaagagctgaaactgatcgacactttcgagttcaacgacagctacagcgaatacgcttctggtatttttaagacttgcatgctgtggaaccgttctggtcagaaagatgaccatctgtctattgaacatgatacctacgtgaaacctactgaatacggcaaacagctggcatacgtaaacgaaatcatcgctaacacctttaagaaagaacacatcaagacggtgcgtctgttcatgtgtatcaacggcctgatcatcccacacaaagactacctggaattcaagaaaggcttcacccgtatccacatcccgctgaaaatcaacgaacacgcactgacctctgaagaagatgttgtttacaacatgcagaaaggtgaaatttggttcatcgaaggccgtaaaatccacagcgctgccaatttcagcaaagtgaaacgtatcaacctggtcatcgacttcgcgccggatattccgtttgaagaactgttcctgaattctgagaactatcaaccgaacctgatcccgaaaatctctcaacgtacccagctgaaagaagaagagctgggttatatcaaaggtctgtctaaaattatcaatgaaatgaactttgacgacatcctgtccattctgagcaaaattcacttctatcgcaacgtttcctccgaactggtttttggctggctggacgaaattgccacggcgtccaacaactataacattcagcgcaaagcgcaggaagtaaccgatctgctgattcgcaaaggcccgattaataactaa

SEQ ID NO: 52 - protein, 276 aa, Artificial Sequence
  amino acid sequence of W40F mutant
MESKIIGKVNFEEHLLDKELKLIDTFEFNDSYSEYASGIFKTCMLWNRSGQKDDHLSIEHDTYVKPTEYGKQLAYVNEIIANTFKKEHIKTVRLFMCINGLIIPHKDYLEFKKGFTRIHIPLKINEHALTSEEDVVYNMQKGEIWFIEGRKIHSAANFSKVKRINLVIDFAPDIPFEELFLNSENYQPNLIPKISQRTQLKEEELGYIKGLSKIINEMNFDDILSILSKIHFYRNVSSELVFGWLDEIATASNNYNIQRKAQEVTDLLIRKGPINN

SEQ ID NO: 53 - DNA, 831 bp, Artificial Sequence
  gene sequence of K41E mutant
atggaatccaagatcatcggtaaagtcaacttcgaggagcatctgctggataaagagctgaaactgatcgacactttcgagttcaacgacagctacagcgaatacgcttctggtatttgggaaacttgcatgctgtggaaccgttctggtcagaaagatgaccatctgtctattgaacatgatacctacgtgaaacctactgaatacggcaaacagctggcatacgtaaacgaaatcatcgctaacacctttaagaaagaacacatcaagacggtgcgtctgttcatgtgtatcaacggcctgatcatcccacacaaagactacctggaattcaagaaaggcttcacccgtatccacatcccgctgaaaatcaacgaacacgcactgacctctgaagaagatgttgtttacaacatgcagaaaggtgaaatttggttcatcgaaggccgtaaaatccacagcgctgccaatttcagcaaagtgaaacgtatcaacctggtcatcgacttcgcgccggatattccgtttgaagaactgttcctgaattctgagaactatcaaccgaacctgatcccgaaaatctctcaacgtacccagctgaaagaagaagagctgggttatatcaaaggtctgtctaaaattatcaatgaaatgaactttgacgacatcctgtccattctgagcaaaattcacttctatcgcaacgtttcctccgaactggtttttggctggctggacgaaattgccacggcgtccaacaactataacattcagcgcaaagcgcaggaagtaaccgatctgctgattcgcaaaggcccgattaataactaa

SEQ ID NO: 54 - protein, 276 aa, Artificial Sequence
  amino acid sequence of K41E mutant
MESKIIGKVNFEEHLLDKELKLIDTFEFNDSYSEYASGIWETCMLWNRSGQKDDHLSIEHDTYVKPTEYGKQLAYVNEIIANTFKKEHIKTVRLFMCINGLIIPHKDYLEFKKGFTRIHIPLKINEHALTSEEDVVYNMQKGEIWFIEGRKIHSAANFSKVKRINLVIDFAPDIPFEELFLNSENYQPNLIPKISQRTQLKEEELGYIKGLSKIINEMNFDDILSILSKIHFYRNVSSELVFGWLDEIATASNNYNIQRKAQEVTDLLIRKGPINN

SEQ ID NO: 55 - DNA, 831 bp, Artificial Sequence
  gene sequence of D54G mutant
atggaatccaagatcatcggtaaagtcaacttcgaggagcatctgctggataaagagctgaaactgatcgacactttcgagttcaacgacagctacagcgaatacgcttctggtatttggaagacttgcatgctgtggaaccgttctggtcagaaagatggtcatctgtctattgaacatgatacctacgtgaaacctactgaatacggcaaacagctggcatacgtaaacgaaatcatcgctaacacctttaagaaagaacacatcaagacggtgcgtctgttcatgtgtatcaacggcctgatcatcccacacaaagactacctggaattcaagaaaggcttcacccgtatccacatcccgctgaaaatcaacgaacacgcactgacctctgaagaagatgttgtttacaacatgcagaaaggtgaaatttggttcatcgaaggccgtaaaatccacagcgctgccaatttcagcaaagtgaaacgtatcaacctggtcatcgacttcgcgccggatattccgtttgaagaactgttcctgaattctgagaactatcaaccgaacctgatcccgaaaatctctcaacgtacccagctgaaagaagaagagctgggttatatcaaaggtctgtctaaaattatcaatgaaatgaactttgacgacatcctgtccattctgagcaaaattcacttctatcgcaacgtttcctccgaactggtttttggctggctggacgaaattgccacggcgtccaacaactataacattcagcgcaaagcgcaggaagtaaccgatctgctgattcgcaaaggcccgattaataactaa

SEQ ID NO: 56 - protein, 276 aa, Artificial Sequence
  amino acid sequence of D54G mutant
MESKIIGKVNFEEHLLDKELKLIDTFEFNDSYSEYASGIWKTCMLWNRSGQKDGHLSIEHDTYVKPTEYGKQLAYVNEIIANTFKKEHIKTVRLFMCINGLIIPHKDYLEFKKGFTRIHIPLKINEHALTSEEDVVYNMQKGEIWFIEGRKIHSAANFSKVKRINLVIDFAPDIPFEELFLNSENYQPNLIPKISQRTQLKEEELGYIKGLSKIINEMNFDDILSILSKIHFYRNVSSELVFGWLDEIATASNNYNIQRKAQEVTDLLIRKGPINN

SEQ ID NO: 57 - DNA, 831 bp, Artificial Sequence
  gene sequence of H55Q mutant
atggaatccaagatcatcggtaaagtcaacttcgaggagcatctgctggataaagagctgaaactgatcgacactttcgagttcaacgacagctacagcgaatacgcttctggtatttggaagacttgcatgctgtggaaccgttctggtcagaaagatgaccagctgtctattgaacatgatacctacgtgaaacctactgaatacggcaaacagctggcatacgtaaacgaaatcatcgctaacacctttaagaaagaacacatcaagacggtgcgtctgttcatgtgtatcaacggcctgatcatcccacacaaagactacctggaattcaagaaaggcttcacccgtatccacatcccgctgaaaatcaacgaacacgcactgacctctgaagaagatgttgtttacaacatgcagaaaggtgaaatttggttcatcgaaggccgtaaaatccacagcgctgccaatttcagcaaagtgaaacgtatcaacctggtcatcgacttcgcgccggatattccgtttgaagaactgttcctgaattctgagaactatcaaccgaacctgatcccgaaaatctctcaacgtacccagctgaaagaagaagagctgggttatatcaaaggtctgtctaaaattatcaatgaaatgaactttgacgacatcctgtccattctgagcaaaattcacttctatcgcaacgtttcctccgaactggtttttggctggctggacgaaattgccacggcgtccaacaactataacattcagcgcaaagcgcaggaagtaaccgatctgctgattcgcaaaggcccgattaataactaa

SEQ ID NO: 58 - protein, 276 aa, Artificial Sequence
  amino acid sequence of H55Q mutant
MESKIIGKVNFEEHLLDKELKLIDTFEFNDSYSEYASGIWKTCMLWNRSGQKDDQLSIEHDTYVKPTEYGKQLAYVNEIIANTFKKEHIKTVRLFMCINGLIIPHKDYLEFKKGFTRIHIPLKINEHALTSEEDVVYNMQKGEIWFIEGRKIHSAANFSKVKRINLVIDFAPDIPFEELFLNSENYQPNLIPKISQRTQLKEEELGYIKGLSKIINEMNFDDILSILSKIHFYRNVSSELVFGWLDEIATASNNYNIQRKAQEVTDLLIRKGPINN

SEQ ID NO: 59 - DNA, 831 bp, Artificial Sequence
  gene sequence of S57L mutant
atggaatccaagatcatcggtaaagtcaacttcgaggagcatctgctggataaagagctgaaactgatcgacactttcgagttcaacgacagctacagcgaatacgcttctggtatttggaagacttgcatgctgtggaaccgttctggtcagaaagatgaccatctgctgattgaacatgatacctacgtgaaacctactgaatacggcaaacagctggcatacgtaaacgaaatcatcgctaacacctttaagaaagaacacatcaagacggtgcgtctgttcatgtgtatcaacggcctgatcatcccacacaaagactacctggaattcaagaaaggcttcacccgtatccacatcccgctgaaaatcaacgaacacgcactgacctctgaagaagatgttgtttacaacatgcagaaaggtgaaatttggttcatcgaaggccgtaaaatccacagcgctgccaatttcagcaaagtgaaacgtatcaacctggtcatcgacttcgcgccggatattccgtttgaagaactgttcctgaattctgagaactatcaaccgaacctgatcccgaaaatctctcaacgtacccagctgaaagaagaagagctgggttatatcaaaggtctgtctaaaattatcaatgaaatgaactttgacgacatcctgtccattctgagcaaaattcacttctatcgcaacgtttcctccgaactggtttttggctggctggacgaaattgccacggcgtccaacaactataacattcagcgcaaagcgcaggaagtaaccgatctgctgattcgcaaaggcccgattaataactaa

SEQ ID NO: 60 - protein, 276 aa, Artificial Sequence
  amino acid sequence of S57L mutant
MESKIIGKVNFEEHLLDKELKLIDTFEFNDSYSEYASGIWKTCMLWNRSGQKDDHLLIEHDTYVKPTEYGKQLAYVNEIIANTFKKEHIKTVRLFMCINGLIIPHKDYLEFKKGFTRIHIPLKINEHALTSEEDVVYNMQKGEIWFIEGRKIHSAANFSKVKRINLVIDFAPDIPFEELFLNSENYQPNLIPKISQRTQLKEEELGYIKGLSKIINEMNFDDILSILSKIHFYRNVSSELVFGWLDEIATASNNYNIQRKAQEVTDLLIRKGPINN

SEQ ID NO: 61 - DNA, 831 bp, Artificial Sequence
  gene sequence of I58T mutant
atggaatccaagatcatcggtaaagtcaacttcgaggagcatctgctggataaagagctgaaactgatcgacactttcgagttcaacgacagctacagcgaatacgcttctggtatttggaagacttgcatgctgtggaaccgttctggtcagaaagatgaccatctgtctaccgaacatgatacctacgtgaaacctactgaatacggcaaacagctggcatacgtaaacgaaatcatcgctaacacctttaagaaagaacacatcaagacggtgcgtctgttcatgtgtatcaacggcctgatcatcccacacaaagactacctggaattcaagaaaggcttcacccgtatccacatcccgctgaaaatcaacgaacacgcactgacctctgaagaagatgttgtttacaacatgcagaaaggtgaaatttggttcatcgaaggccgtaaaatccacagcgctgccaatttcagcaaagtgaaacgtatcaacctggtcatcgacttcgcgccggatattccgtttgaagaactgttcctgaattctgagaactatcaaccgaacctgatcccgaaaatctctcaacgtacccagctgaaagaagaagagctgggttatatcaaaggtctgtctaaaattatcaatgaaatgaactttgacgacatcctgtccattctgagcaaaattcacttctatcgcaacgtttcctccgaactggtttttggctggctggacgaaattgccacggcgtccaacaactataacattcagcgcaaagcgcaggaagtaaccgatctgctgattcgcaaaggcccgattaataactaa

SEQ ID NO: 62 - protein, 276 aa, Artificial Sequence
  amino acid sequence of I58T mutant
MESKIIGKVNFEEHLLDKELKLIDTFEFNDSYSEYASGIWKTCMLWNRSGQKDDHLSTEHDTYVKPTEYGKQLAYVNEIIANTFKKEHIKTVRLFMCINGLIIPHKDYLEFKKGFTRIHIPLKINEHALTSEEDVVYNMQKGEIWFIEGRKIHSAANFSKVKRINLVIDFAPDIPFEELFLNSENYQPNLIPKISQRTQLKEEELGYIKGLSKIINEMNFDDILSILSKIHFYRNVSSELVFGWLDEIATASNNYNIQRKAQEVTDLLIRKGPINN

SEQ ID NO: 63 - DNA, 831 bp, Artificial Sequence
  gene sequence of I58Y mutant
atggaatccaagatcatcggtaaagtcaacttcgaggagcatctgctggataaagagctgaaactgatcgacactttcgagttcaacgacagctacagcgaatacgcttctggtatttggaagacttgcatgctgtggaaccgttctggtcagaaagatgaccatctgtcttatgaacatgatacctacgtgaaacctactgaatacggcaaacagctggcatacgtaaacgaaatcatcgctaacacctttaagaaagaacacatcaagacggtgcgtctgttcatgtgtatcaacggcctgatcatcccacacaaagactacctggaattcaagaaaggcttcacccgtatccacatcccgctgaaaatcaacgaacacgcactgacctctgaagaagatgttgtttacaacatgcagaaaggtgaaatttggttcatcgaaggccgtaaaatccacagcgctgccaatttcagcaaagtgaaacgtatcaacctggtcatcgacttcgcgccggatattccgtttgaagaactgttcctgaattctgagaactatcaaccgaacctgatcccgaaaatctctcaacgtacccagctgaaagaagaagagctgggttatatcaaaggtctgtctaaaattatcaatgaaatgaactttgacgacatcctgtccattctgagcaaaattcacttctatcgcaacgtttcctccgaactggtttttggctggctggacgaaattgccacggcgtccaacaactataacattcagcgcaaagcgcaggaagtaaccgatctgctgattcgcaaaggcccgattaataactaa

SEQ ID NO: 64 - protein, 276 aa, Artificial Sequence
  amino acid sequence of I58Y mutant
MESKIIGKVNFEEHLLDKELKLIDTFEFNDSYSEYASGIWKTCMLWNRSGQKDDHLSYEHDTYVKPTEYGKQLAYVNEIIANTFKKEHIKTVRLFMCINGLIIPHKDYLEFKKGFTRIHIPLKINEHALTSEEDVVYNMQKGEIWFIEGRKIHSAANFSKVKRINLVIDFAPDIPFEELFLNSENYQPNLIPKISQRTQLKEEELGYIKGLSKIINEMNFDDILSILSKIHFYRNVSSELVFGWLDEIATASNNYNIQRKAQEVTDLLIRKGPINN

SEQ ID NO: 65 - DNA, 831 bp, Artificial Sequence
  gene sequence of I58A mutant
atggaatccaagatcatcggtaaagtcaacttcgaggagcatctgctggataaagagctgaaactgatcgacactttcgagttcaacgacagctacagcgaatacgcttctggtatttggaagacttgcatgctgtggaaccgttctggtcagaaagatgaccatctgtctgcagaacatgatacctacgtgaaacctactgaatacggcaaacagctggcatacgtaaacgaaatcatcgctaacacctttaagaaagaacacatcaagacggtgcgtctgttcatgtgtatcaacggcctgatcatcccacacaaagactacctggaattcaagaaaggcttcacccgtatccacatcccgctgaaaatcaacgaacacgcactgacctctgaagaagatgttgtttacaacatgcagaaaggtgaaatttggttcatcgaaggccgtaaaatccacagcgctgccaatttcagcaaagtgaaacgtatcaacctggtcatcgacttcgcgccggatattccgtttgaagaactgttcctgaattctgagaactatcaaccgaacctgatcccgaaaatctctcaacgtacccagctgaaagaagaagagctgggttatatcaaaggtctgtctaaaattatcaatgaaatgaactttgacgacatcctgtccattctgagcaaaattcacttctatcgcaacgtttcctccgaactggtttttggctggctggacgaaattgccacggcgtccaacaactataacattcagcgcaaagcgcaggaagtaaccgatctgctgattcgcaaaggcccgattaataactaa

SEQ ID NO: 66 - protein, 276 aa, Artificial Sequence
  amino acid sequence of I58A mutant
MESKIIGKVNFEEHLLDKELKLIDTFEFNDSYSEYASGIWKTCMLWNRSGQKDDHLSAEHDTYVKPTEYGKQLAYVNEIIANTFKKEHIKTVRLFMCINGLIIPHKDYLEFKKGFTRIHIPLKINEHALTSEEDVVYNMQKGEIWFIEGRKIHSAANFSKVKRINLVIDFAPDIPFEELFLNSENYQPNLIPKISQRTQLKEEELGYIKGLSKIINEMNFDDILSILSKIHFYRNVSSELVFGWLDEIATASNNYNIQRKAQEVTDLLIRKGPINN

SEQ ID NO: 67 - DNA, 831 bp, Artificial Sequence
  gene sequence of I58R mutant
atggaatccaagatcatcggtaaagtcaacttcgaggagcatctgctggataaagagctgaaactgatcgacactttcgagttcaacgacagctacagcgaatacgcttctggtatttggaagacttgcatgctgtggaaccgttctggtcagaaagatgaccatctgtctcgtgaacatgatacctacgtgaaacctactgaatacggcaaacagctggcatacgtaaacgaaatcatcgctaacacctttaagaaagaacacatcaagacggtgcgtctgttcatgtgtatcaacggcctgatcatcccacacaaagactacctggaattcaagaaaggcttcacccgtatccacatcccgctgaaaatcaacgaacacgcactgacctctgaagaagatgttgtttacaacatgcagaaaggtgaaatttggttcatcgaaggccgtaaaatccacagcgctgccaatttcagcaaagtgaaacgtatcaacctggtcatcgacttcgcgccggatattccgtttgaagaactgttcctgaattctgagaactatcaaccgaacctgatcccgaaaatctctcaacgtacccagctgaaagaagaagagctgggttatatcaaaggtctgtctaaaattatcaatgaaatgaactttgacgacatcctgtccattctgagcaaaattcacttctatcgcaacgtttcctccgaactggtttttggctggctggacgaaattgccacggcgtccaacaactataacattcagcgcaaagcgcaggaagtaaccgatctgctgattcgcaaaggcccgattaataactaa

SEQ ID NO: 68 - protein, 276 aa, Artificial Sequence
  amino acid sequence of I58R mutant
MESKIIGKVNFEEHLLDKELKLIDTFEFNDSYSEYASGIWKTCMLWNRSGQKDDHLSREHDTYVKPTEYGKQLAYVNEIIANTFKKEHIKTVRLFMCINGLIIPHKDYLEFKKGFTRIHIPLKINEHALTSEEDVVYNMQKGEIWFIEGRKIHSAANFSKVKRINLVIDFAPDIPFEELFLNSENYQPNLIPKISQRTQLKEEELGYIKGLSKIINEMNFDDILSILSKIHFYRNVSSELVFGWLDEIATASNNYNIQRKAQEVTDLLIRKGPINN

SEQ ID NO: 69 - DNA, 831 bp, Artificial Sequence
  gene sequence of I58V mutant
atggaatccaagatcatcggtaaagtcaacttcgaggagcatctgctggataaagagctgaaactgatcgacactttcgagttcaacgacagctacagcgaatacgcttctggtatttggaagacttgcatgctgtggaaccgttctggtcagaaagatgaccatctgtctgttgaacatgatacctacgtgaaacctactgaatacggcaaacagctggcatacgtaaacgaaatcatcgctaacacctttaagaaagaacacatcaagacggtgcgtctgttcatgtgtatcaacggcctgatcatcccacacaaagactacctggaattcaagaaaggcttcacccgtatccacatcccgctgaaaatcaacgaacacgcactgacctctgaagaagatgttgtttacaacatgcagaaaggtgaaatttggttcatcgaaggccgtaaaatccacagcgctgccaatttcagcaaagtgaaacgtatcaacctggtcatcgacttcgcgccggatattccgtttgaagaactgttcctgaattctgagaactatcaaccgaacctgatcccgaaaatctctcaacgtacccagctgaaagaagaagagctgggttatatcaaaggtctgtctaaaattatcaatgaaatgaactttgacgacatcctgtccattctgagcaaaattcacttctatcgcaacgtttcctccgaactggtttttggctggctggacgaaattgccacggcgtccaacaactataacattcagcgcaaagcgcaggaagtaaccgatctgctgattcgcaaaggcccgattaataactaa

SEQ ID NO: 70 - protein, 276 aa, Artificial Sequence
  amino acid sequence of I58V mutant
MESKIIGKVNFEEHLLDKELKLIDTFEFNDSYSEYASGIWKTCMLWNRSGQKDDHLSVEHDTYVKPTEYGKQLAYVNEIIANTFKKEHIKTVRLFMCINGLIIPHKDYLEFKKGFTRIHIPLKINEHALTSEEDVVYNMQKGEIWFIEGRKIHSAANFSKVKRINLVIDFAPDIPFEELFLNSENYQPNLIPKISQRTQLKEEELGYIKGLSKIINEMNFDDILSILSKIHFYRNVSSELVFGWLDEIATASNNYNIQRKAQEVTDLLIRKGPINN

SEQ ID NO: 71 - DNA, 831 bp, Artificial Sequence
  gene sequence of I58S mutant
atggaatccaagatcatcggtaaagtcaacttcgaggagcatctgctggataaagagctgaaactgatcgacactttcgagttcaacgacagctacagcgaatacgcttctggtatttggaagacttgcatgctgtggaaccgttctggtcagaaagatgaccatctgtctagcgaacatgatacctacgtgaaacctactgaatacggcaaacagctggcatacgtaaacgaaatcatcgctaacacctttaagaaagaacacatcaagacggtgcgtctgttcatgtgtatcaacggcctgatcatcccacacaaagactacctggaattcaagaaaggcttcacccgtatccacatcccgctgaaaatcaacgaacacgcactgacctctgaagaagatgttgtttacaacatgcagaaaggtgaaatttggttcatcgaaggccgtaaaatccacagcgctgccaatttcagcaaagtgaaacgtatcaacctggtcatcgacttcgcgccggatattccgtttgaagaactgttcctgaattctgagaactatcaaccgaacctgatcccgaaaatctctcaacgtacccagctgaaagaagaagagctgggttatatcaaaggtctgtctaaaattatcaatgaaatgaactttgacgacatcctgtccattctgagcaaaattcacttctatcgcaacgtttcctccgaactggtttttggctggctggacgaaattgccacggcgtccaacaactataacattcagcgcaaagcgcaggaagtaaccgatctgctgattcgcaaaggcccgattaataactaa

SEQ ID NO: 72 - protein, 276 aa, Artificial Sequence
  amino acid sequence of I58S mutant
MESKIIGKVNFEEHLLDKELKLIDTFEFNDSYSEYASGIWKTCMLWNRSGQKDDHLSSEHDTYVKPTEYGKQLAYVNEIIANTFKKEHIKTVRLFMCINGLIIPHKDYLEFKKGFTRIHIPLKINEHALTSEEDVVYNMQKGEIWFIEGRKIHSAANFSKVKRINLVIDFAPDIPFEELFLNSENYQPNLIPKISQRTQLKEEELGYIKGLSKIINEMNFDDILSILSKIHFYRNVSSELVFGWLDEIATASNNYNIQRKAQEVTDLLIRKGPINN

SEQ ID NO: 73 - DNA, 831 bp, Artificial Sequence
  gene sequence of I58C mutant
atggaatccaagatcatcggtaaagtcaacttcgaggagcatctgctggataaagagctgaaactgatcgacactttcgagttcaacgacagctacagcgaatacgcttctggtatttggaagacttgcatgctgtggaaccgttctggtcagaaagatgaccatctgtcttgtgaacatgatacctacgtgaaacctactgaatacggcaaacagctggcatacgtaaacgaaatcatcgctaacacctttaagaaagaacacatcaagacggtgcgtctgttcatgtgtatcaacggcctgatcatcccacacaaagactacctggaattcaagaaaggcttcacccgtatccacatcccgctgaaaatcaacgaacacgcactgacctctgaagaagatgttgtttacaacatgcagaaaggtgaaatttggttcatcgaaggccgtaaaatccacagcgctgccaatttcagcaaagtgaaacgtatcaacctggtcatcgacttcgcgccggatattccgtttgaagaactgttcctgaattctgagaactatcaaccgaacctgatcccgaaaatctctcaacgtacccagctgaaagaagaagagctgggttatatcaaaggtctgtctaaaattatcaatgaaatgaactttgacgacatcctgtccattctgagcaaaattcacttctatcgcaacgtttcctccgaactggtttttggctggctggacgaaattgccacggcgtccaacaactataacattcagcgcaaagcgcaggaagtaaccgatctgctgattcgcaaaggcccgattaataactaa

SEQ ID NO: 74 - protein, 276 aa, Artificial Sequence
  amino acid sequence of I58C mutant
MESKIIGKVNFEEHLLDKELKLIDTFEFNDSYSEYASGIWKTCMLWNRSGQKDDHLSCEHDTYVKPTEYGKQLAYVNEIIANTFKKEHIKTVRLFMCINGLIIPHKDYLEFKKGFTRIHIPLKINEHALTSEEDVVYNMQKGEIWFIEGRKIHSAANFSKVKRINLVIDFAPDIPFEELFLNSENYQPNLIPKISQRTQLKEEELGYIKGLSKIINEMNFDDILSILSKIHFYRNVSSELVFGWLDEIATASNNYNIQRKAQEVTDLLIRKGPINN

SEQ ID NO: 75 - DNA, 831 bp, Artificial Sequence
  gene sequence of K86P mutant
atggaatccaagatcatcggtaaagtcaacttcgaggagcatctgctggataaagagctgaaactgatcgacactttcgagttcaacgacagctacagcgaatacgcttctggtatttggaagacttgcatgctgtggaaccgttctggtcagaaagatgaccatctgtctattgaacatgatacctacgtgaaacctactgaatacggcaaacagctggcatacgtaaacgaaatcatcgctaacacctttaagccggaacacatcaagacggtgcgtctgttcatgtgtatcaacggcctgatcatcccacacaaagactacctggaattcaagaaaggcttcacccgtatccacatcccgctgaaaatcaacgaacacgcactgacctctgaagaagatgttgtttacaacatgcagaaaggtgaaatttggttcatcgaaggccgtaaaatccacagcgctgccaatttcagcaaagtgaaacgtatcaacctggtcatcgacttcgcgccggatattccgtttgaagaactgttcctgaattctgagaactatcaaccgaacctgatcccgaaaatctctcaacgtacccagctgaaagaagaagagctgggttatatcaaaggtctgtctaaaattatcaatgaaatgaactttgacgacatcctgtccattctgagcaaaattcacttctatcgcaacgtttcctccgaactggtttttggctggctggacgaaattgccacggcgtccaacaactataacattcagcgcaaagcgcaggaagtaaccgatctgctgattcgcaaaggcccgattaataactaa

SEQ ID NO: 76 - protein, 276 aa, Artificial Sequence
  amino acid sequence of K86P mutant
MESKIIGKVNFEEHLLDKELKLIDTFEFNDSYSEYASGIWKTCMLWNRSGQKDDHLSIEHDTYVKPTEYGKQLAYVNEIIANTFKPEHIKTVRLFMCINGLIIPHKDYLEFKKGFTRIHIPLKINEHALTSEEDVVYNMQKGEIWFIEGRKIHSAANFSKVKRINLVIDFAPDIPFEELFLNSENYQPNLIPKISQRTQLKEEELGYIKGLSKIINEMNFDDILSILSKIHFYRNVSSELVFGWLDEIATASNNYNIQRKAQEVTDLLIRKGPINN

SEQ ID NO: 77 - DNA, 831 bp, Artificial Sequence
  gene sequence of T91A mutant
atggaatccaagatcatcggtaaagtcaacttcgaggagcatctgctggataaagagctgaaactgatcgacactttcgagttcaacgacagctacagcgaatacgcttctggtatttggaagacttgcatgctgtggaaccgttctggtcagaaagatgaccatctgtctattgaacatgatacctacgtgaaacctactgaatacggcaaacagctggcatacgtaaacgaaatcatcgctaacacctttaagaaagaacacatcaaggcagtgcgtctgttcatgtgtatcaacggcctgatcatcccacacaaagactacctggaattcaagaaaggcttcacccgtatccacatcccgctgaaaatcaacgaacacgcactgacctctgaagaagatgttgtttacaacatgcagaaaggtgaaatttggttcatcgaaggccgtaaaatccacagcgctgccaatttcagcaaagtgaaacgtatcaacctggtcatcgacttcgcgccggatattccgtttgaagaactgttcctgaattctgagaactatcaaccgaacctgatcccgaaaatctctcaacgtacccagctgaaagaagaagagctgggttatatcaaaggtctgtctaaaattatcaatgaaatgaactttgacgacatcctgtccattctgagcaaaattcacttctatcgcaacgtttcctccgaactggtttttggctggctggacgaaattgccacggcgtccaacaactataacattcagcgcaaagcgcaggaagtaaccgatctgctgattcgcaaaggcccgattaataactaa

SEQ ID NO: 78 - protein, 276 aa, Artificial Sequence
  amino acid sequence of T91A mutant
MESKIIGKVNFEEHLLDKELKLIDTFEFNDSYSEYASGIWKTCMLWNRSGQKDDHLSIEHDTYVKPTEYGKQLAYVNEIIANTFKKEHIKAVRLFMCINGLIIPHKDYLEFKKGFTRIHIPLKINEHALTSEEDVVYNMQKGEIWFIEGRKIHSAANFSKVKRINLVIDFAPDIPFEELFLNSENYQPNLIPKISQRTQLKEEELGYIKGLSKIINEMNFDDILSILSKIHFYRNVSSELVFGWLDEIATASNNYNIQRKAQEVTDLLIRKGPINN

SEQ ID NO: 79 - DNA, 831 bp, Artificial Sequence
  gene sequence of F95Y mutant
atggaatccaagatcatcggtaaagtcaacttcgaggagcatctgctggataaagagctgaaactgatcgacactttcgagttcaacgacagctacagcgaatacgcttctggtatttggaagacttgcatgctgtggaaccgttctggtcagaaagatgaccatctgtctattgaacatgatacctacgtgaaacctactgaatacggcaaacagctggcatacgtaaacgaaatcatcgctaacacctttaagaaagaacacatcaagacggtgcgtctgtatatgtgtatcaacggcctgatcatcccacacaaagactacctggaattcaagaaaggcttcacccgtatccacatcccgctgaaaatcaacgaacacgcactgacctctgaagaagatgttgtttacaacatgcagaaaggtgaaatttggttcatcgaaggccgtaaaatccacagcgctgccaatttcagcaaagtgaaacgtatcaacctggtcatcgacttcgcgccggatattccgtttgaagaactgttcctgaattctgagaactatcaaccgaacctgatcccgaaaatctctcaacgtacccagctgaaagaagaagagctgggttatatcaaaggtctgtctaaaattatcaatgaaatgaactttgacgacatcctgtccattctgagcaaaattcacttctatcgcaacgtttcctccgaactggtttttggctggctggacgaaattgccacggcgtccaacaactataacattcagcgcaaagcgcaggaagtaaccgatctgctgattcgcaaaggcccgattaataactaa

SEQ ID NO: 80 - protein, 276 aa, Artificial Sequence
  amino acid sequence of F95Y mutant
MESKIIGKVNFEEHLLDKELKLIDTFEFNDSYSEYASGIWKTCMLWNRSGQKDDHLSIEHDTYVKPTEYGKQLAYVNEIIANTFKKEHIKTVRLYMCINGLIIPHKDYLEFKKGFTRIHIPLKINEHALTSEEDVVYNMQKGEIWFIEGRKIHSAANFSKVKRINLVIDFAPDIPFEELFLNSENYQPNLIPKISQRTQLKEEELGYIKGLSKIINEMNFDDILSILSKIHFYRNVSSELVFGWLDEIATASNNYNIQRKAQEVTDLLIRKGPINN

SEQ ID NO: 81 - DNA, 831 bp, Artificial Sequence
  gene sequence of C97Y mutant
atggaatccaagatcatcggtaaagtcaacttcgaggagcatctgctggataaagagctgaaactgatcgacactttcgagttcaacgacagctacagcgaatacgcttctggtatttggaagacttgcatgctgtggaaccgttctggtcagaaagatgaccatctgtctattgaacatgatacctacgtgaaacctactgaatacggcaaacagctggcatacgtaaacgaaatcatcgctaacacctttaagaaagaacacatcaagacggtgcgtctgttcatgtatatcaacggcctgatcatcccacacaaagactacctggaattcaagaaaggcttcacccgtatccacatcccgctgaaaatcaacgaacacgcactgacctctgaagaagatgttgtttacaacatgcagaaaggtgaaatttggttcatcgaaggccgtaaaatccacagcgctgccaatttcagcaaagtgaaacgtatcaacctggtcatcgacttcgcgccggatattccgtttgaagaactgttcctgaattctgagaactatcaaccgaacctgatcccgaaaatctctcaacgtacccagctgaaagaagaagagctgggttatatcaaaggtctgtctaaaattatcaatgaaatgaactttgacgacatcctgtccattctgagcaaaattcacttctatcgcaacgtttcctccgaactggtttttggctggctggacgaaattgccacggcgtccaacaactataacattcagcgcaaagcgcaggaagtaaccgatctgctgattcgcaaaggcccgattaataactaa

SEQ ID NO: 82 - protein, 276 aa, Artificial Sequence
  amino acid sequence of C97Y mutant
MESKIIGKVNFEEHLLDKELKLIDTFEFNDSYSEYASGIWKTCMLWNRSGQKDDHLSIEHDTYVKPTEYGKQLAYVNEIIANTFKKEHIKTVRLFMYINGLIIPHKDYLEFKKGFTRIHIPLKINEHALTSEEDVVYNMQKGEIWFIEGRKIHSAANFSKVKRINLVIDFAPDIPFEELFLNSENYQPNLIPKISQRTQLKEEELGYIKGLSKIINEMNFDDILSILSKIHFYRNVSSELVFGWLDEIATASNNYNIQRKAQEVTDLLIRKGPINN

SEQ ID NO: 83 - DNA, 831 bp, Artificial Sequence
  gene sequence of I98V mutant
atggaatccaagatcatcggtaaagtcaacttcgaggagcatctgctggataaagagctgaaactgatcgacactttcgagttcaacgacagctacagcgaatacgcttctggtatttggaagacttgcatgctgtggaaccgttctggtcagaaagatgaccatctgtctattgaacatgatacctacgtgaaacctactgaatacggcaaacagctggcatacgtaaacgaaatcatcgctaacacctttaagaaagaacacatcaagacggtgcgtctgttcatgtgtgttaacggcctgatcatcccacacaaagactacctggaattcaagaaaggcttcacccgtatccacatcccgctgaaaatcaacgaacacgcactgacctctgaagaagatgttgtttacaacatgcagaaaggtgaaatttggttcatcgaaggccgtaaaatccacagcgctgccaatttcagcaaagtgaaacgtatcaacctggtcatcgacttcgcgccggatattccgtttgaagaactgttcctgaattctgagaactatcaaccgaacctgatcccgaaaatctctcaacgtacccagctgaaagaagaagagctgggttatatcaaaggtctgtctaaaattatcaatgaaatgaactttgacgacatcctgtccattctgagcaaaattcacttctatcgcaacgtttcctccgaactggtttttggctggctggacgaaattgccacggcgtccaacaactataacattcagcgcaaagcgcaggaagtaaccgatctgctgattcgcaaaggcccgattaataactaa

SEQ ID NO: 84 - protein, 276 aa, Artificial Sequence
  amino acid sequence of I98V mutant
MESKIIGKVNFEEHLLDKELKLIDTFEFNDSYSEYASGIWKTCMLWNRSGQKDDHLSIEHDTYVKPTEYGKQLAYVNEIIANTFKKEHIKTVRLFMCVNGLIIPHKDYLEFKKGFTRIHIPLKINEHALTSEEDVVYNMQKGEIWFIEGRKIHSAANFSKVKRINLVIDFAPDIPFEELFLNSENYQPNLIPKISQRTQLKEEELGYIKGLSKIINEMNFDDILSILSKIHFYRNVSSELVFGWLDEIATASNNYNIQRKAQEVTDLLIRKGPINN

SEQ ID NO: 85 - DNA, 831 bp, Artificial Sequence
  gene sequence of K106V mutant
atggaatccaagatcatcggtaaagtcaacttcgaggagcatctgctggataaagagctgaaactgatcgacactttcgagttcaacgacagctacagcgaatacgcttctggtatttggaagacttgcatgctgtggaaccgttctggtcagaaagatgaccatctgtctattgaacatgatacctacgtgaaacctactgaatacggcaaacagctggcatacgtaaacgaaatcatcgctaacacctttaagaaagaacacatcaagacggtgcgtctgttcatgtgtatcaacggcctgatcatcccacacgttgactacctggaattcaagaaaggcttcacccgtatccacatcccgctgaaaatcaacgaacacgcactgacctctgaagaagatgttgtttacaacatgcagaaaggtgaaatttggttcatcgaaggccgtaaaatccacagcgctgccaatttcagcaaagtgaaacgtatcaacctggtcatcgacttcgcgccggatattccgtttgaagaactgttcctgaattctgagaactatcaaccgaacctgatcccgaaaatctctcaacgtacccagctgaaagaagaagagctgggttatatcaaaggtctgtctaaaattatcaatgaaatgaactttgacgacatcctgtccattctgagcaaaattcacttctatcgcaacgtttcctccgaactggtttttggctggctggacgaaattgccacggcgtccaacaactataacattcagcgcaaagcgcaggaagtaaccgatctgctgattcgcaaaggcccgattaataactaa

SEQ ID NO: 86 - protein, 276 aa, Artificial Sequence
  amino acid sequence of K106V mutant
MESKIIGKVNFEEHLLDKELKLIDTFEFNDSYSEYASGIWKTCMLWNRSGQKDDHLSIEHDTYVKPTEYGKQLAYVNEIIANTFKKEHIKTVRLFMCINGLIIPHVDYLEFKKGFTRIHIPLKINEHALTSEEDVVYNMQKGEIWFIEGRKIHSAANFSKVKRINLVIDFAPDIPFEELFLNSENYQPNLIPKISQRTQLKEEELGYIKGLSKIINEMNFDDILSILSKIHFYRNVSSELVFGWLDEIATASNNYNIQRKAQEVTDLLIRKGPINN

SEQ ID NO: 87 - DNA, 831 bp, Artificial Sequence
  gene sequence of K106T mutant
atggaatccaagatcatcggtaaagtcaacttcgaggagcatctgctggataaagagctgaaactgatcgacactttcgagttcaacgacagctacagcgaatacgcttctggtatttggaagacttgcatgctgtggaaccgttctggtcagaaagatgaccatctgtctattgaacatgatacctacgtgaaacctactgaatacggcaaacagctggcatacgtaaacgaaatcatcgctaacacctttaagaaagaacacatcaagacggtgcgtctgttcatgtgtatcaacggcctgatcatcccacacaccgactacctggaattcaagaaaggcttcacccgtatccacatcccgctgaaaatcaacgaacacgcactgacctctgaagaagatgttgtttacaacatgcagaaaggtgaaatttggttcatcgaaggccgtaaaatccacagcgctgccaatttcagcaaagtgaaacgtatcaacctggtcatcgacttcgcgccggatattccgtttgaagaactgttcctgaattctgagaactatcaaccgaacctgatcccgaaaatctctcaacgtacccagctgaaagaagaagagctgggttatatcaaaggtctgtctaaaattatcaatgaaatgaactttgacgacatcctgtccattctgagcaaaattcacttctatcgcaacgtttcctccgaactggtttttggctggctggacgaaattgccacggcgtccaacaactataacattcagcgcaaagcgcaggaagtaaccgatctgctgattcgcaaaggcccgattaataactaa

SEQ ID NO: 88 - protein, 276 aa, Artificial Sequence
  amino acid sequence of K106T mutant
MESKIIGKVNFEEHLLDKELKLIDTFEFNDSYSEYASGIWKTCMLWNRSGQKDDHLSIEHDTYVKPTEYGKQLAYVNEIIANTFKKEHIKTVRLFMCINGLIIPHTDYLEFKKGFTRIHIPLKINEHALTSEEDVVYNMQKGEIWFIEGRKIHSAANFSKVKRINLVIDFAPDIPFEELFLNSENYQPNLIPKISQRTQLKEEELGYIKGLSKIINEMNFDDILSILSKIHFYRNVSSELVFGWLDEIATASNNYNIQRKAQEVTDLLIRKGPINN

SEQ ID NO: 89 - DNA, 831 bp, Artificial Sequence
  gene sequence of K106Q mutant
atggaatccaagatcatcggtaaagtcaacttcgaggagcatctgctggataaagagctgaaactgatcgacactttcgagttcaacgacagctacagcgaatacgcttctggtatttggaagacttgcatgctgtggaaccgttctggtcagaaagatgaccatctgtctattgaacatgatacctacgtgaaacctactgaatacggcaaacagctggcatacgtaaacgaaatcatcgctaacacctttaagaaagaacacatcaagacggtgcgtctgttcatgtgtatcaacggcctgatcatcccacaccaggactacctggaattcaagaaaggcttcacccgtatccacatcccgctgaaaatcaacgaacacgcactgacctctgaagaagatgttgtttacaacatgcagaaaggtgaaatttggttcatcgaaggccgtaaaatccacagcgctgccaatttcagcaaagtgaaacgtatcaacctggtcatcgacttcgcgccggatattccgtttgaagaactgttcctgaattctgagaactatcaaccgaacctgatcccgaaaatctctcaacgtacccagctgaaagaagaagagctgggttatatcaaaggtctgtctaaaattatcaatgaaatgaactttgacgacatcctgtccattctgagcaaaattcacttctatcgcaacgtttcctccgaactggtttttggctggctggacgaaattgccacggcgtccaacaactataacattcagcgcaaagcgcaggaagtaaccgatctgctgattcgcaaaggcccgattaataactaa

SEQ ID NO: 90 - protein, 276 aa, Artificial Sequence
  amino acid sequence of K106Q mutant
MESKIIGKVNFEEHLLDKELKLIDTFEFNDSYSEYASGIWKTCMLWNRSGQKDDHLSIEHDTYVKPTEYGKQLAYVNEIIANTFKKEHIKTVRLFMCINGLIIPHQDYLEFKKGFTRIHIPLKINEHALTSEEDVVYNMQKGEIWFIEGRKIHSAANFSKVKRINLVIDFAPDIPFEELFLNSENYQPNLIPKISQRTQLKEEELGYIKGLSKIINEMNFDDILSILSKIHFYRNVSSELVFGWLDEIATASNNYNIQRKAQEVTDLLIRKGPINN

SEQ ID NO: 91 - DNA, 831 bp, Artificial Sequence
  gene sequence of F111S mutant
atggaatccaagatcatcggtaaagtcaacttcgaggagcatctgctggataaagagctgaaactgatcgacactttcgagttcaacgacagctacagcgaatacgcttctggtatttggaagacttgcatgctgtggaaccgttctggtcagaaagatgaccatctgtctattgaacatgatacctacgtgaaacctactgaatacggcaaacagctggcatacgtaaacgaaatcatcgctaacacctttaagaaagaacacatcaagacggtgcgtctgttcatgtgtatcaacggcctgatcatcccacacaaagactacctggaaagcaagaaaggcttcacccgtatccacatcccgctgaaaatcaacgaacacgcactgacctctgaagaagatgttgtttacaacatgcagaaaggtgaaatttggttcatcgaaggccgtaaaatccacagcgctgccaatttcagcaaagtgaaacgtatcaacctggtcatcgacttcgcgccggatattccgtttgaagaactgttcctgaattctgagaactatcaaccgaacctgatcccgaaaatctctcaacgtacccagctgaaagaagaagagctgggttatatcaaaggtctgtctaaaattatcaatgaaatgaactttgacgacatcctgtccattctgagcaaaattcacttctatcgcaacgtttcctccgaactggtttttggctggctggacgaaattgccacggcgtccaacaactataacattcagcgcaaagcgcaggaagtaaccgatctgctgattcgcaaaggcccgattaataactaa

SEQ ID NO: 92 - protein, 276 aa, Artificial Sequence
  amino acid sequence of F111S mutant
MESKIIGKVNFEEHLLDKELKLIDTFEFNDSYSEYASGIWKTCMLWNRSGQKDDHLSIEHDTYVKPTEYGKQLAYVNEIIANTFKKEHIKTVRLFMCINGLIIPHKDYLESKKGFTRIHIPLKINEHALTSEEDVVYNMQKGEIWFIEGRKIHSAANFSKVKRINLVIDFAPDIPFEELFLNSENYQPNLIPKISQRTQLKEEELGYIKGLSKIINEMNFDDILSILSKIHFYRNVSSELVFGWLDEIATASNNYNIQRKAQEVTDLLIRKGPINN

SEQ ID NO: 93 - DNA, 831 bp, Artificial Sequence
  gene sequence of K112E mutant
atggaatccaagatcatcggtaaagtcaacttcgaggagcatctgctggataaagagctgaaactgatcgacactttcgagttcaacgacagctacagcgaatacgcttctggtatttggaagacttgcatgctgtggaaccgttctggtcagaaagatgaccatctgtctattgaacatgatacctacgtgaaacctactgaatacggcaaacagctggcatacgtaaacgaaatcatcgctaacacctttaagaaagaacacatcaagacggtgcgtctgttcatgtgtatcaacggcctgatcatcccacacaaagactacctggaattcgaaaaaggcttcacccgtatccacatcccgctgaaaatcaacgaacacgcactgacctctgaagaagatgttgtttacaacatgcagaaaggtgaaatttggttcatcgaaggccgtaaaatccacagcgctgccaatttcagcaaagtgaaacgtatcaacctggtcatcgacttcgcgccggatattccgtttgaagaactgttcctgaattctgagaactatcaaccgaacctgatcccgaaaatctctcaacgtacccagctgaaagaagaagagctgggttatatcaaaggtctgtctaaaattatcaatgaaatgaactttgacgacatcctgtccattctgagcaaaattcacttctatcgcaacgtttcctccgaactggtttttggctggctggacgaaattgccacggcgtccaacaactataacattcagcgcaaagcgcaggaagtaaccgatctgctgattcgcaaaggcccgattaataactaa

SEQ ID NO: 94 - protein, 276 aa, Artificial Sequence
  amino acid sequence of K112E mutant
MESKIIGKVNFEEHLLDKELKLIDTFEFNDSYSEYASGIWKTCMLWNRSGQKDDHLSIEHDTYVKPTEYGKQLAYVNEIIANTFKKEHIKTVRLFMCINGLIIPHKDYLEFEKGFTRIHIPLKINEHALTSEEDVVYNMQKGEIWFIEGRKIHSAANFSKVKRINLVIDFAPDIPFEELFLNSENYQPNLIPKISQRTQLKEEELGYIKGLSKIINEMNFDDILSILSKIHFYRNVSSELVFGWLDEIATASNNYNIQRKAQEVTDLLIRKGPINN

SEQ ID NO: 95 - DNA, 831 bp, Artificial Sequence
  gene sequence of I118F mutant
atggaatccaagatcatcggtaaagtcaacttcgaggagcatctgctggataaagagctgaaactgatcgacactttcgagttcaacgacagctacagcgaatacgcttctggtatttggaagacttgcatgctgtggaaccgttctggtcagaaagatgaccatctgtctattgaacatgatacctacgtgaaacctactgaatacggcaaacagctggcatacgtaaacgaaatcatcgctaacacctttaagaaagaacacatcaagacggtgcgtctgttcatgtgtatcaacggcctgatcatcccacacaaagactacctggaattcaagaaaggcttcacccgttttcacatcccgctgaaaatcaacgaacacgcactgacctctgaagaagatgttgtttacaacatgcagaaaggtgaaatttggttcatcgaaggccgtaaaatccacagcgctgccaatttcagcaaagtgaaacgtatcaacctggtcatcgacttcgcgccggatattccgtttgaagaactgttcctgaattctgagaactatcaaccgaacctgatcccgaaaatctctcaacgtacccagctgaaagaagaagagctgggttatatcaaaggtctgtctaaaattatcaatgaaatgaactttgacgacatcctgtccattctgagcaaaattcacttctatcgcaacgtttcctccgaactggtttttggctggctggacgaaattgccacggcgtccaacaactataacattcagcgcaaagcgcaggaagtaaccgatctgctgattcgcaaaggcccgattaataactaa

SEQ ID NO: 96 - protein, 276 aa, Artificial Sequence
  amino acid sequence of I118F mutant
MESKIIGKVNFEEHLLDKELKLIDTFEFNDSYSEYASGIWKTCMLWNRSGQKDDHLSIEHDTYVKPTEYGKQLAYVNEIIANTFKKEHIKTVRLFMCINGLIIPHKDYLEFKKGFTRFHIPLKINEHALTSEEDVVYNMQKGEIWFIEGRKIHSAANFSKVKRINLVIDFAPDIPFEELFLNSENYQPNLIPKISQRTQLKEEELGYIKGLSKIINEMNFDDILSILSKIHFYRNVSSELVFGWLDEIATASNNYNIQRKAQEVTDLLIRKGPINN

SEQ ID NO: 97 - DNA, 831 bp, Artificial Sequence
  gene sequence of H119R mutant
atggaatccaagatcatcggtaaagtcaacttcgaggagcatctgctggataaagagctgaaactgatcgacactttcgagttcaacgacagctacagcgaatacgcttctggtatttggaagacttgcatgctgtggaaccgttctggtcagaaagatgaccatctgtctattgaacatgatacctacgtgaaacctactgaatacggcaaacagctggcatacgtaaacgaaatcatcgctaacacctttaagaaagaacacatcaagacggtgcgtctgttcatgtgtatcaacggcctgatcatcccacacaaagactacctggaattcaagaaaggcttcacccgtatccgtatcccgctgaaaatcaacgaacacgcactgacctctgaagaagatgttgtttacaacatgcagaaaggtgaaatttggttcatcgaaggccgtaaaatccacagcgctgccaatttcagcaaagtgaaacgtatcaacctggtcatcgacttcgcgccggatattccgtttgaagaactgttcctgaattctgagaactatcaaccgaacctgatcccgaaaatctctcaacgtacccagctgaaagaagaagagctgggttatatcaaaggtctgtctaaaattatcaatgaaatgaactttgacgacatcctgtccattctgagcaaaattcacttctatcgcaacgtttcctccgaactggtttttggctggctggacgaaattgccacggcgtccaacaactataacattcagcgcaaagcgcaggaagtaaccgatctgctgattcgcaaaggcccgattaataactaa

SEQ ID NO: 98 - protein, 276 aa, Artificial Sequence
  amino acid sequence of H119R mutant
MESKIIGKVNFEEHLLDKELKLIDTFEFNDSYSEYASGIWKTCMLWNRSGQKDDHLSIEHDTYVKPTEYGKQLAYVNEIIANTFKKEHIKTVRLFMCINGLIIPHKDYLEFKKGFTRIRIPLKINEHALTSEEDVVYNMQKGEIWFIEGRKIHSAANFSKVKRINLVIDFAPDIPFEELFLNSENYQPNLIPKISQRTQLKEEELGYIKGLSKIINEMNFDDILSILSKIHFYRNVSSELVFGWLDEIATASNNYNIQRKAQEVTDLLIRKGPINN

SEQ ID NO: 99 - DNA, 831 bp, Artificial Sequence
  gene sequence of H119F mutant
atggaatccaagatcatcggtaaagtcaacttcgaggagcatctgctggataaagagctgaaactgatcgacactttcgagttcaacgacagctacagcgaatacgcttctggtatttggaagacttgcatgctgtggaaccgttctggtcagaaagatgaccatctgtctattgaacatgatacctacgtgaaacctactgaatacggcaaacagctggcatacgtaaacgaaatcatcgctaacacctttaagaaagaacacatcaagacggtgcgtctgttcatgtgtatcaacggcctgatcatcccacacaaagactacctggaattcaagaaaggcttcacccgtatctttatcccgctgaaaatcaacgaacacgcactgacctctgaagaagatgttgtttacaacatgcagaaaggtgaaatttggttcatcgaaggccgtaaaatccacagcgctgccaatttcagcaaagtgaaacgtatcaacctggtcatcgacttcgcgccggatattccgtttgaagaactgttcctgaattctgagaactatcaaccgaacctgatcccgaaaatctctcaacgtacccagctgaaagaagaagagctgggttatatcaaaggtctgtctaaaattatcaatgaaatgaactttgacgacatcctgtccattctgagcaaaattcacttctatcgcaacgtttcctccgaactggtttttggctggctggacgaaattgccacggcgtccaacaactataacattcagcgcaaagcgcaggaagtaaccgatctgctgattcgcaaaggcccgattaataactaa

SEQ ID NO: 100 - protein, 276 aa, Artificial Sequence
  amino acid sequence of H119F mutant
MESKIIGKVNFEEHLLDKELKLIDTFEFNDSYSEYASGIWKTCMLWNRSGQKDDHLSIEHDTYVKPTEYGKQLAYVNEIIANTFKKEHIKTVRLFMCINGLIIPHKDYLEFKKGFTRIFIPLKINEHALTSEEDVVYNMQKGEIWFIEGRKIHSAANFSKVKRINLVIDFAPDIPFEELFLNSENYQPNLIPKISQRTQLKEEELGYIKGLSKIINEMNFDDILSILSKIHFYRNVSSELVFGWLDEIATASNNYNIQRKAQEVTDLLIRKGPINN

SEQ ID NO: 101 - DNA, 831 bp, Artificial Sequence
  gene sequence of I120V mutant
atggaatccaagatcatcggtaaagtcaacttcgaggagcatctgctggataaagagctgaaactgatcgacactttcgagttcaacgacagctacagcgaatacgcttctggtatttggaagacttgcatgctgtggaaccgttctggtcagaaagatgaccatctgtctattgaacatgatacctacgtgaaacctactgaatacggcaaacagctggcatacgtaaacgaaatcatcgctaacacctttaagaaagaacacatcaagacggtgcgtctgttcatgtgtatcaacggcctgatcatcccacacaaagactacctggaattcaagaaaggcttcacccgtatccacgttccgctgaaaatcaacgaacacgcactgacctctgaagaagatgttgtttacaacatgcagaaaggtgaaatttggttcatcgaaggccgtaaaatccacagcgctgccaatttcagcaaagtgaaacgtatcaacctggtcatcgacttcgcgccggatattccgtttgaagaactgttcctgaattctgagaactatcaaccgaacctgatcccgaaaatctctcaacgtacccagctgaaagaagaagagctgggttatatcaaaggtctgtctaaaattatcaatgaaatgaactttgacgacatcctgtccattctgagcaaaattcacttctatcgcaacgtttcctccgaactggtttttggctggctggacgaaattgccacggcgtccaacaactataacattcagcgcaaagcgcaggaagtaaccgatctgctgattcgcaaaggcccgattaataactaa

SEQ ID NO: 102 - protein, 276 aa, Artificial Sequence
  amino acid sequence of I120V mutant
MESKIIGKVNFEEHLLDKELKLIDTFEFNDSYSEYASGIWKTCMLWNRSGQKDDHLSIEHDTYVKPTEYGKQLAYVNEIIANTFKKEHIKTVRLFMCINGLIIPHKDYLEFKKGFTRIHVPLKINEHALTSEEDVVYNMQKGEIWFIEGRKIHSAANFSKVKRINLVIDFAPDIPFEELFLNSENYQPNLIPKISQRTQLKEEELGYIKGLSKIINEMNFDDILSILSKIHFYRNVSSELVFGWLDEIATASNNYNIQRKAQEVTDLLIRKGPINN

SEQ ID NO: 103 - DNA, 831 bp, Artificial Sequence
  gene sequence of K123D mutant
atggaatccaagatcatcggtaaagtcaacttcgaggagcatctgctggataaagagctgaaactgatcgacactttcgagttcaacgacagctacagcgaatacgcttctggtatttggaagacttgcatgctgtggaaccgttctggtcagaaagatgaccatctgtctattgaacatgatacctacgtgaaacctactgaatacggcaaacagctggcatacgtaaacgaaatcatcgctaacacctttaagaaagaacacatcaagacggtgcgtctgttcatgtgtatcaacggcctgatcatcccacacaaagactacctggaattcaagaaaggcttcacccgtatccacatcccgctggatatcaacgaacacgcactgacctctgaagaagatgttgtttacaacatgcagaaaggtgaaatttggttcatcgaaggccgtaaaatccacagcgctgccaatttcagcaaagtgaaacgtatcaacctggtcatcgacttcgcgccggatattccgtttgaagaactgttcctgaattctgagaactatcaaccgaacctgatcccgaaaatctctcaacgtacccagctgaaagaagaagagctgggttatatcaaaggtctgtctaaaattatcaatgaaatgaactttgacgacatcctgtccattctgagcaaaattcacttctatcgcaacgtttcctccgaactggtttttggctggctggacgaaattgccacggcgtccaacaactataacattcagcgcaaagcgcaggaagtaaccgatctgctgattcgcaaaggcccgattaataactaa

SEQ ID NO: 104 - protein, 276 aa, Artificial Sequence
  amino acid sequence of K123D mutant
MESKIIGKVNFEEHLLDKELKLIDTFEFNDSYSEYASGIWKTCMLWNRSGQKDDHLSIEHDTYVKPTEYGKQLAYVNEIIANTFKKEHIKTVRLFMCINGLIIPHKDYLEFKKGFTRIHIPLDINEHALTSEEDVVYNMQKGEIWFIEGRKIHSAANFSKVKRINLVIDFAPDIPFEELFLNSENYQPNLIPKISQRTQLKEEELGYIKGLSKIINEMNFDDILSILSKIHFYRNVSSELVFGWLDEIATASNNYNIQRKAQEVTDLLIRKGPINN

SEQ ID NO: 105 - DNA, 831 bp, Artificial Sequence
  gene sequence of K123N mutant
atggaatccaagatcatcggtaaagtcaacttcgaggagcatctgctggataaagagctgaaactgatcgacactttcgagttcaacgacagctacagcgaatacgcttctggtatttggaagacttgcatgctgtggaaccgttctggtcagaaagatgaccatctgtctattgaacatgatacctacgtgaaacctactgaatacggcaaacagctggcatacgtaaacgaaatcatcgctaacacctttaagaaagaacacatcaagacggtgcgtctgttcatgtgtatcaacggcctgatcatcccacacaaagactacctggaattcaagaaaggcttcacccgtatccacatcccgctgaatatcaacgaacacgcactgacctctgaagaagatgttgtttacaacatgcagaaaggtgaaatttggttcatcgaaggccgtaaaatccacagcgctgccaatttcagcaaagtgaaacgtatcaacctggtcatcgacttcgcgccggatattccgtttgaagaactgttcctgaattctgagaactatcaaccgaacctgatcccgaaaatctctcaacgtacccagctgaaagaagaagagctgggttatatcaaaggtctgtctaaaattatcaatgaaatgaactttgacgacatcctgtccattctgagcaaaattcacttctatcgcaacgtttcctccgaactggtttttggctggctggacgaaattgccacggcgtccaacaactataacattcagcgcaaagcgcaggaagtaaccgatctgctgattcgcaaaggcccgattaataactaa

SEQ ID NO: 106 - protein, 276 aa, Artificial Sequence
  amino acid sequence of K123N mutant
MESKIIGKVNFEEHLLDKELKLIDTFEFNDSYSEYASGIWKTCMLWNRSGQKDDHLSIEHDTYVKPTEYGKQLAYVNEIIANTFKKEHIKTVRLFMCINGLIIPHKDYLEFKKGFTRIHIPLNINEHALTSEEDVVYNMQKGEIWFIEGRKIHSAANFSKVKRINLVIDFAPDIPFEELFLNSENYQPNLIPKISQRTQLKEEELGYIKGLSKIINEMNFDDILSILSKIHFYRNVSSELVFGWLDEIATASNNYNIQRKAQEVTDLLIRKGPINN

SEQ ID NO: 107 - DNA, 831 bp, Artificial Sequence
  gene sequence of K123Q mutant
atggaatccaagatcatcggtaaagtcaacttcgaggagcatctgctggataaagagctgaaactgatcgacactttcgagttcaacgacagctacagcgaatacgcttctggtatttggaagacttgcatgctgtggaaccgttctggtcagaaagatgaccatctgtctattgaacatgatacctacgtgaaacctactgaatacggcaaacagctggcatacgtaaacgaaatcatcgctaacacctttaagaaagaacacatcaagacggtgcgtctgttcatgtgtatcaacggcctgatcatcccacacaaagactacctggaattcaagaaaggcttcacccgtatccacatcccgctgcagatcaacgaacacgcactgacctctgaagaagatgttgtttacaacatgcagaaaggtgaaatttggttcatcgaaggccgtaaaatccacagcgctgccaatttcagcaaagtgaaacgtatcaacctggtcatcgacttcgcgccggatattccgtttgaagaactgttcctgaattctgagaactatcaaccgaacctgatcccgaaaatctctcaacgtacccagctgaaagaagaagagctgggttatatcaaaggtctgtctaaaattatcaatgaaatgaactttgacgacatcctgtccattctgagcaaaattcacttctatcgcaacgtttcctccgaactggtttttggctggctggacgaaattgccacggcgtccaacaactataacattcagcgcaaagcgcaggaagtaaccgatctgctgattcgcaaaggcccgattaataactaa

SEQ ID NO: 108 - protein, 276 aa, Artificial Sequence
  amino acid sequence of K123Q mutant
MESKIIGKVNFEEHLLDKELKLIDTFEFNDSYSEYASGIWKTCMLWNRSGQKDDHLSIEHDTYVKPTEYGKQLAYVNEIIANTFKKEHIKTVRLFMCINGLIIPHKDYLEFKKGFTRIHIPLQINEHALTSEEDVVYNMQKGEIWFIEGRKIHSAANFSKVKRINLVIDFAPDIPFEELFLNSENYQPNLIPKISQRTQLKEEELGYIKGLSKIINEMNFDDILSILSKIHFYRNVSSELVFGWLDEIATASNNYNIQRKAQEVTDLLIRKGPINN

SEQ ID NO: 109 - DNA, 831 bp, Artificial Sequence
  gene sequence of K123S mutant
atggaatccaagatcatcggtaaagtcaacttcgaggagcatctgctggataaagagctgaaactgatcgacactttcgagttcaacgacagctacagcgaatacgcttctggtatttggaagacttgcatgctgtggaaccgttctggtcagaaagatgaccatctgtctattgaacatgatacctacgtgaaacctactgaatacggcaaacagctggcatacgtaaacgaaatcatcgctaacacctttaagaaagaacacatcaagacggtgcgtctgttcatgtgtatcaacggcctgatcatcccacacaaagactacctggaattcaagaaaggcttcacccgtatccacatcccgctgagcatcaacgaacacgcactgacctctgaagaagatgttgtttacaacatgcagaaaggtgaaatttggttcatcgaaggccgtaaaatccacagcgctgccaatttcagcaaagtgaaacgtatcaacctggtcatcgacttcgcgccggatattccgtttgaagaactgttcctgaattctgagaactatcaaccgaacctgatcccgaaaatctctcaacgtacccagctgaaagaagaagagctgggttatatcaaaggtctgtctaaaattatcaatgaaatgaactttgacgacatcctgtccattctgagcaaaattcacttctatcgcaacgtttcctccgaactggtttttggctggctggacgaaattgccacggcgtccaacaactataacattcagcgcaaagcgcaggaagtaaccgatctgctgattcgcaaaggcccgattaataactaa

SEQ ID NO: 110 - protein, 276 aa, Artificial Sequence
  amino acid sequence of K123S mutant
MESKIIGKVNFEEHLLDKELKLIDTFEFNDSYSEYASGIWKTCMLWNRSGQKDDHLSIEHDTYVKPTEYGKQLAYVNEIIANTFKKEHIKTVRLFMCINGLIIPHKDYLEFKKGFTRIHIPLSINEHALTSEEDVVYNMQKGEIWFIEGRKIHSAANFSKVKRINLVIDFAPDIPFEELFLNSENYQPNLIPKISQRTQLKEEELGYIKGLSKIINEMNFDDILSILSKIHFYRNVSSELVFGWLDEIATASNNYNIQRKAQEVTDLLIRKGPINN

SEQ ID NO: 111 - DNA, 831 bp, Artificial Sequence
  gene sequence of K123I mutant
atggaatccaagatcatcggtaaagtcaacttcgaggagcatctgctggataaagagctgaaactgatcgacactttcgagttcaacgacagctacagcgaatacgcttctggtatttggaagacttgcatgctgtggaaccgttctggtcagaaagatgaccatctgtctattgaacatgatacctacgtgaaacctactgaatacggcaaacagctggcatacgtaaacgaaatcatcgctaacacctttaagaaagaacacatcaagacggtgcgtctgttcatgtgtatcaacggcctgatcatcccacacaaagactacctggaattcaagaaaggcttcacccgtatccacatcccgctgattatcaacgaacacgcactgacctctgaagaagatgttgtttacaacatgcagaaaggtgaaatttggttcatcgaaggccgtaaaatccacagcgctgccaatttcagcaaagtgaaacgtatcaacctggtcatcgacttcgcgccggatattccgtttgaagaactgttcctgaattctgagaactatcaaccgaacctgatcccgaaaatctctcaacgtacccagctgaaagaagaagagctgggttatatcaaaggtctgtctaaaattatcaatgaaatgaactttgacgacatcctgtccattctgagcaaaattcacttctatcgcaacgtttcctccgaactggtttttggctggctggacgaaattgccacggcgtccaacaactataacattcagcgcaaagcgcaggaagtaaccgatctgctgattcgcaaaggcccgattaataactaa

SEQ ID NO: 112 - protein, 276 aa, Artificial Sequence
  amino acid sequence of K123I mutant
MESKIIGKVNFEEHLLDKELKLIDTFEFNDSYSEYASGIWKTCMLWNRSGQKDDHLSIEHDTYVKPTEYGKQLAYVNEIIANTFKKEHIKTVRLFMCINGLIIPHKDYLEFKKGFTRIHIPLIINEHALTSEEDVVYNMQKGEIWFIEGRKIHSAANFSKVKRINLVIDFAPDIPFEELFLNSENYQPNLIPKISQRTQLKEEELGYIKGLSKIINEMNFDDILSILSKIHFYRNVSSELVFGWLDEIATASNNYNIQRKAQEVTDLLIRKGPINN

SEQ ID NO: 113 - DNA, 831 bp, Artificial Sequence
  gene sequence of K123T mutant
atggaatccaagatcatcggtaaagtcaacttcgaggagcatctgctggataaagagctgaaactgatcgacactttcgagttcaacgacagctacagcgaatacgcttctggtatttggaagacttgcatgctgtggaaccgttctggtcagaaagatgaccatctgtctattgaacatgatacctacgtgaaacctactgaatacggcaaacagctggcatacgtaaacgaaatcatcgctaacacctttaagaaagaacacatcaagacggtgcgtctgttcatgtgtatcaacggcctgatcatcccacacaaagactacctggaattcaagaaaggcttcacccgtatccacatcccgctgaccatcaacgaacacgcactgacctctgaagaagatgttgtttacaacatgcagaaaggtgaaatttggttcatcgaaggccgtaaaatccacagcgctgccaatttcagcaaagtgaaacgtatcaacctggtcatcgacttcgcgccggatattccgtttgaagaactgttcctgaattctgagaactatcaaccgaacctgatcccgaaaatctctcaacgtacccagctgaaagaagaagagctgggttatatcaaaggtctgtctaaaattatcaatgaaatgaactttgacgacatcctgtccattctgagcaaaattcacttctatcgcaacgtttcctccgaactggtttttggctggctggacgaaattgccacggcgtccaacaactataacattcagcgcaaagcgcaggaagtaaccgatctgctgattcgcaaaggcccgattaataactaa

SEQ ID NO: 114 - protein, 276 aa, Artificial Sequence
  amino acid sequence of K123T mutant
MESKIIGKVNFEEHLLDKELKLIDTFEFNDSYSEYASGIWKTCMLWNRSGQKDDHLSIEHDTYVKPTEYGKQLAYVNEIIANTFKKEHIKTVRLFMCINGLIIPHKDYLEFKKGFTRIHIPLTINEHALTSEEDVVYNMQKGEIWFIEGRKIHSAANFSKVKRINLVIDFAPDIPFEELFLNSENYQPNLIPKISQRTQLKEEELGYIKGLSKIINEMNFDDILSILSKIHFYRNVSSELVFGWLDEIATASNNYNIQRKAQEVTDLLIRKGPINN

SEQ ID NO: 115 - DNA, 831 bp, Artificial Sequence
  gene sequence of T130N mutant
atggaatccaagatcatcggtaaagtcaacttcgaggagcatctgctggataaagagctgaaactgatcgacactttcgagttcaacgacagctacagcgaatacgcttctggtatttggaagacttgcatgctgtggaaccgttctggtcagaaagatgaccatctgtctattgaacatgatacctacgtgaaacctactgaatacggcaaacagctggcatacgtaaacgaaatcatcgctaacacctttaagaaagaacacatcaagacggtgcgtctgttcatgtgtatcaacggcctgatcatcccacacaaagactacctggaattcaagaaaggcttcacccgtatccacatcccgctgaaaatcaacgaacacgcactgaattctgaagaagatgttgtttacaacatgcagaaaggtgaaatttggttcatcgaaggccgtaaaatccacagcgctgccaatttcagcaaagtgaaacgtatcaacctggtcatcgacttcgcgccggatattccgtttgaagaactgttcctgaattctgagaactatcaaccgaacctgatcccgaaaatctctcaacgtacccagctgaaagaagaagagctgggttatatcaaaggtctgtctaaaattatcaatgaaatgaactttgacgacatcctgtccattctgagcaaaattcacttctatcgcaacgtttcctccgaactggtttttggctggctggacgaaattgccacggcgtccaacaactataacattcagcgcaaagcgcaggaagtaaccgatctgctgattcgcaaaggcccgattaataactaa

SEQ ID NO: 116 - protein, 276 aa, Artificial Sequence
  amino acid sequence of T130N mutant
MESKIIGKVNFEEHLLDKELKLIDTFEFNDSYSEYASGIWKTCMLWNRSGQKDDHLSIEHDTYVKPTEYGKQLAYVNEIIANTFKKEHIKTVRLFMCINGLIIPHKDYLEFKKGFTRIHIPLKINEHALNSEEDVVYNMQKGEIWFIEGRKIHSAANFSKVKRINLVIDFAPDIPFEELFLNSENYQPNLIPKISQRTQLKEEELGYIKGLSKIINEMNFDDILSILSKIHFYRNVSSELVFGWLDEIATASNNYNIQRKAQEVTDLLIRKGPINN

SEQ ID NO: 117 - DNA, 831 bp, Artificial Sequence
  gene sequence of D134G mutant
atggaatccaagatcatcggtaaagtcaacttcgaggagcatctgctggataaagagctgaaactgatcgacactttcgagttcaacgacagctacagcgaatacgcttctggtatttggaagacttgcatgctgtggaaccgttctggtcagaaagatgaccatctgtctattgaacatgatacctacgtgaaacctactgaatacggcaaacagctggcatacgtaaacgaaatcatcgctaacacctttaagaaagaacacatcaagacggtgcgtctgttcatgtgtatcaacggcctgatcatcccacacaaagactacctggaattcaagaaaggcttcacccgtatccacatcccgctgaaaatcaacgaacacgcactgacctctgaagaaggtgttgtttacaacatgcagaaaggtgaaatttggttcatcgaaggccgtaaaatccacagcgctgccaatttcagcaaagtgaaacgtatcaacctggtcatcgacttcgcgccggatattccgtttgaagaactgttcctgaattctgagaactatcaaccgaacctgatcccgaaaatctctcaacgtacccagctgaaagaagaagagctgggttatatcaaaggtctgtctaaaattatcaatgaaatgaactttgacgacatcctgtccattctgagcaaaattcacttctatcgcaacgtttcctccgaactggtttttggctggctggacgaaattgccacggcgtccaacaactataacattcagcgcaaagcgcaggaagtaaccgatctgctgattcgcaaaggcccgattaataactaa

SEQ ID NO: 118 - protein, 276 aa, Artificial Sequence
  amino acid sequence of D134G mutant
MESKIIGKVNFEEHLLDKELKLIDTFEFNDSYSEYASGIWKTCMLWNRSGQKDDHLSIEHDTYVKPTEYGKQLAYVNEIIANTFKKEHIKTVRLFMCINGLIIPHKDYLEFKKGFTRIHIPLKINEHALTSEEGVVYNMQKGEIWFIEGRKIHSAANFSKVKRINLVIDFAPDIPFEELFLNSENYQPNLIPKISQRTQLKEEELGYIKGLSKIINEMNFDDILSILSKIHFYRNVSSELVFGWLDEIATASNNYNIQRKAQEVTDLLIRKGPINN

SEQ ID NO: 119 - DNA, 831 bp, Artificial Sequence
  gene sequence of V135K mutant
atggaatccaagatcatcggtaaagtcaacttcgaggagcatctgctggataaagagctgaaactgatcgacactttcgagttcaacgacagctacagcgaatacgcttctggtatttggaagacttgcatgctgtggaaccgttctggtcagaaagatgaccatctgtctattgaacatgatacctacgtgaaacctactgaatacggcaaacagctggcatacgtaaacgaaatcatcgctaacacctttaagaaagaacacatcaagacggtgcgtctgttcatgtgtatcaacggcctgatcatcccacacaaagactacctggaattcaagaaaggcttcacccgtatccacatcccgctgaaaatcaacgaacacgcactgacctctgaagaagataaagtttacaacatgcagaaaggtgaaatttggttcatcgaaggccgtaaaatccacagcgctgccaatttcagcaaagtgaaacgtatcaacctggtcatcgacttcgcgccggatattccgtttgaagaactgttcctgaattctgagaactatcaaccgaacctgatcccgaaaatctctcaacgtacccagctgaaagaagaagagctgggttatatcaaaggtctgtctaaaattatcaatgaaatgaactttgacgacatcctgtccattctgagcaaaattcacttctatcgcaacgtttcctccgaactggtttttggctggctggacgaaattgccacggcgtccaacaactataacattcagcgcaaagcgcaggaagtaaccgatctgctgattcgcaaaggcccgattaataactaa

SEQ ID NO: 120 - protein, 276 aa, Artificial Sequence
  amino acid sequence of V135K mutant
MESKIIGKVNFEEHLLDKELKLIDTFEFNDSYSEYASGIWKTCMLWNRSGQKDDHLSIEHDTYVKPTEYGKQLAYVNEIIANTFKKEHIKTVRLFMCINGLIIPHKDYLEFKKGFTRIHIPLKINEHALTSEEDKVYNMQKGEIWFIEGRKIHSAANFSKVKRINLVIDFAPDIPFEELFLNSENYQPNLIPKISQRTQLKEEELGYIKGLSKIINEMNFDDILSILSKIHFYRNVSSELVFGWLDEIATASNNYNIQRKAQEVTDLLIRKGPINN

SEQ ID NO: 121 - DNA, 831 bp, Artificial Sequence
  gene sequence of N165H mutant
atggaatccaagatcatcggtaaagtcaacttcgaggagcatctgctggataaagagctgaaactgatcgacactttcgagttcaacgacagctacagcgaatacgcttctggtatttggaagacttgcatgctgtggaaccgttctggtcagaaagatgaccatctgtctattgaacatgatacctacgtgaaacctactgaatacggcaaacagctggcatacgtaaacgaaatcatcgctaacacctttaagaaagaacacatcaagacggtgcgtctgttcatgtgtatcaacggcctgatcatcccacacaaagactacctggaattcaagaaaggcttcacccgtatccacatcccgctgaaaatcaacgaacacgcactgacctctgaagaagatgttgtttacaacatgcagaaaggtgaaatttggttcatcgaaggccgtaaaatccacagcgctgccaatttcagcaaagtgaaacgtatccatctggtcatcgacttcgcgccggatattccgtttgaagaactgttcctgaattctgagaactatcaaccgaacctgatcccgaaaatctctcaacgtacccagctgaaagaagaagagctgggttatatcaaaggtctgtctaaaattatcaatgaaatgaactttgacgacatcctgtccattctgagcaaaattcacttctatcgcaacgtttcctccgaactggtttttggctggctggacgaaattgccacggcgtccaacaactataacattcagcgcaaagcgcaggaagtaaccgatctgctgattcgcaaaggcccgattaataactaa

SEQ ID NO: 122 - protein, 276 aa, Artificial Sequence
  amino acid sequence of N165H mutant
MESKIIGKVNFEEHLLDKELKLIDTFEFNDSYSEYASGIWKTCMLWNRSGQKDDHLSIEHDTYVKPTEYGKQLAYVNEIIANTFKKEHIKTVRLFMCINGLIIPHKDYLEFKKGFTRIHIPLKINEHALTSEEDVVYNMQKGEIWFIEGRKIHSAANFSKVKRIHLVIDFAPDIPFEELFLNSENYQPNLIPKISQRTQLKEEELGYIKGLSKIINEMNFDDILSILSKIHFYRNVSSELVFGWLDEIATASNNYNIQRKAQEVTDLLIRKGPINN

SEQ ID NO: 123 - DNA, 831 bp, Artificial Sequence
  gene sequence of K209R mutant
atggaatccaagatcatcggtaaagtcaacttcgaggagcatctgctggataaagagctgaaactgatcgacactttcgagttcaacgacagctacagcgaatacgcttctggtatttggaagacttgcatgctgtggaaccgttctggtcagaaagatgaccatctgtctattgaacatgatacctacgtgaaacctactgaatacggcaaacagctggcatacgtaaacgaaatcatcgctaacacctttaagaaagaacacatcaagacggtgcgtctgttcatgtgtatcaacggcctgatcatcccacacaaagactacctggaattcaagaaaggcttcacccgtatccacatcccgctgaaaatcaacgaacacgcactgacctctgaagaagatgttgtttacaacatgcagaaaggtgaaatttggttcatcgaaggccgtaaaatccacagcgctgccaatttcagcaaagtgaaacgtatcaacctggtcatcgacttcgcgccggatattccgtttgaagaactgttcctgaattctgagaactatcaaccgaacctgatcccgaaaatctctcaacgtacccagctgaaagaagaagagctgggttatatccgtggtctgtctaaaattatcaatgaaatgaactttgacgacatcctgtccattctgagcaaaattcacttctatcgcaacgtttcctccgaactggtttttggctggctggacgaaattgccacggcgtccaacaactataacattcagcgcaaagcgcaggaagtaaccgatctgctgattcgcaaaggcccgattaataactaa

SEQ ID NO: 124 - protein, 276 aa, Artificial Sequence
  amino acid sequence of K209R mutant
MESKIIGKVNFEEHLLDKELKLIDTFEFNDSYSEYASGIWKTCMLWNRSGQKDDHLSIEHDTYVKPTEYGKQLAYVNEIIANTFKKEHIKTVRLFMCINGLIIPHKDYLEFKKGFTRIHIPLKINEHALTSEEDVVYNMQKGEIWFIEGRKIHSAANFSKVKRINLVIDFAPDIPFEELFLNSENYQPNLIPKISQRTQLKEEELGYIRGLSKIINEMNFDDILSILSKIHFYRNVSSELVFGWLDEIATASNNYNIQRKAQEVTDLLIRKGPINN

SEQ ID NO: 125 - DNA, 831 bp, Artificial Sequence
  gene sequence of I223V mutant
atggaatccaagatcatcggtaaagtcaacttcgaggagcatctgctggataaagagctgaaactgatcgacactttcgagttcaacgacagctacagcgaatacgcttctggtatttggaagacttgcatgctgtggaaccgttctggtcagaaagatgaccatctgtctattgaacatgatacctacgtgaaacctactgaatacggcaaacagctggcatacgtaaacgaaatcatcgctaacacctttaagaaagaacacatcaagacggtgcgtctgttcatgtgtatcaacggcctgatcatcccacacaaagactacctggaattcaagaaaggcttcacccgtatccacatcccgctgaaaatcaacgaacacgcactgacctctgaagaagatgttgtttacaacatgcagaaaggtgaaatttggttcatcgaaggccgtaaaatccacagcgctgccaatttcagcaaagtgaaacgtatcaacctggtcatcgacttcgcgccggatattccgtttgaagaactgttcctgaattctgagaactatcaaccgaacctgatcccgaaaatctctcaacgtacccagctgaaagaagaagagctgggttatatcaaaggtctgtctaaaattatcaatgaaatgaactttgacgacgttctgtccattctgagcaaaattcacttctatcgcaacgtttcctccgaactggtttttggctggctggacgaaattgccacggcgtccaacaactataacattcagcgcaaagcgcaggaagtaaccgatctgctgattcgcaaaggcccgattaataactaa

SEQ ID NO: 126 - protein, 276 aa, Artificial Sequence
  amino acid sequence of I223V mutant
MESKIIGKVNFEEHLLDKELKLIDTFEFNDSYSEYASGIWKTCMLWNRSGQKDDHLSIEHDTYVKPTEYGKQLAYVNEIIANTFKKEHIKTVRLFMCINGLIIPHKDYLEFKKGFTRIHIPLKINEHALTSEEDVVYNMQKGEIWFIEGRKIHSAANFSKVKRINLVIDFAPDIPFEELFLNSENYQPNLIPKISQRTQLKEEELGYIKGLSKIINEMNFDDVLSILSKIHFYRNVSSELVFGWLDEIATASNNYNIQRKAQEVTDLLIRKGPINN

SEQ ID NO: 127 - DNA, 831 bp, Artificial Sequence
  gene sequence of E27K+ K123D mutant
atggaatccaagatcatcggtaaagtcaacttcgaggagcatctgctggataaagagctgaaactgatcgacactttcaaattcaacgacagctacagcgaatacgcttctggtatttggaagacttgcatgctgtggaaccgttctggtcagaaagatgaccatctgtctattgaacatgatacctacgtgaaacctactgaatacggcaaacagctggcatacgtaaacgaaatcatcgctaacacctttaagaaagaacacatcaagacggtgcgtctgttcatgtgtatcaacggcctgatcatcccacacaaagactacctggaattcaagaaaggcttcacccgtatccacatcccgctggatatcaacgaacacgcactgacctctgaagaagatgttgtttacaacatgcagaaaggtgaaatttggttcatcgaaggccgtaaaatccacagcgctgccaatttcagcaaagtgaaacgtatcaacctggtcatcgacttcgcgccggatattccgtttgaagaactgttcctgaattctgagaactatcaaccgaacctgatcccgaaaatctctcaacgtacccagctgaaagaagaagagctgggttatatcaaaggtctgtctaaaattatcaatgaaatgaactttgacgacatcctgtccattctgagcaaaattcacttctatcgcaacgtttcctccgaactggtttttggctggctggacgaaattgccacggcgtccaacaactataacattcagcgcaaagcgcaggaagtaaccgatctgctgattcgcaaaggcccgattaataactaa

SEQ ID NO: 128 - protein, 276 aa, Artificial Sequence
  amino acid sequence of E27K+ K123D mutant
MESKIIGKVNFEEHLLDKELKLIDTFKFNDSYSEYASGIWKTCMLWNRSGQKDDHLSIEHDTYVKPTEYGKQLAYVNEIIANTFKKEHIKTVRLFMCINGLIIPHKDYLEFKKGFTRIHIPLDINEHALTSEEDVVYNMQKGEIWFIEGRKIHSAANFSKVKRINLVIDFAPDIPFEELFLNSENYQPNLIPKISQRTQLKEEELGYIKGLSKIINEMNFDDILSILSKIHFYRNVSSELVFGWLDEIATASNNYNIQRKAQEVTDLLIRKGPINN

SEQ ID NO: 129 - DNA, 831 bp, Artificial Sequence
  gene sequence of E27K+ I39K mutant
atggaatccaagatcatcggtaaagtcaacttcgaggagcatctgctggataaagagctgaaactgatcgacactttcaaattcaacgacagctacagcgaatacgcttctggtaaatggaagacttgcatgctgtggaaccgttctggtcagaaagatgaccatctgtctattgaacatgatacctacgtgaaacctactgaatacggcaaacagctggcatacgtaaacgaaatcatcgctaacacctttaagaaagaacacatcaagacggtgcgtctgttcatgtgtatcaacggcctgatcatcccacacaaagactacctggaattcaagaaaggcttcacccgtatccacatcccgctgaaaatcaacgaacacgcactgacctctgaagaagatgttgtttacaacatgcagaaaggtgaaatttggttcatcgaaggccgtaaaatccacagcgctgccaatttcagcaaagtgaaacgtatcaacctggtcatcgacttcgcgccggatattccgtttgaagaactgttcctgaattctgagaactatcaaccgaacctgatcccgaaaatctctcaacgtacccagctgaaagaagaagagctgggttatatcaaaggtctgtctaaaattatcaatgaaatgaactttgacgacatcctgtccattctgagcaaaattcacttctatcgcaacgtttcctccgaactggtttttggctggctggacgaaattgccacggcgtccaacaactataacattcagcgcaaagcgcaggaagtaaccgatctgctgattcgcaaaggcccgattaataactaa

SEQ ID NO: 130 - protein, 276 aa, Artificial Sequence
  amino acid sequence of E27K+I39K mutant
MESKIIGKVNFEEHLLDKELKLIDTFKFNDSYSEYASGKWKTCMLWNRSGQKDDHLSIEHDTYVKPTEYGKQLAYVNEIIANTFKKEHIKTVRLFMCINGLIIPHKDYLEFKKGFTRIHIPLKINEHALTSEEDVVYNMQKGEIWFIEGRKIHSAANFSKVKRINLVIDFAPDIPFEELFLNSENYQPNLIPKISQRTQLKEEELGYIKGLSKIINEMNFDDILSILSKIHFYRNVSSELVFGWLDEIATASNNYNIQRKAQEVTDLLIRKGPINN

SEQ ID NO: 131 - DNA, 831 bp, Artificial Sequence
  gene sequence of I39K+K123Q mutant
atggaatccaagatcatcggtaaagtcaacttcgaggagcatctgctggataaagagctgaaactgatcgacactttcgagttcaacgacagctacagcgaatacgcttctggtaaatggaagacttgcatgctgtggaaccgttctggtcagaaagatgaccatctgtctattgaacatgatacctacgtgaaacctactgaatacggcaaacagctggcatacgtaaacgaaatcatcgctaacacctttaagaaagaacacatcaagacggtgcgtctgttcatgtgtatcaacggcctgatcatcccacacaaagactacctggaattcaagaaaggcttcacccgtatccacatcccgctggatatcaacgaacacgcactgacctctgaagaagatgttgtttacaacatgcagaaaggtgaaatttggttcatcgaaggccgtaaaatccacagcgctgccaatttcagcaaagtgaaacgtatcaacctggtcatcgacttcgcgccggatattccgtttgaagaactgttcctgaattctgagaactatcaaccgaacctgatcccgaaaatctctcaacgtacccagctgaaagaagaagagctgggttatatcaaaggtctgtctaaaattatcaatgaaatgaactttgacgacatcctgtccattctgagcaaaattcacttctatcgcaacgtttcctccgaactggtttttggctggctggacaaaattgccacggcgtccaacaactataacattcagcgcaaagcgcaggaagtaaccgatctgctgattcgcaaaggcccgattaataactaa

SEQ ID NO: 132 - protein, 276 aa, Artificial Sequence
  amino acid sequence of I39K+K123Q mutant
MESKIIGKVNFEEHLLDKELKLIDTFEFNDSYSEYASGKWKTCMLWNRSGQKDDHLSIEHDTYVKPTEYGKQLAYVNEIIANTFKKEHIKTVRLFMCINGLIIPHKDYLEFKKGFTRIHIPLDINEHALTSEEDVVYNMQKGEIWFIEGRKIHSAANFSKVKRINLVIDFAPDIPFEELFLNSENYQPNLIPKISQRTQLKEEELGYIKGLSKIINEMNFDDILSILSKIHFYRNVSSELVFGWLDKIATASNNYNIQRKAQEVTDLLIRKGPINN

SEQ ID NO: 133 - DNA, 831 bp, Artificial Sequence
  gene sequence of I39K+ K123D mutant
atggaatccaagatcatcggtaaagtcaacttcgaggagcatctgctggataaagagctgaaactgatcgacactttcgagttcaacgacagctacagcgaatacgcttctggtaaatggaagacttgcatgctgtggaaccgttctggtcagaaagatgaccatctgtctattgaacatgatacctacgtgaaacctactgaatacggcaaacagctggcatacgtaaacgaaatcatcgctaacacctttaagaaagaacacatcaagacggtgcgtctgttcatgtgtatcaacggcctgatcatcccacacaaagactacctggaattcaagaaaggcttcacccgtatccacatcccgctggatatcaacgaacacgcactgacctctgaagaagatgttgtttacaacatgcagaaaggtgaaatttggttcatcgaaggccgtaaaatccacagcgctgccaatttcagcaaagtgaaacgtatcaacctggtcatcgacttcgcgccggatattccgtttgaagaactgttcctgaattctgagaactatcaaccgaacctgatcccgaaaatctctcaacgtacccagctgaaagaagaagagctgggttatatcaaaggtctgtctaaaattatcaatgaaatgaactttgacgacatcctgtccattctgagcaaaattcacttctatcgcaacgtttcctccgaactggtttttggctggctggacgaaattgccacggcgtccaacaactataacattcagcgcaaagcgcaggaagtaaccgatctgctgattcgcaaaggcccgattaataactaa

SEQ ID NO: 134 - protein, 276 aa, Artificial Sequence
  amino acid sequence of I39K+ K123D mutant
MESKIIGKVNFEEHLLDKELKLIDTFEFNDSYSEYASGKWKTCMLWNRSGQKDDHLSIEHDTYVKPTEYGKQLAYVNEIIANTFKKEHIKTVRLFMCINGLIIPHKDYLEFKKGFTRIHIPLDINEHALTSEEDVVYNMQKGEIWFIEGRKIHSAANFSKVKRINLVIDFAPDIPFEELFLNSENYQPNLIPKISQRTQLKEEELGYIKGLSKIINEMNFDDILSILSKIHFYRNVSSELVFGWLDEIATASNNYNIQRKAQEVTDLLIRKGPINN

SEQ ID NO: 135 - DNA, 831 bp, Artificial Sequence
  gene sequence of S37C+I223V+ K123D mutant
atggaatccaagatcatcggtaaagtcaacttcgaggagcatctgctggataaagagctgaaactgatcgacactttcgagttcaacgacagctacagcgaatacgcttgtggtatttggaagacttgcatgctgtggaaccgttctggtcagaaagatgaccatctgtctattgaacatgatacctacgtgaaacctactgaatacggcaaacagctggcatacgtaaacgaaatcatcgctaacacctttaagaaagaacacatcaagacggtgcgtctgttcatgtgtatcaacggcctgatcatcccacacaaagactacctggaattcaagaaaggcttcacccgtatccacatcccgctggatatcaacgaacacgcactgacctctgaagaagatgttgtttacaacatgcagaaaggtgaaatttggttcatcgaaggccgtaaaatccacagcgctgccaatttcagcaaagtgaaacgtatcaacctggtcatcgacttcgcgccggatattccgtttgaagaactgttcctgaattctgagaactatcaaccgaacctgatcccgaaaatctctcaacgtacccagctgaaagaagaagagctgggttatatcaaaggtctgtctaaaattatcaatgaaatgaactttgacgacgttctgtccattctgagcaaaattcacttctatcgcaacgtttcctccgaactggtttttggctggctggacgaaattgccacggcgtccaacaactataacattcagcgcaaagcgcaggaagtaaccgatctgctgattcgcaaaggcccgattaataactaa

SEQ ID NO: 136 - protein, 276 aa, Artificial Sequence
  amino acid sequence of S37C+I223V+ K123D mutant
MESKIIGKVNFEEHLLDKELKLIDTFEFNDSYSEYACGIWKTCMLWNRSGQKDDHLSIEHDTYVKPTEYGKQLAYVNEIIANTFKKEHIKTVRLFMCINGLIIPHKDYLEFKKGFTRIHIPLDINEHALTSEEDVVYNMQKGEIWFIEGRKIHSAANFSKVKRINLVIDFAPDIPFEELFLNSENYQPNLIPKISQRTQLKEEELGYIKGLSKIINEMNFDDVLSILSKIHFYRNVSSELVFGWLDEIATASNNYNIQRKAQEVTDLLIRKGPINN

SEQ ID NO: 137 - DNA, 831 bp, Artificial Sequence
  gene sequence of K123D+N165H mutant
atggaatccaagatcatcggtaaagtcaacttcgaggagcatctgctggataaagagctgaaactgatcgacactttcgagttcaacgacagctacagcgaatacgcttctggtatttggaagacttgcatgctgtggaaccgttctggtcagaaagatgaccatctgtctattgaacatgatacctacgtgaaacctactgaatacggcaaacagctggcatacgtaaacgaaatcatcgctaacacctttaagaaagaacacatcaagacggtgcgtctgttcatgtgtatcaacggcctgatcatcccacacaaagactacctggaattcaagaaaggcttcacccgtatccacatcccgctggatatcaacgaacacgcactgacctctgaagaagatgttgtttacaacatgcagaaaggtgaaatttggttcatcgaaggccgtaaaatccacagcgctgccaatttcagcaaagtgaaacgtatccatctggtcatcgacttcgcgccggatattccgtttgaagaactgttcctgaattctgagaactatcaaccgaacctgatcccgaaaatctctcaacgtacccagctgaaagaagaagagctgggttatatcaaaggtctgtctaaaattatcaatgaaatgaactttgacgacatcctgtccattctgagcaaaattcacttctatcgcaacgtttcctccgaactggtttttggctggctggacgaaattgccacggcgtccaacaactataacattcagcgcaaagcgcaggaagtaaccgatctgctgattcgcaaaggcccgattaataactaa

SEQ ID NO: 138 - protein, 276 aa, Artificial Sequence
  amino acid sequence of K123D+N165H mutant
MESKIIGKVNFEEHLLDKELKLIDTFEFNDSYSEYASGIWKTCMLWNRSGQKDDHLSIEHDTYVKPTEYGKQLAYVNEIIANTFKKEHIKTVRLFMCINGLIIPHKDYLEFKKGFTRIHIPLDINEHALTSEEDVVYNMQKGEIWFIEGRKIHSAANFSKVKRIHLVIDFAPDIPFEELFLNSENYQPNLIPKISQRTQLKEEELGYIKGLSKIINEMNFDDILSILSKIHFYRNVSSELVFGWLDEIATASNNYNIQRKAQEVTDLLIRKGPINN

SEQ ID NO: 139 - DNA, 831 bp, Artificial Sequence
  gene sequence of I39R+K123D mutant
atggaatccaagatcatcggtaaagtcaacttcgaggagcatctgctggataaagagctgaaactgatcgacactttcgagttcaacgacagctacagcgaatacgcttctggtcgttggaagacttgcatgctgtggaaccgttctggtcagaaagatgaccatctgtctattgaacatgatacctacgtgaaacctactgaatacggcaaacagctggcatacgtaaacgaaatcatcgctaacacctttaagaaagaacacatcaagacggtgcgtctgttcatgtgtatcaacggcctgatcatcccacacaaagactacctggaattcaagaaaggcttcacccgtatccacatcccgctggatatcaacgaacacgcactgacctctgaagaagatgttgtttacaacatgcagaaaggtgaaatttggttcatcgaaggccgtaaaatccacagcgctgccaatttcagcaaagtgaaacgtatcaacctggtcatcgacttcgcgccggatattccgtttgaagaactgttcctgaattctgagaactatcaaccgaacctgatcccgaaaatctctcaacgtacccagctgaaagaagaagagctgggttatatcaaaggtctgtctaaaattatcaatgaaatgaactttgacgacatcctgtccattctgagcaaaattcacttctatcgcaacgtttcctccgaactggtttttggctggctggacgaaattgccacggcgtccaacaactataacattcagcgcaaagcgcaggaagtaaccgatctgctgattcgcaaaggcccgattaataactaa

SEQ ID NO: 140 - protein, 276 aa, Artificial Sequence
  amino acid sequence of I39R+K123D mutant
MESKIIGKVNFEEHLLDKELKLIDTFEFNDSYSEYASGRWKTCMLWNRSGQKDDHLSIEHDTYVKPTEYGKQLAYVNEIIANTFKKEHIKTVRLFMCINGLIIPHKDYLEFKKGFTRIHIPLDINEHALTSEEDVVYNMQKGEIWFIEGRKIHSAANFSKVKRINLVIDFAPDIPFEELFLNSENYQPNLIPKISQRTQLKEEELGYIKGLSKIINEMNFDDILSILSKIHFYRNVSSELVFGWLDEIATASNNYNIQRKAQEVTDLLIRKGPINN

SEQ ID NO: 141 - DNA, 831 bp, Artificial Sequence
  gene sequence of E27K+I39K+K123D mutant
atggaatccaagatcatcggtaaagtcaacttcgaggagcatctgctggataaagagctgaaactgatcgacactttcaaattcaacgacagctacagcgaatacgcttctggtaaatggaagacttgcatgctgtggaaccgttctggtcagaaagatgaccatctgtctattgaacatgatacctacgtgaaacctactgaatacggcaaacagctggcatacgtaaacgaaatcatcgctaacacctttaagaaagaacacatcaagacggtgcgtctgttcatgtgtatcaacggcctgatcatcccacacaaagactacctggaattcaagaaaggcttcacccgtatccacatcccgctggatatcaacgaacacgcactgacctctgaagaagatgttgtttacaacatgcagaaaggtgaaatttggttcatcgaaggccgtaaaatccacagcgctgccaatttcagcaaagtgaaacgtatcaacctggtcatcgacttcgcgccggatattccgtttgaagaactgttcctgaattctgagaactatcaaccgaacctgatcccgaaaatctctcaacgtacccagctgaaagaagaagagctgggttatatcaaaggtctgtctaaaattatcaatgaaatgaactttgacgacatcctgtccattctgagcaaaattcacttctatcgcaacgtttcctccgaactggtttttggctggctggacgaaattgccacggcgtccaacaactataacattcagcgcaaagcgcaggaagtaaccgatctgctgattcgcaaaggcccgattaataactaa

SEQ ID NO: 142 - protein, 276 aa, Artificial Sequence
  amino acid sequence of E27K+I39K+K123D mutant
MESKIIGKVNFEEHLLDKELKLIDTFKFNDSYSEYASGKWKTCMLWNRSGQKDDHLSIEHDTYVKPTEYGKQLAYVNEIIANTFKKEHIKTVRLFMCINGLIIPHKDYLEFKKGFTRIHIPLDINEHALTSEEDVVYNMQKGEIWFIEGRKIHSAANFSKVKRINLVIDFAPDIPFEELFLNSENYQPNLIPKISQRTQLKEEELGYIKGLSKIINEMNFDDILSILSKIHFYRNVSSELVFGWLDEIATASNNYNIQRKAQEVTDLLIRKGPINN

SEQ ID NO: 143 - DNA, 831 bp, Artificial Sequence
  gene sequence of E27K+ I39R mutant
atggaatccaagatcatcggtaaagtcaacttcgaggagcatctgctggataaagagctgaaactgatcgacactttcaaattcaacgacagctacagcgaatacgcttctggtcgttggaagacttgcatgctgtggaaccgttctggtcagaaagatgaccatctgtctattgaacatgatacctacgtgaaacctactgaatacggcaaacagctggcatacgtaaacgaaatcatcgctaacacctttaagaaagaacacatcaagacggtgcgtctgttcatgtgtatcaacggcctgatcatcccacacaaagactacctggaattcaagaaaggcttcacccgtatccacatcccgctgaaaatcaacgaacacgcactgacctctgaagaagatgttgtttacaacatgcagaaaggtgaaatttggttcatcgaaggccgtaaaatccacagcgctgccaatttcagcaaagtgaaacgtatcaacctggtcatcgacttcgcgccggatattccgtttgaagaactgttcctgaattctgagaactatcaaccgaacctgatcccgaaaatctctcaacgtacccagctgaaagaagaagagctgggttatatcaaaggtctgtctaaaattatcaatgaaatgaactttgacgacatcctgtccattctgagcaaaattcacttctatcgcaacgtttcctccgaactggtttttggctggctggacgaaattgccacggcgtccaacaactataacattcagcgcaaagcgcaggaagtaaccgatctgctgattcgcaaaggcccgattaataactaa

SEQ ID NO: 144 - protein, 276 aa, Artificial Sequence
  amino acid sequence of E27K+ I39R mutant
MESKIIGKVNFEEHLLDKELKLIDTFKFNDSYSEYASGRWKTCMLWNRSGQKDDHLSIEHDTYVKPTEYGKQLAYVNEIIANTFKKEHIKTVRLFMCINGLIIPHKDYLEFKKGFTRIHIPLKINEHALTSEEDVVYNMQKGEIWFIEGRKIHSAANFSKVKRINLVIDFAPDIPFEELFLNSENYQPNLIPKISQRTQLKEEELGYIKGLSKIINEMNFDDILSILSKIHFYRNVSSELVFGWLDEIATASNNYNIQRKAQEVTDLLIRKGPINN

SEQ ID NO: 145 - DNA, 831 bp, Artificial Sequence
  gene sequence of I39R+N165H mutant
atggaatccaagatcatcggtaaagtcaacttcgaggagcatctgctggataaagagctgaaactgatcgacactttcgagttcaacgacagctacagcgaatacgcttctggtcgttggaagacttgcatgctgtggaaccgttctggtcagaaagatgaccatctgtctattgaacatgatacctacgtgaaacctactgaatacggcaaacagctggcatacgtaaacgaaatcatcgctaacacctttaagaaagaacacatcaagacggtgcgtctgttcatgtgtatcaacggcctgatcatcccacacaaagactacctggaattcaagaaaggcttcacccgtatccacatcccgctgaaaatcaacgaacacgcactgacctctgaagaagatgttgtttacaacatgcagaaaggtgaaatttggttcatcgaaggccgtaaaatccacagcgctgccaatttcagcaaagtgaaacgtatccatctggtcatcgacttcgcgccggatattccgtttgaagaactgttcctgaattctgagaactatcaaccgaacctgatcccgaaaatctctcaacgtacccagctgaaagaagaagagctgggttatatcaaaggtctgtctaaaattatcaatgaaatgaactttgacgacatcctgtccattctgagcaaaattcacttctatcgcaacgtttcctccgaactggtttttggctggctggacgaaattgccacggcgtccaacaactataacattcagcgcaaagcgcaggaagtaaccgatctgctgattcgcaaaggcccgattaataactaa

SEQ ID NO: 146 - protein, 276 aa, Artificial Sequence
  amino acid sequence of I39R+N165H mutant
MESKIIGKVNFEEHLLDKELKLIDTFEFNDSYSEYASGRWKTCMLWNRSGQKDDHLSIEHDTYVKPTEYGKQLAYVNEIIANTFKKEHIKTVRLFMCINGLIIPHKDYLEFKKGFTRIHIPLKINEHALTSEEDVVYNMQKGEIWFIEGRKIHSAANFSKVKRIHLVIDFAPDIPFEELFLNSENYQPNLIPKISQRTQLKEEELGYIKGLSKIINEMNFDDILSILSKIHFYRNVSSELVFGWLDEIATASNNYNIQRKAQEVTDLLIRKGPINN

SEQ ID NO: 147 - DNA, 831 bp, Artificial Sequence
  gene sequence of I39K+N165H mutant
atggaatccaagatcatcggtaaagtcaacttcgaggagcatctgctggataaagagctgaaactgatcgacactttcgagttcaacgacagctacagcgaatacgcttctggtaaatggaagacttgcatgctgtggaaccgttctggtcagaaagatgaccatctgtctattgaacatgatacctacgtgaaacctactgaatacggcaaacagctggcatacgtaaacgaaatcatcgctaacacctttaagaaagaacacatcaagacggtgcgtctgttcatgtgtatcaacggcctgatcatcccacacaaagactacctggaattcaagaaaggcttcacccgtatccacatcccgctgaaaatcaacgaacacgcactgacctctgaagaagatgttgtttacaacatgcagaaaggtgaaatttggttcatcgaaggccgtaaaatccacagcgctgccaatttcagcaaagtgaaacgtatccatctggtcatcgacttcgcgccggatattccgtttgaagaactgttcctgaattctgagaactatcaaccgaacctgatcccgaaaatctctcaacgtacccagctgaaagaagaagagctgggttatatcaaaggtctgtctaaaattatcaatgaaatgaactttgacgacatcctgtccattctgagcaaaattcacttctatcgcaacgtttcctccgaactggtttttggctggctggacgaaattgccacggcgtccaacaactataacattcagcgcaaagcgcaggaagtaaccgatctgctgattcgcaaaggcccgattaataactaa

SEQ ID NO: 148 - protein, 276 aa, Artificial Sequence
  amino acid sequence of I39K+N165H mutant
MESKIIGKVNFEEHLLDKELKLIDTFEFNDSYSEYASGKWKTCMLWNRSGQKDDHLSIEHDTYVKPTEYGKQLAYVNEIIANTFKKEHIKTVRLFMCINGLIIPHKDYLEFKKGFTRIHIPLKINEHALTSEEDVVYNMQKGEIWFIEGRKIHSAANFSKVKRIHLVIDFAPDIPFEELFLNSENYQPNLIPKISQRTQLKEEELGYIKGLSKIINEMNFDDILSILSKIHFYRNVSSELVFGWLDEIATASNNYNIQRKAQEVTDLLIRKGPINN

SEQ ID NO: 149 - DNA, 831 bp, Artificial Sequence; identical to SEQ ID NO: 141
  gene sequence of E27K+ I39K+K123D mutant

SEQ ID NO: 150 - protein, 276 aa, Artificial Sequence; identical to SEQ ID NO: 142
  amino acid sequence of E27K+ I39K+K123D mutant

SEQ ID NO: 151 - DNA, 831 bp, Artificial Sequence
  gene sequence of S37C+I223V+N165H mutant
atggaatccaagatcatcggtaaagtcaacttcgaggagcatctgctggataaagagctgaaactgatcgacactttcgagttcaacgacagctacagcgaatacgcttgtggtatttggaagacttgcatgctgtggaaccgttctggtcagaaagatgaccatctgtctattgaacatgatacctacgtgaaacctactgaatacggcaaacagctggcatacgtaaacgaaatcatcgctaacacctttaagaaagaacacatcaagacggtgcgtctgttcatgtgtatcaacggcctgatcatcccacacaaagactacctggaattcaagaaaggcttcacccgtatccacatcccgctgaaaatcaacgaacacgcactgacctctgaagaagatgttgtttacaacatgcagaaaggtgaaatttggttcatcgaaggccgtaaaatccacagcgctgccaatttcagcaaagtgaaacgtatccatctggtcatcgacttcgcgccggatattccgtttgaagaactgttcctgaattctgagaactatcaaccgaacctgatcccgaaaatctctcaacgtacccagctgaaagaagaagagctgggttatatcaaaggtctgtctaaaattatcaatgaaatgaactttgacgacgttctgtccattctgagcaaaattcacttctatcgcaacgtttcctccgaactggtttttggctggctggacgaaattgccacggcgtccaacaactataacattcagcgcaaagcgcaggaagtaaccgatctgctgattcgcaaaggcccgattaataactaa

SEQ ID NO: 152 - protein, 276 aa, Artificial Sequence
  amino acid sequence of S37C+I223V+N165H mutant
MESKIIGKVNFEEHLLDKELKLIDTFEFNDSYSEYACGIWKTCMLWNRSGQKDDHLSIEHDTYVKPTEYGKQLAYVNEIIANTFKKEHIKTVRLFMCINGLIIPHKDYLEFKKGFTRIHIPLKINEHALTSEEDVVYNMQKGEIWFIEGRKIHSAANFSKVKRIHLVIDFAPDIPFEELFLNSENYQPNLIPKISQRTQLKEEELGYIKGLSKIINEMNFDDVLSILSKIHFYRNVSSELVFGWLDEIATASNNYNIQRKAQEVTDLLIRKGPINN

SEQ ID NO: 153 - DNA, 831 bp, Artificial Sequence
  gene sequence of K123D+W40F mutant
atggaatccaagatcatcggtaaagtcaacttcgaggagcatctgctggataaagagctgaaactgatcgacactttcgagttcaacgacagctacagcgaatacgcttctggtatttttaagacttgcatgctgtggaaccgttctggtcagaaagatgaccatctgtctattgaacatgatacctacgtgaaacctactgaatacggcaaacagctggcatacgtaaacgaaatcatcgctaacacctttaagaaagaacacatcaagacggtgcgtctgttcatgtgtatcaacggcctgatcatcccacacaaagactacctggaattcaagaaaggcttcacccgtatccacatcccgctggatatcaacgaacacgcactgacctctgaagaagatgttgtttacaacatgcagaaaggtgaaatttggttcatcgaaggccgtaaaatccacagcgctgccaatttcagcaaagtgaaacgtatcaacctggtcatcgacttcgcgccggatattccgtttgaagaactgttcctgaattctgagaactatcaaccgaacctgatcccgaaaatctctcaacgtacccagctgaaagaagaagagctgggttatatcaaaggtctgtctaaaattatcaatgaaatgaactttgacgacatcctgtccattctgagcaaaattcacttctatcgcaacgtttcctccgaactggtttttggctggctggacgaaattgccacggcgtccaacaactataacattcagcgcaaagcgcaggaagtaaccgatctgctgattcgcaaaggcccgattaataactaa

SEQ ID NO: 154 - protein, 276 aa, Artificial Sequence
  amino acid sequence of K123D+W40F mutant
MESKIIGKVNFEEHLLDKELKLIDTFEFNDSYSEYASGIFKTCMLWNRSGQKDDHLSIEHDTYVKPTEYGKQLAYVNEIIANTFKKEHIKTVRLFMCINGLIIPHKDYLEFKKGFTRIHIPLDINEHALTSEEDVVYNMQKGEIWFIEGRKIHSAANFSKVKRINLVIDFAPDIPFEELFLNSENYQPNLIPKISQRTQLKEEELGYIKGLSKIINEMNFDDILSILSKIHFYRNVSSELVFGWLDEIATASNNYNIQRKAQEVTDLLIRKGPINN

SEQ ID NO: 155 - DNA, 831 bp, Artificial Sequence
  gene sequence of E27K+N165H mutant
atggaatccaagatcatcggtaaagtcaacttcgaggagcatctgctggataaagagctgaaactgatcgacactttcaaattcaacgacagctacagcgaatacgcttctggtatttggaagacttgcatgctgtggaaccgttctggtcagaaagatgaccatctgtctattgaacatgatacctacgtgaaacctactgaatacggcaaacagctggcatacgtaaacgaaatcatcgctaacacctttaagaaagaacacatcaagacggtgcgtctgttcatgtgtatcaacggcctgatcatcccacacaaagactacctggaattcaagaaaggcttcacccgtatccacatcccgctgaaaatcaacgaacacgcactgacctctgaagaagatgttgtttacaacatgcagaaaggtgaaatttggttcatcgaaggccgtaaaatccacagcgctgccaatttcagcaaagtgaaacgtatccatctggtcatcgacttcgcgccggatattccgtttgaagaactgttcctgaattctgagaactatcaaccgaacctgatcccgaaaatctctcaacgtacccagctgaaagaagaagagctgggttatatcaaaggtctgtctaaaattatcaatgaaatgaactttgacgacatcctgtccattctgagcaaaattcacttctatcgcaacgtttcctccgaactggtttttggctggctggacgaaattgccacggcgtccaacaactataacattcagcgcaaagcgcaggaagtaaccgatctgctgattcgcaaaggcccgattaataactaa

SEQ ID NO: 156 - protein, 276 aa, Artificial Sequence
  amino acid sequence of E27K+N165H mutant
MESKIIGKVNFEEHLLDKELKLIDTFKFNDSYSEYASGIWKTCMLWNRSGQKDDHLSIEHDTYVKPTEYGKQLAYVNEIIANTFKKEHIKTVRLFMCINGLIIPHKDYLEFKKGFTRIHIPLKINEHALTSEEDVVYNMQKGEIWFIEGRKIHSAANFSKVKRIHLVIDFAPDIPFEELFLNSENYQPNLIPKISQRTQLKEEELGYIKGLSKIINEMNFDDILSILSKIHFYRNVSSELVFGWLDEIATASNNYNIQRKAQEVTDLLIRKGPINN

SEQ ID NO: 157 - DNA, 831 bp, Artificial Sequence
  gene sequence of E27K+ S37C+I223V+ K123D mutant
atggaatccaagatcatcggtaaagtcaacttcgaggagcatctgctggataaagagctgaaactgatcgacactttcaaattcaacgacagctacagcgaatacgcttgtggtatttggaagacttgcatgctgtggaaccgttctggtcagaaagatgaccatctgtctattgaacatgatacctacgtgaaacctactgaatacggcaaacagctggcatacgtaaacgaaatcatcgctaacacctttaagaaagaacacatcaagacggtgcgtctgttcatgtgtatcaacggcctgatcatcccacacaaagactacctggaattcaagaaaggcttcacccgtatccacatcccgctggatatcaacgaacacgcactgacctctgaagaagatgttgtttacaacatgcagaaaggtgaaatttggttcatcgaaggccgtaaaatccacagcgctgccaatttcagcaaagtgaaacgtatcaacctggtcatcgacttcgcgccggatattccgtttgaagaactgttcctgaattctgagaactatcaaccgaacctgatcccgaaaatctctcaacgtacccagctgaaagaagaagagctgggttatatcaaaggtctgtctaaaattatcaatgaaatgaactttgacgacgttctgtccattctgagcaaaattcacttctatcgcaacgtttcctccgaactggtttttggctggctggacgaaattgccacggcgtccaacaactataacattcagcgcaaagcgcaggaagtaaccgatctgctgattcgcaaaggcccgattaataactaa

SEQ ID NO: 158 - protein, 276 aa, Artificial Sequence
  amino acid sequence of E27K+ S37C+I223V+ K123D mutant
MESKIIGKVNFEEHLLDKELKLIDTFKFNDSYSEYACGIWKTCMLWNRSGQKDDHLSIEHDTYVKPTEYGKQLAYVNEIIANTFKKEHIKTVRLFMCINGLIIPHKDYLEFKKGFTRIHIPLDINEHALTSEEDVVYNMQKGEIWFIEGRKIHSAANFSKVKRINLVIDFAPDIPFEELFLNSENYQPNLIPKISQRTQLKEEELGYIKGLSKIINEMNFDDVLSILSKIHFYRNVSSELVFGWLDEIATASNNYNIQRKAQEVTDLLIRKGPINN

SEQ ID NO: 159 - DNA, 831 bp, Artificial Sequence
  gene sequence of S37C+I39K+I223V+ K123D mutant
atggaatccaagatcatcggtaaagtcaacttcgaggagcatctgctggataaagagctgaaactgatcgacactttcgagttcaacgacagctacagcgaatacgcttgtggtaaatggaagacttgcatgctgtggaaccgttctggtcagaaagatgaccatctgtctattgaacatgatacctacgtgaaacctactgaatacggcaaacagctggcatacgtaaacgaaatcatcgctaacacctttaagaaagaacacatcaagacggtgcgtctgttcatgtgtatcaacggcctgatcatcccacacaaagactacctggaattcaagaaaggcttcacccgtatccacatcccgctggatatcaacgaacacgcactgacctctgaagaagatgttgtttacaacatgcagaaaggtgaaatttggttcatcgaaggccgtaaaatccacagcgctgccaatttcagcaaagtgaaacgtatcaacctggtcatcgacttcgcgccggatattccgtttgaagaactgttcctgaattctgagaactatcaaccgaacctgatcccgaaaatctctcaacgtacccagctgaaagaagaagagctgggttatatcaaaggtctgtctaaaattatcaatgaaatgaactttgacgacgttctgtccattctgagcaaaattcacttctatcgcaacgtttcctccgaactggtttttggctggctggacgaaattgccacggcgtccaacaactataacattcagcgcaaagcgcaggaagtaaccgatctgctgattcgcaaaggcccgattaataactaa

SEQ ID NO: 160 - protein, 276 aa, Artificial Sequence
  amino acid sequence of S37C+I39K+I223V+ K123D mutant
MESKIIGKVNFEEHLLDKELKLIDTFEFNDSYSEYACGKWKTCMLWNRSGQKDDHLSIEHDTYVKPTEYGKQLAYVNEIIANTFKKEHIKTVRLFMCINGLIIPHKDYLEFKKGFTRIHIPLDINEHALTSEEDVVYNMQKGEIWFIEGRKIHSAANFSKVKRINLVIDFAPDIPFEELFLNSENYQPNLIPKISQRTQLKEEELGYIKGLSKIINEMNFDDVLSILSKIHFYRNVSSELVFGWLDEIATASNNYNIQRKAQEVTDLLIRKGPINN

SEQ ID NO: 161 - DNA, 831 bp, Artificial Sequence
  gene sequence of E27K+S37C+I39K+K123D+I98V mutant
atggaatccaagatcatcggtaaagtcaacttcgaggagcatctgctggataaagagctgaaactgatcgacactttcaaattcaacgacagctacagcgaatacgcttgtggtaaatggaagacttgcatgctgtggaaccgttctggtcagaaagatgaccatctgtctattgaacatgatacctacgtgaaacctactgaatacggcaaacagctggcatacgtaaacgaaatcatcgctaacacctttaagaaagaacacatcaagacggtgcgtctgttcatgtgtgttaacggcctgatcatcccacacaaagactacctggaattcaagaaaggcttcacccgtatccacatcccgctggatatcaacgaacacgcactgacctctgaagaagatgttgtttacaacatgcagaaaggtgaaatttggttcatcgaaggccgtaaaatccacagcgctgccaatttcagcaaagtgaaacgtatcaacctggtcatcgacttcgcgccggatattccgtttgaagaactgttcctgaattctgagaactatcaaccgaacctgatcccgaaaatctctcaacgtacccagctgaaagaagaagagctgggttatatcaaaggtctgtctaaaattatcaatgaaatgaactttgacgacattctgtccattctgagcaaaattcacttctatcgcaacgtttcctccgaactggtttttggctggctggacgaaattgccacggcgtccaacaactataacattcagcgcaaagcgcaggaagtaaccgatctgctgattcgcaaaggcccgattaataactaa

SEQ ID NO: 162 - protein, 276 aa, Artificial Sequence
  amino acid sequence of E27K+S37C+I39K+K123D+I98V mutant
MESKIIGKVNFEEHLLDKELKLIDTFKFNDSYSEYACGKWKTCMLWNRSGQKDDHLSIEHDTYVKPTEYGKQLAYVNEIIANTFKKEHIKTVRLFMCVNGLIIPHKDYLEFKKGFTRIHIPLDINEHALTSEEDVVYNMQKGEIWFIEGRKIHSAANFSKVKRINLVIDFAPDIPFEELFLNSENYQPNLIPKISQRTQLKEEELGYIKGLSKIINEMNFDDILSILSKIHFYRNVSSELVFGWLDEIATASNNYNIQRKAQEVTDLLIRKGPINN

SEQ ID NO: 163 - DNA, 831 bp, Artificial Sequence
  gene sequence of E27K+S37C+I39K+K123D+I223V mutant
atggaatccaagatcatcggtaaagtcaacttcgaggagcatctgctggataaagagctgaaactgatcgacactttcaaattcaacgacagctacagcgaatacgcttgtggtaaatggaagacttgcatgctgtggaaccgttctggtcagaaagatgaccatctgtctattgaacatgatacctacgtgaaacctactgaatacggcaaacagctggcatacgtaaacgaaatcatcgctaacacctttaagaaagaacacatcaagacggtgcgtctgttcatgtgtatcaacggcctgatcatcccacacaaagactacctggaattcaagaaaggcttcacccgtatccacatcccgctggatatcaacgaacacgcactgacctctgaagaagatgttgtttacaacatgcagaaaggtgaaatttggttcatcgaaggccgtaaaatccacagcgctgccaatttcagcaaagtgaaacgtatcaacctggtcatcgacttcgcgccggatattccgtttgaagaactgttcctgaattctgagaactatcaaccgaacctgatcccgaaaatctctcaacgtacccagctgaaagaagaagagctgggttatatcaaaggtctgtctaaaattatcaatgaaatgaactttgacgacgttctgtccattctgagcaaaattcacttctatcgcaacgtttcctccgaactggtttttggctggctggacgaaattgccacggcgtccaacaactataacattcagcgcaaagcgcaggaagtaaccgatctgctgattcgcaaaggcccgattaataactaa

SEQ ID NO: 164 - protein, 276 aa, Artificial Sequence
  amino acid sequence of E27K+S37C+I39K+K123D+I223V mutant
MESKIIGKVNFEEHLLDKELKLIDTFKFNDSYSEYACGKWKTCMLWNRSGQKDDHLSIEHDTYVKPTEYGKQLAYVNEIIANTFKKEHIKTVRLFMCINGLIIPHKDYLEFKKGFTRIHIPLDINEHALTSEEDVVYNMQKGEIWFIEGRKIHSAANFSKVKRINLVIDFAPDIPFEELFLNSENYQPNLIPKISQRTQLKEEELGYIKGLSKIINEMNFDDVLSILSKIHFYRNVSSELVFGWLDEIATASNNYNIQRKAQEVTDLLIRKGPINN

SEQ ID NO: 165 - DNA, 831 bp, Artificial Sequence
  gene sequence of F26L+E27K+I39K+K123D mutant
atggaatccaagatcatcggtaaagtcaacttcgaggagcatctgctggataaagagctgaaactgatcgacactctgaaattcaacgacagctacagcgaatacgcttctggtaaatggaagacttgcatgctgtggaaccgttctggtcagaaagatgaccatctgtctattgaacatgatacctacgtgaaacctactgaatacggcaaacagctggcatacgtaaacgaaatcatcgctaacacctttaagaaagaacacatcaagacggtgcgtctgttcatgtgtatcaacggcctgatcatcccacacaaagactacctggaattcaagaaaggcttcacccgtatccacatcccgctggatatcaacgaacacgcactgacctctgaagaagatgttgtttacaacatgcagaaaggtgaaatttggttcatcgaaggccgtaaaatccacagcgctgccaatttcagcaaagtgaaacgtatcaacctggtcatcgacttcgcgccggatattccgtttgaagaactgttcctgaattctgagaactatcaaccgaacctgatcccgaaaatctctcaacgtacccagctgaaagaagaagagctgggttatatcaaaggtctgtctaaaattatcaatgaaatgaactttgacgacatcctgtccattctgagcaaaattcacttctatcgcaacgtttcctccgaactggtttttggctggctggacgaaattgccacggcgtccaacaactataacattcagcgcaaagcgcaggaagtaaccgatctgctgattcgcaaaggcccgattaataactaa

SEQ ID NO: 166 - protein, 276 aa, Artificial Sequence
  amino acid sequence of F26L+E27K+I39K+K123D mutant
MESKIIGKVNFEEHLLDKELKLIDTLKFNDSYSEYASGKWKTCMLWNRSGQKDDHLSIEHDTYVKPTEYGKQLAYVNEIIANTFKKEHIKTVRLFMCINGLIIPHKDYLEFKKGFTRIHIPLDINEHALTSEEDVVYNMQKGEIWFIEGRKIHSAANFSKVKRINLVIDFAPDIPFEELFLNSENYQPNLIPKISQRTQLKEEELGYIKGLSKIINEMNFDDILSILSKIHFYRNVSSELVFGWLDEIATASNNYNIQRKAQEVTDLLIRKGPINN

SEQ ID NO: 167 - DNA, 831 bp, Artificial Sequence
  gene sequence of I223V+S37C+E27K+I39K mutant
atggaatccaagatcatcggtaaagtcaacttcgaggagcatctgctggataaagagctgaaactgatcgacactttcaaattcaacgacagctacagcgaatacgcttgtggtaaatggaagacttgcatgctgtggaaccgttctggtcagaaagatgaccatctgtctattgaacatgatacctacgtgaaacctactgaatacggcaaacagctggcatacgtaaacgaaatcatcgctaacacctttaagaaagaacacatcaagacggtgcgtctgttcatgtgtatcaacggcctgatcatcccacacaaagactacctggaattcaagaaaggcttcacccgtatccacatcccgctgaaaatcaacgaacacgcactgacctctgaagaagatgttgtttacaacatgcagaaaggtgaaatttggttcatcgaaggccgtaaaatccacagcgctgccaatttcagcaaagtgaaacgtatcaacctggtcatcgacttcgcgccggatattccgtttgaagaactgttcctgaattctgagaactatcaaccgaacctgatcccgaaaatctctcaacgtacccagctgaaagaagaagagctgggttatatcaaaggtctgtctaaaattatcaatgaaatgaactttgacgacgttctgtccattctgagcaaaattcacttctatcgcaacgtttcctccgaactggtttttggctggctggacgaaattgccacggcgtccaacaactataacattcagcgcaaagcgcaggaagtaaccgatctgctgattcgcaaaggcccgattaataactaa

SEQ ID NO: 168 - protein, 276 aa, Artificial Sequence
  amino acid sequence of I223V+S37C+E27K+I39K mutant
MESKIIGKVNFEEHLLDKELKLIDTFKFNDSYSEYACGKWKTCMLWNRSGQKDDHLSIEHDTYVKPTEYGKQLAYVNEIIANTFKKEHIKTVRLFMCINGLIIPHKDYLEFKKGFTRIHIPLKINEHALTSEEDVVYNMQKGEIWFIEGRKIHSAANFSKVKRINLVIDFAPDIPFEELFLNSENYQPNLIPKISQRTQLKEEELGYIKGLSKIINEMNFDDVLSILSKIHFYRNVSSELVFGWLDEIATASNNYNIQRKAQEVTDLLIRKGPINN

SEQ ID NO: 169 - DNA, 831 bp, Artificial Sequence
  gene sequence of I223V+S37C+E27K+N165H mutant
atggaatccaagatcatcggtaaagtcaacttcgaggagcatctgctggataaagagctgaaactgatcgacactttcaaattcaacgacagctacagcgaatacgcttgtggtatttggaagacttgcatgctgtggaaccgttctggtcagaaagatgaccatctgtctattgaacatgatacctacgtgaaacctactgaatacggcaaacagctggcatacgtaaacgaaatcatcgctaacacctttaagaaagaacacatcaagacggtgcgtctgttcatgtgtatcaacggcctgatcatcccacacaaagactacctggaattcaagaaaggcttcacccgtatccacatcccgctgaaaatcaacgaacacgcactgacctctgaagaagatgttgtttacaacatgcagaaaggtgaaatttggttcatcgaaggccgtaaaatccacagcgctgccaatttcagcaaagtgaaacgtatccatctggtcatcgacttcgcgccggatattccgtttgaagaactgttcctgaattctgagaactatcaaccgaacctgatcccgaaaatctctcaacgtacccagctgaaagaagaagagctgggttatatcaaaggtctgtctaaaattatcaatgaaatgaactttgacgacgttctgtccattctgagcaaaattcacttctatcgcaacgtttcctccgaactggtttttggctggctggacgaaattgccacggcgtccaacaactataacattcagcgcaaagcgcaggaagtaaccgatctgctgattcgcaaaggcccgattaataactaa

SEQ ID NO: 170 - protein, 276 aa, Artificial Sequence
  amino acid sequence of I223V+S37C+E27K+N165H mutant
MESKIIGKVNFEEHLLDKELKLIDTFKFNDSYSEYACGIWKTCMLWNRSGQKDDHLSIEHDTYVKPTEYGKQLAYVNEIIANTFKKEHIKTVRLFMCINGLIIPHKDYLEFKKGFTRIHIPLKINEHALTSEEDVVYNMQKGEIWFIEGRKIHSAANFSKVKRIHLVIDFAPDIPFEELFLNSENYQPNLIPKISQRTQLKEEELGYIKGLSKIINEMNFDDVLSILSKIHFYRNVSSELVFGWLDEIATASNNYNIQRKAQEVTDLLIRKGPINN

SEQ ID NO: 171 - DNA, 831 bp, Artificial Sequence
  gene sequence of K123D+Y35W mutant
atggaatccaagatcatcggtaaagtcaacttcgaggagcatctgctggataaagagctgaaactgatcgacactttcgagttcaacgacagctacagcgaatgggcttctggtatttggaagacttgcatgctgtggaaccgttctggtcagaaagatgaccatctgtctattgaacatgatacctacgtgaaacctactgaatacggcaaacagctggcatacgtaaacgaaatcatcgctaacacctttaagaaagaacacatcaagacggtgcgtctgttcatgtgtatcaacggcctgatcatcccacacaaagactacctggaattcaagaaaggcttcacccgtatccacatcccgctggatatcaacgaacacgcactgacctctgaagaagatgttgtttacaacatgcagaaaggtgaaatttggttcatcgaaggccgtaaaatccacagcgctgccaatttcagcaaagtgaaacgtatcaacctggtcatcgacttcgcgccggatattccgtttgaagaactgttcctgaattctgagaactatcaaccgaacctgatcccgaaaatctctcaacgtacccagctgaaagaagaagagctgggttatatcaaaggtctgtctaaaattatcaatgaaatgaactttgacgacatcctgtccattctgagcaaaattcacttctatcgcaacgtttcctccgaactggtttttggctggctggacgaaattgccacggcgtccaacaactataacattcagcgcaaagcgcaggaagtaaccgatctgctgattcgcaaaggcccgattaataactaa

SEQ ID NO: 172 - protein, 276 aa, Artificial Sequence
  amino acid sequence of K123D+Y35W mutant
MESKIIGKVNFEEHLLDKELKLIDTFEFNDSYSEWASGIWKTCMLWNRSGQKDDHLSIEHDTYVKPTEYGKQLAYVNEIIANTFKKEHIKTVRLFMCINGLIIPHKDYLEFKKGFTRIHIPLDINEHALTSEEDVVYNMQKGEIWFIEGRKIHSAANFSKVKRINLVIDFAPDIPFEELFLNSENYQPNLIPKISQRTQLKEEELGYIKGLSKIINEMNFDDILSILSKIHFYRNVSSELVFGWLDEIATASNNYNIQRKAQEVTDLLIRKGPINN

SEQ ID NO: 173 - DNA, 831 bp, Artificial Sequence
  gene sequence of K123D+Y35W+I120V mutant
atggaatccaagatcatcggtaaagtcaacttcgaggagcatctgctggataaagagctgaaactgatcgacactttcgagttcaacgacagctacagcgaatgggcttctggtatttggaagacttgcatgctgtggaaccgttctggtcagaaagatgaccatctgtctattgaacatgatacctacgtgaaacctactgaatacggcaaacagctggcatacgtaaacgaaatcatcgctaacacctttaagaaagaacacatcaagacggtgcgtctgttcatgtgtatcaacggcctgatcatcccacacaaagactacctggaattcaagaaaggcttcacccgtatccacgtgccgctggatatcaacgaacacgcactgacctctgaagaagatgttgtttacaacatgcagaaaggtgaaatttggttcatcgaaggccgtaaaatccacagcgctgccaatttcagcaaagtgaaacgtatcaacctggtcatcgacttcgcgccggatattccgtttgaagaactgttcctgaattctgagaactatcaaccgaacctgatcccgaaaatctctcaacgtacccagctgaaagaagaagagctgggttatatcaaaggtctgtctaaaattatcaatgaaatgaactttgacgacatcctgtccattctgagcaaaattcacttctatcgcaacgtttcctccgaactggtttttggctggctggacgaaattgccacggcgtccaacaactataacattcagcgcaaagcgcaggaagtaaccgatctgctgattcgcaaaggcccgattaataactaa

SEQ ID NO: 174 - protein, 276 aa, Artificial Sequence
  amino acid sequence of K123D+Y35W+I120V mutant
MESKIIGKVNFEEHLLDKELKLIDTFEFNDSYSEWASGIWKTCMLWNRSGQKDDHLSIEHDTYVKPTEYGKQLAYVNEIIANTFKKEHIKTVRLFMCINGLIIPHKDYLEFKKGFTRIHVPLDINEHALTSEEDVVYNMQKGEIWFIEGRKIHSAANFSKVKRINLVIDFAPDIPFEELFLNSENYQPNLIPKISQRTQLKEEELGYIKGLSKIINEMNFDDILSILSKIHFYRNVSSELVFGWLDEIATASNNYNIQRKAQEVTDLLIRKGPINN

SEQ ID NO: 175 - DNA, 831 bp, Artificial Sequence
  gene sequence of E27K+Y35W mutant
atggaatccaagatcatcggtaaagtcaacttcgaggagcatctgctggataaagagctgaaactgatcgacactttcaaattcaacgacagctacagcgaatgggcttctggtatttggaagacttgcatgctgtggaaccgttctggtcagaaagatgaccatctgtctattgaacatgatacctacgtgaaacctactgaatacggcaaacagctggcatacgtaaacgaaatcatcgctaacacctttaagaaagaacacatcaagacggtgcgtctgttcatgtgtatcaacggcctgatcatcccacacaaagactacctggaattcaagaaaggcttcacccgtatccacatcccgctgaaaatcaacgaacacgcactgacctctgaagaagatgttgtttacaacatgcagaaaggtgaaatttggttcatcgaaggccgtaaaatccacagcgctgccaatttcagcaaagtgaaacgtatcaacctggtcatcgacttcgcgccggatattccgtttgaagaactgttcctgaattctgagaactatcaaccgaacctgatcccgaaaatctctcaacgtacccagctgaaagaagaagagctgggttatatcaaaggtctgtctaaaattatcaatgaaatgaactttgacgacatcctgtccattctgagcaaaattcacttctatcgcaacgtttcctccgaactggtttttggctggctggacgaaattgccacggcgtccaacaactataacattcagcgcaaagcgcaggaagtaaccgatctgctgattcgcaaaggcccgattaataactaa

SEQ ID NO: 176 - protein, 276 aa, Artificial Sequence
  amino acid sequence of E27K+Y35W mutant
MESKIIGKVNFEEHLLDKELKLIDTFKFNDSYSEWASGIWKTCMLWNRSGQKDDHLSIEHDTYVKPTEYGKQLAYVNEIIANTFKKEHIKTVRLFMCINGLIIPHKDYLEFKKGFTRIHIPLKINEHALTSEEDVVYNMQKGEIWFIEGRKIHSAANFSKVKRINLVIDFAPDIPFEELFLNSENYQPNLIPKISQRTQLKEEELGYIKGLSKIINEMNFDDILSILSKIHFYRNVSSELVFGWLDEIATASNNYNIQRKAQEVTDLLIRKGPINN

SEQ ID NO: 177 - DNA, 831 bp, Artificial Sequence
  gene sequence of I39R+Y35W mutant
atggaatccaagatcatcggtaaagtcaacttcgaggagcatctgctggataaagagctgaaactgatcgacactttcgagttcaacgacagctacagcgaatgggcttctggtcgttggaagacttgcatgctgtggaaccgttctggtcagaaagatgaccatctgtctattgaacatgatacctacgtgaaacctactgaatacggcaaacagctggcatacgtaaacgaaatcatcgctaacacctttaagaaagaacacatcaagacggtgcgtctgttcatgtgtatcaacggcctgatcatcccacacaaagactacctggaattcaagaaaggcttcacccgtatccacatcccgctgaaaatcaacgaacacgcactgacctctgaagaagatgttgtttacaacatgcagaaaggtgaaatttggttcatcgaaggccgtaaaatccacagcgctgccaatttcagcaaagtgaaacgtatcaacctggtcatcgacttcgcgccggatattccgtttgaagaactgttcctgaattctgagaactatcaaccgaacctgatcccgaaaatctctcaacgtacccagctgaaagaagaagagctgggttatatcaaaggtctgtctaaaattatcaatgaaatgaactttgacgacatcctgtccattctgagcaaaattcacttctatcgcaacgtttcctccgaactggtttttggctggctggacgaaattgccacggcgtccaacaactataacattcagcgcaaagcgcaggaagtaaccgatctgctgattcgcaaaggcccgattaataactaa

SEQ ID NO: 178 - protein, 276 aa, Artificial Sequence
  amino acid sequence of I39R+Y35W mutant
MESKIIGKVNFEEHLLDKELKLIDTFEFNDSYSEWASGRWKTCMLWNRSGQKDDHLSIEHDTYVKPTEYGKQLAYVNEIIANTFKKEHIKTVRLFMCINGLIIPHKDYLEFKKGFTRIHIPLKINEHALTSEEDVVYNMQKGEIWFIEGRKIHSAANFSKVKRINLVIDFAPDIPFEELFLNSENYQPNLIPKISQRTQLKEEELGYIKGLSKIINEMNFDDILSILSKIHFYRNVSSELVFGWLDEIATASNNYNIQRKAQEVTDLLIRKGPINN

SEQ ID NO: 179 - DNA, 831 bp, Artificial Sequence
  gene sequence of S37C+I223V mutant
atggaatccaagatcatcggtaaagtcaacttcgaggagcatctgctggataaagagctgaaactgatcgacactttcgagttcaacgacagctacagcgaatacgcttgtggtatttggaagacttgcatgctgtggaaccgttctggtcagaaagatgaccatctgtctattgaacatgatacctacgtgaaacctactgaatacggcaaacagctggcatacgtaaacgaaatcatcgctaacacctttaagaaagaacacatcaagacggtgcgtctgttcatgtgtatcaacggcctgatcatcccacacaaagactacctggaattcaagaaaggcttcacccgtatccacatcccgctgaaaatcaacgaacacgcactgacctctgaagaagatgttgtttacaacatgcagaaaggtgaaatttggttcatcgaaggccgtaaaatccacagcgctgccaatttcagcaaagtgaaacgtatcaacctggtcatcgacttcgcgccggatattccgtttgaagaactgttcctgaattctgagaactatcaaccgaacctgatcccgaaaatctctcaacgtacccagctgaaagaagaagagctgggttatatcaaaggtctgtctaaaattatcaatgaaatgaactttgacgacgttctgtccattctgagcaaaattcacttctatcgcaacgtttcctccgaactggtttttggctggctggacgaaattgccacggcgtccaacaactataacattcagcgcaaagcgcaggaagtaaccgatctgctgattcgcaaaggcccgattaataactaa

SEQ ID NO: 180 - protein, 276 aa, Artificial Sequence
  amino acid sequence of S37C+I223V mutant
MESKIIGKVNFEEHLLDKELKLIDTFEFNDSYSEYACGIWKTCMLWNRSGQKDDHLSIEHDTYVKPTEYGKQLAYVNEIIANTFKKEHIKTVRLFMCINGLIIPHKDYLEFKKGFTRIHIPLKINEHALTSEEDVVYNMQKGEIWFIEGRKIHSAANFSKVKRINLVIDFAPDIPFEELFLNSENYQPNLIPKISQRTQLKEEELGYIKGLSKIINEMNFDDVLSILSKIHFYRNVSSELVFGWLDEIATASNNYNIQRKAQEVTDLLIRKGPINN

SEQ ID NO: 181 - DNA, 831 bp, Artificial Sequence
  gene sequence of E27K+I39K+Y35W mutant
atggaatccaagatcatcggtaaagtcaacttcgaggagcatctgctggataaagagctgaaactgatcgacactttcaaattcaacgacagctacagcgaatgggcttctggtaaatggaagacttgcatgctgtggaaccgttctggtcagaaagatgaccatctgtctattgaacatgatacctacgtgaaacctactgaatacggcaaacagctggcatacgtaaacgaaatcatcgctaacacctttaagaaagaacacatcaagacggtgcgtctgttcatgtgtatcaacggcctgatcatcccacacaaagactacctggaattcaagaaaggcttcacccgtatccacatcccgctgaaaatcaacgaacacgcactgacctctgaagaagatgttgtttacaacatgcagaaaggtgaaatttggttcatcgaaggccgtaaaatccacagcgctgccaatttcagcaaagtgaaacgtatcaacctggtcatcgacttcgcgccggatattccgtttgaagaactgttcctgaattctgagaactatcaaccgaacctgatcccgaaaatctctcaacgtacccagctgaaagaagaagagctgggttatatcaaaggtctgtctaaaattatcaatgaaatgaactttgacgacatcctgtccattctgagcaaaattcacttctatcgcaacgtttcctccgaactggtttttggctggctggacgaaattgccacggcgtccaacaactataacattcagcgcaaagcgcaggaagtaaccgatctgctgattcgcaaaggcccgattaataactaa

SEQ ID NO: 182 - protein, 276 aa, Artificial Sequence
  amino acid sequence of E27K+I39K+Y35W mutant
MESKIIGKVNFEEHLLDKELKLIDTFKFNDSYSEWASGKWKTCMLWNRSGQKDDHLSIEHDTYVKPTEYGKQLAYVNEIIANTFKKEHIKTVRLFMCINGLIIPHKDYLEFKKGFTRIHIPLKINEHALTSEEDVVYNMQKGEIWFIEGRKIHSAANFSKVKRINLVIDFAPDIPFEELFLNSENYQPNLIPKISQRTQLKEEELGYIKGLSKIINEMNFDDILSILSKIHFYRNVSSELVFGWLDEIATASNNYNIQRKAQEVTDLLIRKGPINN

SEQ ID NO: 183 - DNA, 831 bp, Artificial Sequence
  gene sequence of E27K+S37C+I39K+I98V+K123D+I223V mutant
atggaatccaagatcatcggtaaagtcaacttcgaggagcatctgctggataaagagctgaaactgatcgacactttcaaattcaacgacagctacagcgaatacgcttgtggtaaatggaagacttgcatgctgtggaaccgttctggtcagaaagatgaccatctgtctattgaacatgatacctacgtgaaacctactgaatacggcaaacagctggcatacgtaaacgaaatcatcgctaacacctttaagaaagaacacatcaagacggtgcgtctgttcatgtgtgttaacggcctgatcatcccacacaaagactacctggaattcaagaaaggcttcacccgtatccacatcccgctggatatcaacgaacacgcactgacctctgaagaagatgttgtttacaacatgcagaaaggtgaaatttggttcatcgaaggccgtaaaatccacagcgctgccaatttcagcaaagtgaaacgtatcaacctggtcatcgacttcgcgccggatattccgtttgaagaactgttcctgaattctgagaactatcaaccgaacctgatcccgaaaatctctcaacgtacccagctgaaagaagaagagctgggttatatcaaaggtctgtctaaaattatcaatgaaatgaactttgacgacgttctgtccattctgagcaaaattcacttctatcgcaacgtttcctccgaactggtttttggctggctggacgaaattgccacggcgtccaacaactataacattcagcgcaaagcgcaggaagtaaccgatctgctgattcgcaaaggcccgattaataactaa

SEQ ID NO: 184 - protein, 276 aa, Artificial Sequence
  amino acid sequence of E27K+S37C+I39K+I98V+K123D+I223V mutant
MESKIIGKVNFEEHLLDKELKLIDTFKFNDSYSEYACGKWKTCMLWNRSGQKDDHLSIEHDTYVKPTEYGKQLAYVNEIIANTFKKEHIKTVRLFMCVNGLIIPHKDYLEFKKGFTRIHIPLDINEHALTSEEDVVYNMQKGEIWFIEGRKIHSAANFSKVKRINLVIDFAPDIPFEELFLNSENYQPNLIPKISQRTQLKEEELGYIKGLSKIINEMNFDDVLSILSKIHFYRNVSSELVFGWLDEIATASNNYNIQRKAQEVTDLLIRKGPINN

SEQ ID NO: 185 - DNA, 831 bp, Artificial Sequence
  gene sequence of E27K+I39K+K123D+N165H mutant
atggaatccaagatcatcggtaaagtcaacttcgaggagcatctgctggataaagagctgaaactgatcgacactttcaaattcaacgacagctacagcgaatacgcttctggtaaatggaagacttgcatgctgtggaaccgttctggtcagaaagatgaccatctgtctattgaacatgatacctacgtgaaacctactgaatacggcaaacagctggcatacgtaaacgaaatcatcgctaacacctttaagaaagaacacatcaagacggtgcgtctgttcatgtgtatcaacggcctgatcatcccacacaaagactacctggaattcaagaaaggcttcacccgtatccacatcccgctggatatcaacgaacacgcactgacctctgaagaagatgttgtttacaacatgcagaaaggtgaaatttggttcatcgaaggccgtaaaatccacagcgctgccaatttcagcaaagtgaaacgtatccatctggtcatcgacttcgcgccggatattccgtttgaagaactgttcctgaattctgagaactatcaaccgaacctgatcccgaaaatctctcaacgtacccagctgaaagaagaagagctgggttatatcaaaggtctgtctaaaattatcaatgaaatgaactttgacgacatcctgtccattctgagcaaaattcacttctatcgcaacgtttcctccgaactggtttttggctggctggacgaaattgccacggcgtccaacaactataacattcagcgcaaagcgcaggaagtaaccgatctgctgattcgcaaaggcccgattaataactaa

SEQ ID NO: 186 - protein, 276 aa, Artificial Sequence
  amino acid sequence of E27K+I39K+K123D+N165H mutant
MESKIIGKVNFEEHLLDKELKLIDTFKFNDSYSEYASGKWKTCMLWNRSGQKDDHLSIEHDTYVKPTEYGKQLAYVNEIIANTFKKEHIKTVRLFMCINGLIIPHKDYLEFKKGFTRIHIPLDINEHALTSEEDVVYNMQKGEIWFIEGRKIHSAANFSKVKRIHLVIDFAPDIPFEELFLNSENYQPNLIPKISQRTQLKEEELGYIKGLSKIINEMNFDDILSILSKIHFYRNVSSELVFGWLDEIATASNNYNIQRKAQEVTDLLIRKGPINN

SEQ ID NO: 187 - DNA, 831 bp, Artificial Sequence
  gene sequence of E27K+I39R+Y35W mutant
atggaatccaagatcatcggtaaagtcaacttcgaggagcatctgctggataaagagctgaaactgatcgacactttcaaattcaacgacagctacagcgaatgggcttctggtcgttggaagacttgcatgctgtggaaccgttctggtcagaaagatgaccatctgtctattgaacatgatacctacgtgaaacctactgaatacggcaaacagctggcatacgtaaacgaaatcatcgctaacacctttaagaaagaacacatcaagacggtgcgtctgttcatgtgtatcaacggcctgatcatcccacacaaagactacctggaattcaagaaaggcttcacccgtatccacatcccgctgaaaatcaacgaacacgcactgacctctgaagaagatgttgtttacaacatgcagaaaggtgaaatttggttcatcgaaggccgtaaaatccacagcgctgccaatttcagcaaagtgaaacgtatcaacctggtcatcgacttcgcgccggatattccgtttgaagaactgttcctgaattctgagaactatcaaccgaacctgatcccgaaaatctctcaacgtacccagctgaaagaagaagagctgggttatatcaaaggtctgtctaaaattatcaatgaaatgaactttgacgacatcctgtccattctgagcaaaattcacttctatcgcaacgtttcctccgaactggtttttggctggctggacgaaattgccacggcgtccaacaactataacattcagcgcaaagcgcaggaagtaaccgatctgctgattcgcaaaggcccgattaataactaa

SEQ ID NO: 188 - protein, 276 aa, Artificial Sequence
  amino acid sequence of E27K+I39R+Y35W mutant
MESKIIGKVNFEEHLLDKELKLIDTFKFNDSYSEWASGRWKTCMLWNRSGQKDDHLSIEHDTYVKPTEYGKQLAYVNEIIANTFKKEHIKTVRLFMCINGLIIPHKDYLEFKKGFTRIHIPLKINEHALTSEEDVVYNMQKGEIWFIEGRKIHSAANFSKVKRINLVIDFAPDIPFEELFLNSENYQPNLIPKISQRTQLKEEELGYIKGLSKIINEMNFDDILSILSKIHFYRNVSSELVFGWLDEIATASNNYNIQRKAQEVTDLLIRKGPINN

SEQ ID NO: 189 - DNA, 831 bp, Artificial Sequence
  gene sequence of S37C+I39K+N165H mutant
atggaatccaagatcatcggtaaagtcaacttcgaggagcatctgctggataaagagctgaaactgattatcactttcgagttcaacgacagctacagcgaatacgcttctggtatttggaagacttgcatgctgtggaaccgttctggtcagaaagatgaccatctgtctattgaacatgatacctacgtgaaacctactgaatacggcaaacagctggcatacgtaaacgaaatcatcgctaacacctttaagaaagaacacatcaagacggtgcgtctgttcatgtgtatcaacggcctgatcatcccacacaaagactacctggaattcaagaaaggcttcacccgtatccacatcccgctgaaaatcaacgaacacgcactgacctctgaagaagatgttgtttacaacatgcagaaaggtgaaatttggttcatcgaaggccgtaaaatccacagcgctgccaatttcggtaaagtgaaacgtatcgttctggtcatcgacttcgcgccggatattccgtttgaagaactgttcctgaattctgagaactatcaaccgaacctgatcccgaaaatctctcaacgtacccagctgaaagaagaagagctgggttatatcaaaggtctgtctaaaattatcaatgaaatgaactttgacgacatcctgtccattctgagcaaaattcacttctatcgcaacgtttcctccgaactggtttttggctggctggacgaaattgccacggcgtccaacaactataacattcagcgcaaagcgcaggaagtaaccgatctgctgattcgcaaaggcccgattaataactaa

SEQ ID NO: 190 - protein, 276 aa, Artificial Sequence
  amino acid sequence of S37C+I39K+N165H mutant
MESKIIGKVNFEEHLLDKELKLIITFEFNDSYSEYASGIWKTCMLWNRSGQKDDHLSIEHDTYVKPTEYGKQLAYVNEIIANTFKKEHIKTVRLFMCINGLIIPHKDYLEFKKGFTRIHIPLKINEHALTSEEDVVYNMQKGEIWFIEGRKIHSAANFGKVKRIVLVIDFAPDIPFEELFLNSENYQPNLIPKISQRTQLKEEELGYIKGLSKIINEMNFDDILSILSKIHFYRNVSSELVFGWLDEIATASNNYNIQRKAQEVTDLLIRKGPINN

SEQ ID NO: 191 - DNA, 831 bp, Artificial Sequence
  gene sequence of E27K+ I39K+D30S mutant
atggaatccaagatcatcggtaaagtcaacttcgaggagcatctgctggataaagagctgaaactgatcgacactttcaaattcaacagcagctacagcgaatacgcttctggtaaatggaagacttgcatgctgtggaaccgttctggtcagaaagatgaccatctgtctattgaacatgatacctacgtgaaacctactgaatacggcaaacagctggcatacgtaaacgaaatcatcgctaacacctttaagaaagaacacatcaagacggtgcgtctgttcatgtgtatcaacggcctgatcatcccacacaaagactacctggaattcaagaaaggcttcacccgtatccacatcccgctgaaaatcaacgaacacgcactgacctctgaagaagatgttgtttacaacatgcagaaaggtgaaatttggttcatcgaaggccgtaaaatccacagcgctgccaatttcagcaaagtgaaacgtatcaacctggtcatcgacttcgcgccggatattccgtttgaagaactgttcctgaattctgagaactatcaaccgaacctgatcccgaaaatctctcaacgtacccagctgaaagaagaagagctgggttatatcaaaggtctgtctaaaattatcaatgaaatgaactttgacgacatcctgtccattctgagcaaaattcacttctatcgcaacgtttcctccgaactggtttttggctggctggacgaaattgccacggcgtccaacaactataacattcagcgcaaagcgcaggaagtaaccgatctgctgattcgcaaaggcccgattaataactaa

SEQ ID NO: 192 - protein, 276 aa, Artificial Sequence
  amino acid sequence of E27K+ I39K+D30S mutant
MESKIIGKVNFEEHLLDKELKLIDTFKFNSSYSEYASGKWKTCMLWNRSGQKDDHLSIEHDTYVKPTEYGKQLAYVNEIIANTFKKEHIKTVRLFMCINGLIIPHKDYLEFKKGFTRIHIPLKINEHALTSEEDVVYNMQKGEIWFIEGRKIHSAANFSKVKRINLVIDFAPDIPFEELFLNSENYQPNLIPKISQRTQLKEEELGYIKGLSKIINEMNFDDILSILSKIHFYRNVSSELVFGWLDEIATASNNYNIQRKAQEVTDLLIRKGPINN

SEQ ID NO: 193 - DNA, 831 bp, Artificial Sequence
  gene sequence of E27K+I39K+E34N mutant
atggaatccaagatcatcggtaaagtcaacttcgaggagcatctgctggataaagagctgaaactgatcgacactttcaaattcaacgacagctacagcaattacgcttctggtaaatggaagacttgcatgctgtggaaccgttctggtcagaaagatgaccatctgtctattgaacatgatacctacgtgaaacctactgaatacggcaaacagctggcatacgtaaacgaaatcatcgctaacacctttaagaaagaacacatcaagacggtgcgtctgttcatgtgtatcaacggcctgatcatcccacacaaagactacctggaattcaagaaaggcttcacccgtatccacatcccgctgaaaatcaacgaacacgcactgacctctgaagaagatgttgtttacaacatgcagaaaggtgaaatttggttcatcgaaggccgtaaaatccacagcgctgccaatttcagcaaagtgaaacgtatcaacctggtcatcgacttcgcgccggatattccgtttgaagaactgttcctgaattctgagaactatcaaccgaacctgatcccgaaaatctctcaacgtacccagctgaaagaagaagagctgggttatatcaaaggtctgtctaaaattatcaatgaaatgaactttgacgacatcctgtccattctgagcaaaattcacttctatcgcaacgtttcctccgaactggtttttggctggctggacgaaattgccacggcgtccaacaactataacattcagcgcaaagcgcaggaagtaaccgatctgctgattcgcaaaggcccgattaataactaa

SEQ ID NO: 194 - protein, 276 aa, Artificial Sequence
  amino acid sequence of E27K+I39K+E34N mutant
MESKIIGKVNFEEHLLDKELKLIDTFKFNDSYSNYASGKWKTCMLWNRSGQKDDHLSIEHDTYVKPTEYGKQLAYVNEIIANTFKKEHIKTVRLFMCINGLIIPHKDYLEFKKGFTRIHIPLKINEHALTSEEDVVYNMQKGEIWFIEGRKIHSAANFSKVKRINLVIDFAPDIPFEELFLNSENYQPNLIPKISQRTQLKEEELGYIKGLSKIINEMNFDDILSILSKIHFYRNVSSELVFGWLDEIATASNNYNIQRKAQEVTDLLIRKGPINN

SEQ ID NO: 195 - DNA, 831 bp, Artificial Sequence
  gene sequence of E27K+I39K+E34G mutant
atggaatccaagatcatcggtaaagtcaacttcgaggagcatctgctggataaagagctgaaactgatcgacactttcaaattcaacgacagctacagcggttacgcttctggtaaatggaagacttgcatgctgtggaaccgttctggtcagaaagatgaccatctgtctattgaacatgatacctacgtgaaacctactgaatacggcaaacagctggcatacgtaaacgaaatcatcgctaacacctttaagaaagaacacatcaagacggtgcgtctgttcatgtgtatcaacggcctgatcatcccacacaaagactacctggaattcaagaaaggcttcacccgtatccacatcccgctgaaaatcaacgaacacgcactgacctctgaagaagatgttgtttacaacatgcagaaaggtgaaatttggttcatcgaaggccgtaaaatccacagcgctgccaatttcagcaaagtgaaacgtatcaacctggtcatcgacttcgcgccggatattccgtttgaagaactgttcctgaattctgagaactatcaaccgaacctgatcccgaaaatctctcaacgtacccagctgaaagaagaagagctgggttatatcaaaggtctgtctaaaattatcaatgaaatgaactttgacgacatcctgtccattctgagcaaaattcacttctatcgcaacgtttcctccgaactggtttttggctggctggacgaaattgccacggcgtccaacaactataacattcagcgcaaagcgcaggaagtaaccgatctgctgattcgcaaaggcccgattaataactaa

SEQ ID NO: 196 - protein, 276 aa, Artificial Sequence
  amino acid sequence of E27K+I39K+E34G mutant
MESKIIGKVNFEEHLLDKELKLIDTFKFNDSYSGYASGKWKTCMLWNRSGQKDDHLSIEHDTYVKPTEYGKQLAYVNEIIANTFKKEHIKTVRLFMCINGLIIPHKDYLEFKKGFTRIHIPLKINEHALTSEEDVVYNMQKGEIWFIEGRKIHSAANFSKVKRINLVIDFAPDIPFEELFLNSENYQPNLIPKISQRTQLKEEELGYIKGLSKIINEMNFDDILSILSKIHFYRNVSSELVFGWLDEIATASNNYNIQRKAQEVTDLLIRKGPINN

SEQ ID NO: 197 - DNA, 831 bp, Artificial Sequence
  gene sequence of E27K+I39K+S37W mutant
atggaatccaagatcatcggtaaagtcaacttcgaggagcatctgctggataaagagctgaaactgatcgacactttcaaattcaacgacagctacagcgaatacgcttggggtaaatggaagacttgcatgctgtggaaccgttctggtcagaaagatgaccatctgtctattgaacatgatacctacgtgaaacctactgaatacggcaaacagctggcatacgtaaacgaaatcatcgctaacacctttaagaaagaacacatcaagacggtgcgtctgttcatgtgtatcaacggcctgatcatcccacacaaagactacctggaattcaagaaaggcttcacccgtatccacatcccgctgaaaatcaacgaacacgcactgacctctgaagaagatgttgtttacaacatgcagaaaggtgaaatttggttcatcgaaggccgtaaaatccacagcgctgccaatttcagcaaagtgaaacgtatcaacctggtcatcgacttcgcgccggatattccgtttgaagaactgttcctgaattctgagaactatcaaccgaacctgatcccgaaaatctctcaacgtacccagctgaaagaagaagagctgggttatatcaaaggtctgtctaaaattatcaatgaaatgaactttgacgacatcctgtccattctgagcaaaattcacttctatcgcaacgtttcctccgaactggtttttggctggctggacgaaattgccacggcgtccaacaactataacattcagcgcaaagcgcaggaagtaaccgatctgctgattcgcaaaggcccgattaataactaa

SEQ ID NO: 198 - protein, 276 aa, Artificial Sequence
  amino acid sequence of E27K+I39K+S37W mutant
MESKIIGKVNFEEHLLDKELKLIDTFKFNDSYSEYAWGKWKTCMLWNRSGQKDDHLSIEHDTYVKPTEYGKQLAYVNEIIANTFKKEHIKTVRLFMCINGLIIPHKDYLEFKKGFTRIHIPLKINEHALTSEEDVVYNMQKGEIWFIEGRKIHSAANFSKVKRINLVIDFAPDIPFEELFLNSENYQPNLIPKISQRTQLKEEELGYIKGLSKIINEMNFDDILSILSKIHFYRNVSSELVFGWLDEIATASNNYNIQRKAQEVTDLLIRKGPINN

SEQ ID NO: 199 - DNA, 831 bp, Artificial Sequence
  gene sequence of E27K+I39K+S37E mutant
atggaatccaagatcatcggtaaagtcaacttcgaggagcatctgctggataaagagctgaaactgatcgacactttcaaattcaacgacagctacagcgaatacgctgaaggtaaatggaagacttgcatgctgtggaaccgttctggtcagaaagatgaccatctgtctattgaacatgatacctacgtgaaacctactgaatacggcaaacagctggcatacgtaaacgaaatcatcgctaacacctttaagaaagaacacatcaagacggtgcgtctgttcatgtgtatcaacggcctgatcatcccacacaaagactacctggaattcaagaaaggcttcacccgtatccacatcccgctgaaaatcaacgaacacgcactgacctctgaagaagatgttgtttacaacatgcagaaaggtgaaatttggttcatcgaaggccgtaaaatccacagcgctgccaatttcagcaaagtgaaacgtatcaacctggtcatcgacttcgcgccggatattccgtttgaagaactgttcctgaattctgagaactatcaaccgaacctgatcccgaaaatctctcaacgtacccagctgaaagaagaagagctgggttatatcaaaggtctgtctaaaattatcaatgaaatgaactttgacgacatcctgtccattctgagcaaaattcacttctatcgcaacgtttcctccgaactggtttttggctggctggacgaaattgccacggcgtccaacaactataacattcagcgcaaagcgcaggaagtaaccgatctgctgattcgcaaaggcccgattaataactaa

SEQ ID NO: 200 - protein, 276 aa, Artificial Sequence
  amino acid sequence of E27K+I39K+S37E mutant
MESKIIGKVNFEEHLLDKELKLIDTFKFNDSYSEYAEGKWKTCMLWNRSGQKDDHLSIEHDTYVKPTEYGKQLAYVNEIIANTFKKEHIKTVRLFMCINGLIIPHKDYLEFKKGFTRIHIPLKINEHALTSEEDVVYNMQKGEIWFIEGRKIHSAANFSKVKRINLVIDFAPDIPFEELFLNSENYQPNLIPKISQRTQLKEEELGYIKGLSKIINEMNFDDILSILSKIHFYRNVSSELVFGWLDEIATASNNYNIQRKAQEVTDLLIRKGPINN

SEQ ID NO: 201 - DNA, 831 bp, Artificial Sequence
  gene sequence of E27K+I39K+Y35K mutant
atggaatccaagatcatcggtaaagtcaacttcgaggagcatctgctggataaagagctgaaactgatcgacactttcaaattcaacgacagctacagcgaaaaagcttctggtaaatggaagacttgcatgctgtggaaccgttctggtcagaaagatgaccatctgtctattgaacatgatacctacgtgaaacctactgaatacggcaaacagctggcatacgtaaacgaaatcatcgctaacacctttaagaaagaacacatcaagacggtgcgtctgttcatgtgtatcaacggcctgatcatcccacacaaagactacctggaattcaagaaaggcttcacccgtatccacatcccgctgaaaatcaacgaacacgcactgacctctgaagaagatgttgtttacaacatgcagaaaggtgaaatttggttcatcgaaggccgtaaaatccacagcgctgccaatttcagcaaagtgaaacgtatcaacctggtcatcgacttcgcgccggatattccgtttgaagaactgttcctgaattctgagaactatcaaccgaacctgatcccgaaaatctctcaacgtacccagctgaaagaagaagagctgggttatatcaaaggtctgtctaaaattatcaatgaaatgaactttgacgacatcctgtccattctgagcaaaattcacttctatcgcaacgtttcctccgaactggtttttggctggctggacgaaattgccacggcgtccaacaactataacattcagcgcaaagcgcaggaagtaaccgatctgctgattcgcaaaggcccgattaataactaa

SEQ ID NO: 202 - protein, 276 aa, Artificial Sequence
  amino acid sequence of E27K+I39K+Y35K mutant
MESKIIGKVNFEEHLLDKELKLIDTFKFNDSYSEKASGKWKTCMLWNRSGQKDDHLSIEHDTYVKPTEYGKQLAYVNEIIANTFKKEHIKTVRLFMCINGLIIPHKDYLEFKKGFTRIHIPLKINEHALTSEEDVVYNMQKGEIWFIEGRKIHSAANFSKVKRINLVIDFAPDIPFEELFLNSENYQPNLIPKISQRTQLKEEELGYIKGLSKIINEMNFDDILSILSKIHFYRNVSSELVFGWLDEIATASNNYNIQRKAQEVTDLLIRKGPINN

SEQ ID NO: 203 - DNA, 831 bp, Artificial Sequence
  gene sequence of E27K+I39K+S37N mutant
atggaatccaagatcatcggtaaagtcaacttcgaggagcatctgctggataaagagctgaaactgatcgacactttcaaattcaacgacagctacagcgaatacgctaatggtaaatggaagacttgcatgctgtggaaccgttctggtcagaaagatgaccatctgtctattgaacatgatacctacgtgaaacctactgaatacggcaaacagctggcatacgtaaacgaaatcatcgctaacacctttaagaaagaacacatcaagacggtgcgtctgttcatgtgtatcaacggcctgatcatcccacacaaagactacctggaattcaagaaaggcttcacccgtatccacatcccgctgaaaatcaacgaacacgcactgacctctgaagaagatgttgtttacaacatgcagaaaggtgaaatttggttcatcgaaggccgtaaaatccacagcgctgccaatttcagcaaagtgaaacgtatcaacctggtcatcgacttcgcgccggatattccgtttgaagaactgttcctgaattctgagaactatcaaccgaacctgatcccgaaaatctctcaacgtacccagctgaaagaagaagagctgggttatatcaaaggtctgtctaaaattatcaatgaaatgaactttgacgacatcctgtccattctgagcaaaattcacttctatcgcaacgtttcctccgaactggtttttggctggctggacgaaattgccacggcgtccaacaactataacattcagcgcaaagcgcaggaagtaaccgatctgctgattcgcaaaggcccgattaataactaa

SEQ ID NO: 204 - protein, 276 aa, Artificial Sequence
  amino acid sequence of E27K+I39K+S37N mutant
MESKIIGKVNFEEHLLDKELKLIDTFKFNDSYSEYANGKWKTCMLWNRSGQKDDHLSIEHDTYVKPTEYGKQLAYVNEIIANTFKKEHIKTVRLFMCINGLIIPHKDYLEFKKGFTRIHIPLKINEHALTSEEDVVYNMQKGEIWFIEGRKIHSAANFSKVKRINLVIDFAPDIPFEELFLNSENYQPNLIPKISQRTQLKEEELGYIKGLSKIINEMNFDDILSILSKIHFYRNVSSELVFGWLDEIATASNNYNIQRKAQEVTDLLIRKGPINN

SEQ ID NO: 205 - DNA, 831 bp, Artificial Sequence
  gene sequence of E27K+I39K+K123Q mutant
atggaatccaagatcatcggtaaagtcaacttcgaggagcatctgctggataaagagctgaaactgatcgacactttcaaattcaacgacagctacagcgaatacgcttctggtaaatggaagacttgcatgctgtggaaccgttctggtcagaaagatgaccatctgtctattgaacatgatacctacgtgaaacctactgaatacggcaaacagctggcatacgtaaacgaaatcatcgctaacacctttaagaaagaacacatcaagacggtgcgtctgttcatgtgtatcaacggcctgatcatcccacacaaagactacctggaattcaagaaaggcttcacccgtatccacatcccgctgcagatcaacgaacacgcactgacctctgaagaagatgttgtttacaacatgcagaaaggtgaaatttggttcatcgaaggccgtaaaatccacagcgctgccaatttcagcaaagtgaaacgtatcaacctggtcatcgacttcgcgccggatattccgtttgaagaactgttcctgaattctgagaactatcaaccgaacctgatcccgaaaatctctcaacgtacccagctgaaagaagaagagctgggttatatcaaaggtctgtctaaaattatcaatgaaatgaactttgacgacatcctgtccattctgagcaaaattcacttctatcgcaacgtttcctccgaactggtttttggctggctggacgaaattgccacggcgtccaacaactataacattcagcgcaaagcgcaggaagtaaccgatctgctgattcgcaaaggcccgattaataactaa

SEQ ID NO: 206 - protein, 276 aa, Artificial Sequence
  amino acid sequence of E27K+I39K+K123Q mutant
MESKIIGKVNFEEHLLDKELKLIDTFKFNDSYSEYASGKWKTCMLWNRSGQKDDHLSIEHDTYVKPTEYGKQLAYVNEIIANTFKKEHIKTVRLFMCINGLIIPHKDYLEFKKGFTRIHIPLQINEHALTSEEDVVYNMQKGEIWFIEGRKIHSAANFSKVKRINLVIDFAPDIPFEELFLNSENYQPNLIPKISQRTQLKEEELGYIKGLSKIINEMNFDDILSILSKIHFYRNVSSELVFGWLDEIATASNNYNIQRKAQEVTDLLIRKGPINN

SEQ ID NO: 207 - DNA, 831 bp, Artificial Sequence
  gene sequence of E27K+I39K+K123S mutant
atggaatccaagatcatcggtaaagtcaacttcgaggagcatctgctggataaagagctgaaactgatcgacactttcaaattcaacgacagctacagcgaatacgcttctggtaaatggaagacttgcatgctgtggaaccgttctggtcagaaagatgaccatctgtctattgaacatgatacctacgtgaaacctactgaatacggcaaacagctggcatacgtaaacgaaatcatcgctaacacctttaagaaagaacacatcaagacggtgcgtctgttcatgtgtatcaacggcctgatcatcccacacaaagactacctggaattcaagaaaggcttcacccgtatccacatcccgctgagcatcaacgaacacgcactgacctctgaagaagatgttgtttacaacatgcagaaaggtgaaatttggttcatcgaaggccgtaaaatccacagcgctgccaatttcagcaaagtgaaacgtatcaacctggtcatcgacttcgcgccggatattccgtttgaagaactgttcctgaattctgagaactatcaaccgaacctgatcccgaaaatctctcaacgtacccagctgaaagaagaagagctgggttatatcaaaggtctgtctaaaattatcaatgaaatgaactttgacgacatcctgtccattctgagcaaaattcacttctatcgcaacgtttcctccgaactggtttttggctggctggacgaaattgccacggcgtccaacaactataacattcagcgcaaagcgcaggaagtaaccgatctgctgattcgcaaaggcccgattaataactaa

SEQ ID NO: 208 - protein, 276 aa, Artificial Sequence
  amino acid sequence of E27K+I39K+K123S mutant
MESKIIGKVNFEEHLLDKELKLIDTFKFNDSYSEYASGKWKTCMLWNRSGQKDDHLSIEHDTYVKPTEYGKQLAYVNEIIANTFKKEHIKTVRLFMCINGLIIPHKDYLEFKKGFTRIHIPLSINEHALTSEEDVVYNMQKGEIWFIEGRKIHSAANFSKVKRINLVIDFAPDIPFEELFLNSENYQPNLIPKISQRTQLKEEELGYIKGLSKIINEMNFDDILSILSKIHFYRNVSSELVFGWLDEIATASNNYNIQRKAQEVTDLLIRKGPINN

SEQ ID NO: 209 - DNA, 831 bp, Artificial Sequence
  gene sequence of E27K+I39K+K106Q+K112E mutant
atggaatccaagatcatcggtaaagtcaacttcgaggagcatctgctggataaagagctgaaactgatcgacactttcaaattcaacgacagctacagcgaatacgcttctggtaaatggaagacttgcatgctgtggaaccgttctggtcagaaagatgaccatctgtctattgaacatgatacctacgtgaaacctactgaatacggcaaacagctggcatacgtaaacgaaatcatcgctaacacctttaagaaagaacacatcaagacggtgcgtctgttcatgtgtatcaacggcctgatcatcccacaccaggactacctggaattcgaaaaaggcttcacccgtatccacatcccgctgaaaatcaacgaacacgcactgacctctgaagaagatgttgtttacaacatgcagaaaggtgaaatttggttcatcgaaggccgtaaaatccacagcgctgccaatttcagcaaagtgaaacgtatcaacctggtcatcgacttcgcgccggatattccgtttgaagaactgttcctgaattctgagaactatcaaccgaacctgatcccgaaaatctctcaacgtacccagctgaaagaagaagagctgggttatatcaaaggtctgtctaaaattatcaatgaaatgaactttgacgacatcctgtccattctgagcaaaattcacttctatcgcaacgtttcctccgaactggtttttggctggctggacgaaattgccacggcgtccaacaactataacattcagcgcaaagcgcaggaagtaaccgatctgctgattcgcaaaggcccgattaataactaa

SEQ ID NO: 210 - protein, 276 aa, Artificial Sequence
  amino acid sequence of E27K+I39K+K106Q+K112E mutant
MESKIIGKVNFEEHLLDKELKLIDTFKFNDSYSEYASGKWKTCMLWNRSGQKDDHLSIEHDTYVKPTEYGKQLAYVNEIIANTFKKEHIKTVRLFMCINGLIIPHQDYLEFEKGFTRIHIPLKINEHALTSEEDVVYNMQKGEIWFIEGRKIHSAANFSKVKRINLVIDFAPDIPFEELFLNSENYQPNLIPKISQRTQLKEEELGYIKGLSKIINEMNFDDILSILSKIHFYRNVSSELVFGWLDEIATASNNYNIQRKAQEVTDLLIRKGPINN

SEQ ID NO: 211 - DNA, 831 bp, Artificial Sequence
  gene sequence of I98V+E27K+I39K mutant
atggaatccaagatcatcggtaaagtcaacttcgaggagcatctgctggataaagagctgaaactgatcgacactttcaaattcaacgacagctacagcgaatacgcttctggtaaatggaagacttgcatgctgtggaaccgttctggtcagaaagatgaccatctgtctattgaacatgatacctacgtgaaacctactgaatacggcaaacagctggcatacgtaaacgaaatcatcgctaacacctttaagaaagaacacatcaagacggtgcgtctgttcatgtgtgttaacggcctgatcatcccacacaaagactacctggaattcaagaaaggcttcacccgtatccacatcccgctgaaaatcaacgaacacgcactgacctctgaagaagatgttgtttacaacatgcagaaaggtgaaatttggttcatcgaaggccgtaaaatccacagcgctgccaatttcagcaaagtgaaacgtatcaacctggtcatcgacttcgcgccggatattccgtttgaagaactgttcctgaattctgagaactatcaaccgaacctgatcccgaaaatctctcaacgtacccagctgaaagaagaagagctgggttatatcaaaggtctgtctaaaattatcaatgaaatgaactttgacgacatcctgtccattctgagcaaaattcacttctatcgcaacgtttcctccgaactggtttttggctggctggacgaaattgccacggcgtccaacaactataacattcagcgcaaagcgcaggaagtaaccgatctgctgattcgcaaaggcccgattaataactaa

SEQ ID NO: 212 - protein, 276 aa, Artificial Sequence
  amino acid sequence of I98V+E27K+I39K mutant
MESKIIGKVNFEEHLLDKELKLIDTFKFNDSYSEYASGKWKTCMLWNRSGQKDDHLSIEHDTYVKPTEYGKQLAYVNEIIANTFKKEHIKTVRLFMCVNGLIIPHKDYLEFKKGFTRIHIPLKINEHALTSEEDVVYNMQKGEIWFIEGRKIHSAANFSKVKRINLVIDFAPDIPFEELFLNSENYQPNLIPKISQRTQLKEEELGYIKGLSKIINEMNFDDILSILSKIHFYRNVSSELVFGWLDEIATASNNYNIQRKAQEVTDLLIRKGPINN

SEQ ID NO: 213 - DNA, 831 bp, Artificial Sequence
  gene sequence of E27K+I39K+I118F mutant
atggaatccaagatcatcggtaaagtcaacttcgaggagcatctgctggataaagagctgaaactgatcgacactttcaaattcaacgacagctacagcgaatacgcttctggtaaatggaagacttgcatgctgtggaaccgttctggtcagaaagatgaccatctgtctattgaacatgatacctacgtgaaacctactgaatacggcaaacagctggcatacgtaaacgaaatcatcgctaacacctttaagaaagaacacatcaagacggtgcgtctgttcatgtgtatcaacggcctgatcatcccacacaaagactacctggaattcaagaaaggcttcacccgttttcacatcccgctgaaaatcaacgaacacgcactgacctctgaagaagatgttgtttacaacatgcagaaaggtgaaatttggttcatcgaaggccgtaaaatccacagcgctgccaatttcagcaaagtgaaacgtatcaacctggtcatcgacttcgcgccggatattccgtttgaagaactgttcctgaattctgagaactatcaaccgaacctgatcccgaaaatctctcaacgtacccagctgaaagaagaagagctgggttatatcaaaggtctgtctaaaattatcaatgaaatgaactttgacgacatcctgtccattctgagcaaaattcacttctatcgcaacgtttcctccgaactggtttttggctggctggacgaaattgccacggcgtccaacaactataacattcagcgcaaagcgcaggaagtaaccgatctgctgattcgcaaaggcccgattaataactaa

SEQ ID NO: 214 - protein, 276 aa, Artificial Sequence
  amino acid sequence of E27K+I39K+I118F mutant
MESKIIGKVNFEEHLLDKELKLIDTFKFNDSYSEYASGKWKTCMLWNRSGQKDDHLSIEHDTYVKPTEYGKQLAYVNEIIANTFKKEHIKTVRLFMCINGLIIPHKDYLEFKKGFTRFHIPLKINEHALTSEEDVVYNMQKGEIWFIEGRKIHSAANFSKVKRINLVIDFAPDIPFEELFLNSENYQPNLIPKISQRTQLKEEELGYIKGLSKIINEMNFDDILSILSKIHFYRNVSSELVFGWLDEIATASNNYNIQRKAQEVTDLLIRKGPINN

SEQ ID NO: 215 - DNA, 831 bp, Artificial Sequence
  gene sequence of E27K+I39K+S37T mutant
atggaatccaagatcatcggtaaagtcaacttcgaggagcatctgctggataaagagctgaaactgatcgacactttcaaattcaacgacagctacagcgaatacgctaccggtaaatggaagacttgcatgctgtggaaccgttctggtcagaaagatgaccatctgtctattgaacatgatacctacgtgaaacctactgaatacggcaaacagctggcatacgtaaacgaaatcatcgctaacacctttaagaaagaacacatcaagacggtgcgtctgttcatgtgtatcaacggcctgatcatcccacacaaagactacctggaattcaagaaaggcttcacccgtatccacatcccgctgaaaatcaacgaacacgcactgacctctgaagaagatgttgtttacaacatgcagaaaggtgaaatttggttcatcgaaggccgtaaaatccacagcgctgccaatttcagcaaagtgaaacgtatcaacctggtcatcgacttcgcgccggatattccgtttgaagaactgttcctgaattctgagaactatcaaccgaacctgatcccgaaaatctctcaacgtacccagctgaaagaagaagagctgggttatatcaaaggtctgtctaaaattatcaatgaaatgaactttgacgacatcctgtccattctgagcaaaattcacttctatcgcaacgtttcctccgaactggtttttggctggctggacgaaattgccacggcgtccaacaactataacattcagcgcaaagcgcaggaagtaaccgatctgctgattcgcaaaggcccgattaataactaa

SEQ ID NO: 216 - protein, 276 aa, Artificial Sequence
  amino acid sequence of E27K+I39K+S37T mutant
MESKIIGKVNFEEHLLDKELKLIDTFKFNDSYSEYATGKWKTCMLWNRSGQKDDHLSIEHDTYVKPTEYGKQLAYVNEIIANTFKKEHIKTVRLFMCINGLIIPHKDYLEFKKGFTRIHIPLKINEHALTSEEDVVYNMQKGEIWFIEGRKIHSAANFSKVKRINLVIDFAPDIPFEELFLNSENYQPNLIPKISQRTQLKEEELGYIKGLSKIINEMNFDDILSILSKIHFYRNVSSELVFGWLDEIATASNNYNIQRKAQEVTDLLIRKGPINN

SEQ ID NO: 217 - DNA, 831 bp, Artificial Sequence
  gene sequence of E27K+I39K+K123I mutant
atggaatccaagatcatcggtaaagtcaacttcgaggagcatctgctggataaagagctgaaactgatcgacactttcaaattcaacgacagctacagcgaatacgcttctggtaaatggaagacttgcatgctgtggaaccgttctggtcagaaagatgaccatctgtctattgaacatgatacctacgtgaaacctactgaatacggcaaacagctggcatacgtaaacgaaatcatcgctaacacctttaagaaagaacacatcaagacggtgcgtctgttcatgtgtatcaacggcctgatcatcccacacaaagactacctggaattcaagaaaggcttcacccgtatccacatcccgctgattatcaacgaacacgcactgacctctgaagaagatgttgtttacaacatgcagaaaggtgaaatttggttcatcgaaggccgtaaaatccacagcgctgccaatttcagcaaagtgaaacgtatcaacctggtcatcgacttcgcgccggatattccgtttgaagaactgttcctgaattctgagaactatcaaccgaacctgatcccgaaaatctctcaacgtacccagctgaaagaagaagagctgggttatatcaaaggtctgtctaaaattatcaatgaaatgaactttgacgacatcctgtccattctgagcaaaattcacttctatcgcaacgtttcctccgaactggtttttggctggctggacgaaattgccacggcgtccaacaactataacattcagcgcaaagcgcaggaagtaaccgatctgctgattcgcaaaggcccgattaataactaa

SEQ ID NO: 218 - protein, 276 aa, Artificial Sequence
  amino acid sequence of E27K+I39K+K123I mutant
MESKIIGKVNFEEHLLDKELKLIDTFKFNDSYSEYASGKWKTCMLWNRSGQKDDHLSIEHDTYVKPTEYGKQLAYVNEIIANTFKKEHIKTVRLFMCINGLIIPHKDYLEFKKGFTRIHIPLIINEHALTSEEDVVYNMQKGEIWFIEGRKIHSAANFSKVKRINLVIDFAPDIPFEELFLNSENYQPNLIPKISQRTQLKEEELGYIKGLSKIINEMNFDDILSILSKIHFYRNVSSELVFGWLDEIATASNNYNIQRKAQEVTDLLIRKGPINN

SEQ ID NO: 219 - DNA, 831 bp, Artificial Sequence
  gene sequence of K106Q+K112E+I223V mutant
atggaatccaagatcatcggtaaagtcaacttcgaggagcatctgctggataaagagctgaaactgatcgacactttcgagttcaacgacagctacagcgaatacgcttctggtatttggaagacttgcatgctgtggaaccgttctggtcagaaagatgaccatctgtctattgaacatgatacctacgtgaaacctactgaatacggcaaacagctggcatacgtaaacgaaatcatcgctaacacctttaagaaagaacacatcaagacggtgcgtctgttcatgtgtatcaacggcctgatcatcccacaccaggactacctggaattcgaaaaaggcttcacccgtatccacatcccgctgaaaatcaacgaacacgcactgacctctgaagaagatgttgtttacaacatgcagaaaggtgaaatttggttcatcgaaggccgtaaaatccacagcgctgccaatttcagcaaagtgaaacgtatcaacctggtcatcgacttcgcgccggatattccgtttgaagaactgttcctgaattctgagaactatcaaccgaacctgatcccgaaaatctctcaacgtacccagctgaaagaagaagagctgggttatatcaaaggtctgtctaaaattatcaatgaaatgaactttgacgacgttctgtccattctgagcaaaattcacttctatcgcaacgtttcctccgaactggtttttggctggctggacgaaattgccacggcgtccaacaactataacattcagcgcaaagcgcaggaagtaaccgatctgctgattcgcaaaggcccgattaataactaa

SEQ ID NO: 220 - protein, 276 aa, Artificial Sequence
  amino acid sequence of K106Q+K112E+I223V mutant
MESKIIGKVNFEEHLLDKELKLIDTFEFNDSYSEYASGIWKTCMLWNRSGQKDDHLSIEHDTYVKPTEYGKQLAYVNEIIANTFKKEHIKTVRLFMCINGLIIPHQDYLEFEKGFTRIHIPLKINEHALTSEEDVVYNMQKGEIWFIEGRKIHSAANFSKVKRINLVIDFAPDIPFEELFLNSENYQPNLIPKISQRTQLKEEELGYIKGLSKIINEMNFDDVLSILSKIHFYRNVSSELVFGWLDEIATASNNYNIQRKAQEVTDLLIRKGPINN

SEQ ID NO: 221 - DNA, 831 bp, Artificial Sequence
  gene sequence of H14R+E34G+K106Q+K112E+I223V mutant
atggaatccaagatcatcggtaaagtcaacttcgaggagcgtctgctggataaagagctgaaactgatcgacactttcgagttcaacgacagctacagcggttacgcttctggtatttggaagacttgcatgctgtggaaccgttctggtcagaaagatgaccatctgtctattgaacatgatacctacgtgaaacctactgaatacggcaaacagctggcatacgtaaacgaaatcatcgctaacacctttaagaaagaacacatcaagacggtgcgtctgttcatgtgtatcaacggcctgatcatcccacaccaggactacctggaattcgaaaaaggcttcacccgtatccacatcccgctgaaaatcaacgaacacgcactgacctctgaagaagatgttgtttacaacatgcagaaaggtgaaatttggttcatcgaaggccgtaaaatccacagcgctgccaatttcagcaaagtgaaacgtatcaacctggtcatcgacttcgcgccggatattccgtttgaagaactgttcctgaattctgagaactatcaaccgaacctgatcccgaaaatctctcaacgtacccagctgaaagaagaagagctgggttatatcaaaggtctgtctaaaattatcaatgaaatgaactttgacgacgttctgtccattctgagcaaaattcacttctatcgcaacgtttcctccgaactggtttttggctggctggacgaaattgccacggcgtccaacaactataacattcagcgcaaagcgcaggaagtaaccgatctgctgattcgcaaaggcccgattaataactaa

SEQ ID NO: 222 - protein, 276 aa, Artificial Sequence
  amino acid sequence of H14R+E34G+K106Q+K112E+I223V mutant
MESKIIGKVNFEERLLDKELKLIDTFEFNDSYSGYASGIWKTCMLWNRSGQKDDHLSIEHDTYVKPTEYGKQLAYVNEIIANTFKKEHIKTVRLFMCINGLIIPHQDYLEFEKGFTRIHIPLKINEHALTSEEDVVYNMQKGEIWFIEGRKIHSAANFSKVKRINLVIDFAPDIPFEELFLNSENYQPNLIPKISQRTQLKEEELGYIKGLSKIINEMNFDDVLSILSKIHFYRNVSSELVFGWLDEIATASNNYNIQRKAQEVTDLLIRKGPINN

SEQ ID NO: 223 - DNA, 831 bp, Artificial Sequence
  gene sequence of E27K+I39K+E34L mutant
atggaatccaagatcatcggtaaagtcaacttcgaggagcatctgctggataaagagctgaaactgatcgacactttcaaattcaacgacagctacagcctgtacgcttctggtaaatggaagacttgcatgctgtggaaccgttctggtcagaaagatgaccatctgtctattgaacatgatacctacgtgaaacctactgaatacggcaaacagctggcatacgtaaacgaaatcatcgctaacacctttaagaaagaacacatcaagacggtgcgtctgttcatgtgtatcaacggcctgatcatcccacacaaagactacctggaattcaagaaaggcttcacccgtatccacatcccgctgaaaatcaacgaacacgcactgacctctgaagaagatgttgtttacaacatgcagaaaggtgaaatttggttcatcgaaggccgtaaaatccacagcgctgccaatttcagcaaagtgaaacgtatcaacctggtcatcgacttcgcgccggatattccgtttgaagaactgttcctgaattctgagaactatcaaccgaacctgatcccgaaaatctctcaacgtacccagctgaaagaagaagagctgggttatatcaaaggtctgtctaaaattatcaatgaaatgaactttgacgacatcctgtccattctgagcaaaattcacttctatcgcaacgtttcctccgaactggtttttggctggctggacgaaattgccacggcgtccaacaactataacattcagcgcaaagcgcaggaagtaaccgatctgctgattcgcaaaggcccgattaataactaa

SEQ ID NO: 224 - protein, 276 aa, Artificial Sequence
  amino acid sequence of E27K+I39K+E34L mutant
MESKIIGKVNFEEHLLDKELKLIDTFKFNDSYSLYASGKWKTCMLWNRSGQKDDHLSIEHDTYVKPTEYGKQLAYVNEIIANTFKKEHIKTVRLFMCINGLIIPHKDYLEFKKGFTRIHIPLKINEHALTSEEDVVYNMQKGEIWFIEGRKIHSAANFSKVKRINLVIDFAPDIPFEELFLNSENYQPNLIPKISQRTQLKEEELGYIKGLSKIINEMNFDDILSILSKIHFYRNVSSELVFGWLDEIATASNNYNIQRKAQEVTDLLIRKGPINN

SEQ ID NO: 225 - DNA, 831 bp, Artificial Sequence
  gene sequence of E27K+I39K+S37F+I58T mutant
atggaatccaagatcatcggtaaagtcaacttcgaggagcatctgctggataaagagctgaaactgatcgacactttcaaattcaacgacagctacagcgaatacgcttttggtaaatggaagacttgcatgctgtggaaccgttctggtcagaaagatgaccatctgtctaccgaacatgatacctacgtgaaacctactgaatacggcaaacagctggcatacgtaaacgaaatcatcgctaacacctttaagaaagaacacatcaagacggtgcgtctgttcatgtgtatcaacggcctgatcatcccacacaaagactacctggaattcaagaaaggcttcacccgtatccacatcccgctgaaaatcaacgaacacgcactgacctctgaagaagatgttgtttacaacatgcagaaaggtgaaatttggttcatcgaaggccgtaaaatccacagcgctgccaatttcagcaaagtgaaacgtatcaacctggtcatcgacttcgcgccggatattccgtttgaagaactgttcctgaattctgagaactatcaaccgaacctgatcccgaaaatctctcaacgtacccagctgaaagaagaagagctgggttatatcaaaggtctgtctaaaattatcaatgaaatgaactttgacgacatcctgtccattctgagcaaaattcacttctatcgcaacgtttcctccgaactggtttttggctggctggacgaaattgccacggcgtccaacaactataacattcagcgcaaagcgcaggaagtaaccgatctgctgattcgcaaaggcccgattaataactaa

SEQ ID NO: 226 - protein, 276 aa, Artificial Sequence
  amino acid sequence of E27K+I39K+S37F+I58T mutant
MESKIIGKVNFEEHLLDKELKLIDTFKFNDSYSEYAFGKWKTCMLWNRSGQKDDHLSTEHDTYVKPTEYGKQLAYVNEIIANTFKKEHIKTVRLFMCINGLIIPHKDYLEFKKGFTRIHIPLKINEHALTSEEDVVYNMQKGEIWFIEGRKIHSAANFSKVKRINLVIDFAPDIPFEELFLNSENYQPNLIPKISQRTQLKEEELGYIKGLSKIINEMNFDDILSILSKIHFYRNVSSELVFGWLDEIATASNNYNIQRKAQEVTDLLIRKGPINN

SEQ ID NO: 227 - DNA, 831 bp, Artificial Sequence
  gene sequence of E27K+I39K+S37F+I58Y mutant
atggaatccaagatcatcggtaaagtcaacttcgaggagcatctgctggataaagagctgaaactgatcgacactttcaaattcaacgacagctacagcgaatacgcttttggtaaatggaagacttgcatgctgtggaaccgttctggtcagaaagatgaccatctgtcttatgaacatgatacctacgtgaaacctactgaatacggcaaacagctggcatacgtaaacgaaatcatcgctaacacctttaagaaagaacacatcaagacggtgcgtctgttcatgtgtatcaacggcctgatcatcccacacaaagactacctggaattcaagaaaggcttcacccgtatccacatcccgctgaaaatcaacgaacacgcactgacctctgaagaagatgttgtttacaacatgcagaaaggtgaaatttggttcatcgaaggccgtaaaatccacagcgctgccaatttcagcaaagtgaaacgtatcaacctggtcatcgacttcgcgccggatattccgtttgaagaactgttcctgaattctgagaactatcaaccgaacctgatcccgaaaatctctcaacgtacccagctgaaagaagaagagctgggttatatcaaaggtctgtctaaaattatcaatgaaatgaactttgacgacatcctgtccattctgagcaaaattcacttctatcgcaacgtttcctccgaactggtttttggctggctggacgaaattgccacggcgtccaacaactataacattcagcgcaaagcgcaggaagtaaccgatctgctgattcgcaaaggcccgattaataactaa

SEQ ID NO: 228 - protein, 276 aa, Artificial Sequence
  amino acid sequence of E27K+I39K+S37F+I58Y mutant
MESKIIGKVNFEEHLLDKELKLIDTFKFNDSYSEYAFGKWKTCMLWNRSGQKDDHLSYEHDTYVKPTEYGKQLAYVNEIIANTFKKEHIKTVRLFMCINGLIIPHKDYLEFKKGFTRIHIPLKINEHALTSEEDVVYNMQKGEIWFIEGRKIHSAANFSKVKRINLVIDFAPDIPFEELFLNSENYQPNLIPKISQRTQLKEEELGYIKGLSKIINEMNFDDILSILSKIHFYRNVSSELVFGWLDEIATASNNYNIQRKAQEVTDLLIRKGPINN

SEQ ID NO: 229 - DNA, 831 bp, Artificial Sequence
  gene sequence of E27K+I39K+S37F+I58A mutant
atggaatccaagatcatcggtaaagtcaacttcgaggagcatctgctggataaagagctgaaactgatcgacactttcaaattcaacgacagctacagcgaatacgcttttggtaaatggaagacttgcatgctgtggaaccgttctggtcagaaagatgaccatctgtctgcagaacatgatacctacgtgaaacctactgaatacggcaaacagctggcatacgtaaacgaaatcatcgctaacacctttaagaaagaacacatcaagacggtgcgtctgttcatgtgtatcaacggcctgatcatcccacacaaagactacctggaattcaagaaaggcttcacccgtatccacatcccgctgaaaatcaacgaacacgcactgacctctgaagaagatgttgtttacaacatgcagaaaggtgaaatttggttcatcgaaggccgtaaaatccacagcgctgccaatttcagcaaagtgaaacgtatcaacctggtcatcgacttcgcgccggatattccgtttgaagaactgttcctgaattctgagaactatcaaccgaacctgatcccgaaaatctctcaacgtacccagctgaaagaagaagagctgggttatatcaaaggtctgtctaaaattatcaatgaaatgaactttgacgacatcctgtccattctgagcaaaattcacttctatcgcaacgtttcctccgaactggtttttggctggctggacgaaattgccacggcgtccaacaactataacattcagcgcaaagcgcaggaagtaaccgatctgctgattcgcaaaggcccgattaataactaa

SEQ ID NO: 230 - protein, 276 aa, Artificial Sequence
  amino acid sequence of E27K+I39K+S37F+I58A mutant
MESKIIGKVNFEEHLLDKELKLIDTFKFNDSYSEYAFGKWKTCMLWNRSGQKDDHLSAEHDTYVKPTEYGKQLAYVNEIIANTFKKEHIKTVRLFMCINGLIIPHKDYLEFKKGFTRIHIPLKINEHALTSEEDVVYNMQKGEIWFIEGRKIHSAANFSKVKRINLVIDFAPDIPFEELFLNSENYQPNLIPKISQRTQLKEEELGYIKGLSKIINEMNFDDILSILSKIHFYRNVSSELVFGWLDEIATASNNYNIQRKAQEVTDLLIRKGPINN

SEQ ID NO: 231 - DNA, 831 bp, Artificial Sequence
  gene sequence of E27K+I39K+S37F+I58R mutant
atggaatccaagatcatcggtaaagtcaacttcgaggagcatctgctggataaagagctgaaactgatcgacactttcaaattcaacgacagctacagcgaatacgcttttggtaaatggaagacttgcatgctgtggaaccgttctggtcagaaagatgaccatctgtctcgtgaacatgatacctacgtgaaacctactgaatacggcaaacagctggcatacgtaaacgaaatcatcgctaacacctttaagaaagaacacatcaagacggtgcgtctgttcatgtgtatcaacggcctgatcatcccacacaaagactacctggaattcaagaaaggcttcacccgtatccacatcccgctgaaaatcaacgaacacgcactgacctctgaagaagatgttgtttacaacatgcagaaaggtgaaatttggttcatcgaaggccgtaaaatccacagcgctgccaatttcagcaaagtgaaacgtatcaacctggtcatcgacttcgcgccggatattccgtttgaagaactgttcctgaattctgagaactatcaaccgaacctgatcccgaaaatctctcaacgtacccagctgaaagaagaagagctgggttatatcaaaggtctgtctaaaattatcaatgaaatgaactttgacgacatcctgtccattctgagcaaaattcacttctatcgcaacgtttcctccgaactggtttttggctggctggacgaaattgccacggcgtccaacaactataacattcagcgcaaagcgcaggaagtaaccgatctgctgattcgcaaaggcccgattaataactaa

SEQ ID NO: 232 - protein, 276 aa, Artificial Sequence
  amino acid sequence of E27K+I39K+S37F+I58R mutant
MESKIIGKVNFEEHLLDKELKLIDTFKFNDSYSEYAFGKWKTCMLWNRSGQKDDHLSREHDTYVKPTEYGKQLAYVNEIIANTFKKEHIKTVRLFMCINGLIIPHKDYLEFKKGFTRIHIPLKINEHALTSEEDVVYNMQKGEIWFIEGRKIHSAANFSKVKRINLVIDFAPDIPFEELFLNSENYQPNLIPKISQRTQLKEEELGYIKGLSKIINEMNFDDILSILSKIHFYRNVSSELVFGWLDEIATASNNYNIQRKAQEVTDLLIRKGPINN

SEQ ID NO: 233 - DNA, 831 bp, Artificial Sequence
  gene sequence of E27K+I39K+S37F+I58V mutant
atggaatccaagatcatcggtaaagtcaacttcgaggagcatctgctggataaagagctgaaactgatcgacactttcaaattcaacgacagctacagcgaatacgcttttggtaaatggaagacttgcatgctgtggaaccgttctggtcagaaagatgaccatctgtctgttgaacatgatacctacgtgaaacctactgaatacggcaaacagctggcatacgtaaacgaaatcatcgctaacacctttaagaaagaacacatcaagacggtgcgtctgttcatgtgtatcaacggcctgatcatcccacacaaagactacctggaattcaagaaaggcttcacccgtatccacatcccgctgaaaatcaacgaacacgcactgacctctgaagaagatgttgtttacaacatgcagaaaggtgaaatttggttcatcgaaggccgtaaaatccacagcgctgccaatttcagcaaagtgaaacgtatcaacctggtcatcgacttcgcgccggatattccgtttgaagaactgttcctgaattctgagaactatcaaccgaacctgatcccgaaaatctctcaacgtacccagctgaaagaagaagagctgggttatatcaaaggtctgtctaaaattatcaatgaaatgaactttgacgacatcctgtccattctgagcaaaattcacttctatcgcaacgtttcctccgaactggtttttggctggctggacgaaattgccacggcgtccaacaactataacattcagcgcaaagcgcaggaagtaaccgatctgctgattcgcaaaggcccgattaataactaa

SEQ ID NO: 234 - protein, 276 aa, Artificial Sequence
  amino acid sequence of E27K+I39K+S37F+I58V mutant
MESKIIGKVNFEEHLLDKELKLIDTFKFNDSYSEYAFGKWKTCMLWNRSGQKDDHLSVEHDTYVKPTEYGKQLAYVNEIIANTFKKEHIKTVRLFMCINGLIIPHKDYLEFKKGFTRIHIPLKINEHALTSEEDVVYNMQKGEIWFIEGRKIHSAANFSKVKRINLVIDFAPDIPFEELFLNSENYQPNLIPKISQRTQLKEEELGYIKGLSKIINEMNFDDILSILSKIHFYRNVSSELVFGWLDEIATASNNYNIQRKAQEVTDLLIRKGPINN

SEQ ID NO: 235 - DNA, 831 bp, Artificial Sequence
  gene sequence of E27K+I39K+S37F+I58S mutant
atggaatccaagatcatcggtaaagtcaacttcgaggagcatctgctggataaagagctgaaactgatcgacactttcaaattcaacgacagctacagcgaatacgcttttggtaaatggaagacttgcatgctgtggaaccgttctggtcagaaagatgaccatctgtctagtgaacatgatacctacgtgaaacctactgaatacggcaaacagctggcatacgtaaacgaaatcatcgctaacacctttaagaaagaacacatcaagacggtgcgtctgttcatgtgtatcaacggcctgatcatcccacacaaagactacctggaattcaagaaaggcttcacccgtatccacatcccgctgaaaatcaacgaacacgcactgacctctgaagaagatgttgtttacaacatgcagaaaggtgaaatttggttcatcgaaggccgtaaaatccacagcgctgccaatttcagcaaagtgaaacgtatcaacctggtcatcgacttcgcgccggatattccgtttgaagaactgttcctgaattctgagaactatcaaccgaacctgatcccgaaaatctctcaacgtacccagctgaaagaagaagagctgggttatatcaaaggtctgtctaaaattatcaatgaaatgaactttgacgacatcctgtccattctgagcaaaattcacttctatcgcaacgtttcctccgaactggtttttggctggctggacgaaattgccacggcgtccaacaactataacattcagcgcaaagcgcaggaagtaaccgatctgctgattcgcaaaggcccgattaataactaa

SEQ ID NO: 236 - protein, 276 aa, Artificial Sequence
  amino acid sequence of E27K+I39K+S37F+I58S mutant
MESKIIGKVNFEEHLLDKELKLIDTFKFNDSYSEYAFGKWKTCMLWNRSGQKDDHLSSEHDTYVKPTEYGKQLAYVNEIIANTFKKEHIKTVRLFMCINGLIIPHKDYLEFKKGFTRIHIPLKINEHALTSEEDVVYNMQKGEIWFIEGRKIHSAANFSKVKRINLVIDFAPDIPFEELFLNSENYQPNLIPKISQRTQLKEEELGYIKGLSKIINEMNFDDILSILSKIHFYRNVSSELVFGWLDEIATASNNYNIQRKAQEVTDLLIRKGPINN

SEQ ID NO: 237 - DNA, 831 bp, Artificial Sequence
  gene sequence of E27K+I39K+S37N+I58C mutant
atggaatccaagatcatcggtaaagtcaacttcgaggagcatctgctggataaagagctgaaactgatcgacactttcaaattcaacgacagctacagcgaatacgctaatggtaaatggaagacttgcatgctgtggaaccgttctggtcagaaagatgaccatctgtcttgtgaacatgatacctacgtgaaacctactgaatacggcaaacagctggcatacgtaaacgaaatcatcgctaacacctttaagaaagaacacatcaagacggtgcgtctgttcatgtgtatcaacggcctgatcatcccacacaaagactacctggaattcaagaaaggcttcacccgtatccacatcccgctgaaaatcaacgaacacgcactgacctctgaagaagatgttgtttacaacatgcagaaaggtgaaatttggttcatcgaaggccgtaaaatccacagcgctgccaatttcagcaaagtgaaacgtatcaacctggtcatcgacttcgcgccggatattccgtttgaagaactgttcctgaattctgagaactatcaaccgaacctgatcccgaaaatctctcaacgtacccagctgaaagaagaagagctgggttatatcaaaggtctgtctaaaattatcaatgaaatgaactttgacgacatcctgtccattctgagcaaaattcacttctatcgcaacgtttcctccgaactggtttttggctggctggacgaaattgccacggcgtccaacaactataacattcagcgcaaagcgcaggaagtaaccgatctgctgattcgcaaaggcccgattaataactaa

SEQ ID NO: 238 - protein, 276 aa, Artificial Sequence
  amino acid sequence of E27K+I39K+S37N+I58C mutant
MESKIIGKVNFEEHLLDKELKLIDTFKFNDSYSEYANGKWKTCMLWNRSGQKDDHLSCEHDTYVKPTEYGKQLAYVNEIIANTFKKEHIKTVRLFMCINGLIIPHKDYLEFKKGFTRIHIPLKINEHALTSEEDVVYNMQKGEIWFIEGRKIHSAANFSKVKRINLVIDFAPDIPFEELFLNSENYQPNLIPKISQRTQLKEEELGYIKGLSKIINEMNFDDILSILSKIHFYRNVSSELVFGWLDEIATASNNYNIQRKAQEVTDLLIRKGPINN

SEQ ID NO: 239 - DNA, 831 bp, Artificial Sequence
  gene sequence of E27K+D30S+I39K+I58R+K112E mutant
atggaatccaagatcatcggtaaagtcaacttcgaggagcatctgctggataaagagctgaaactgatcgacactttcaaattcaacagcagctacagcgaatacgcttctggtaaatggaagacttgcatgctgtggaaccgttctggtcagaaagatgaccatctgtctcgtgaacatgatacctacgtgaaacctactgaatacggcaaacagctggcatacgtaaacgaaatcatcgctaacacctttaagaaagaacacatcaagacggtgcgtctgttcatgtgtatcaacggcctgatcatcccacacaaagactacctggaattcgagaaaggcttcacccgtatccacatcccgctgaaaatcaacgaacacgcactgacctctgaagaagatgttgtttacaacatgcagaaaggtgaaatttggttcatcgaaggccgtaaaatccacagcgctgccaatttcagcaaagtgaaacgtatcaacctggtcatcgacttcgcgccggatattccgtttgaagaactgttcctgaattctgagaactatcaaccgaacctgatcccgaaaatctctcaacgtacccagctgaaagaagaagagctgggttatatcaaaggtctgtctaaaattatcaatgaaatgaactttgacgacatcctgtccattctgagcaaaattcacttctatcgcaacgtttcctccgaactggtttttggctggctggacgaaattgccacggcgtccaacaactataacattcagcgcaaagcgcaggaagtaaccgatctgctgattcgcaaaggcccgattaataactaa

SEQ ID NO: 240 - protein, 276 aa, Artificial Sequence
  amino acid sequence of E27K+D30S+I39K+I58R+K112E mutant
MESKIIGKVNFEEHLLDKELKLIDTFKFNSSYSEYASGKWKTCMLWNRSGQKDDHLSREHDTYVKPTEYGKQLAYVNEIIANTFKKEHIKTVRLFMCINGLIIPHKDYLEFEKGFTRIHIPLKINEHALTSEEDVVYNMQKGEIWFIEGRKIHSAANFSKVKRINLVIDFAPDIPFEELFLNSENYQPNLIPKISQRTQLKEEELGYIKGLSKIINEMNFDDILSILSKIHFYRNVSSELVFGWLDEIATASNNYNIQRKAQEVTDLLIRKGPINN

SEQ ID NO: 241 - DNA, 831 bp, Artificial Sequence
  gene sequence of E27K+E34N+I39K+I58Y+I223V mutant
atggaatccaagatcatcggtaaagtcaacttcgaggagcatctgctggataaagagctgaaactgatcgacactttcaaattcaacgacagctacagcaattacgcttctggtaaatggaagacttgcatgctgtggaaccgttctggtcagaaagatgaccatctgtcttatgaacatgatacctacgtgaaacctactgaatacggcaaacagctggcatacgtaaacgaaatcatcgctaacacctttaagaaagaacacatcaagacggtgcgtctgttcatgtgtatcaacggcctgatcatcccacacaaagactacctggaattcaagaaaggcttcacccgtatccacatcccgctgaaaatcaacgaacacgcactgacctctgaagaagatgttgtttacaacatgcagaaaggtgaaatttggttcatcgaaggccgtaaaatccacagcgctgccaatttcagcaaagtgaaacgtatcaacctggtcatcgacttcgcgccggatattccgtttgaagaactgttcctgaattctgagaactatcaaccgaacctgatcccgaaaatctctcaacgtacccagctgaaagaagaagagctgggttatatcaaaggtctgtctaaaattatcaatgaaatgaactttgacgacgttctgtccattctgagcaaaattcacttctatcgcaacgtttcctccgaactggtttttggctggctggacgaaattgccacggcgtccaacaactataacattcagcgcaaagcgcaggaagtaaccgatctgctgattcgcaaaggcccgattaataactaa

SEQ ID NO: 242 - protein, 276 aa, Artificial Sequence
  amino acid sequence of E27K+E34N+I39K+I58Y+I223V mutant
MESKIIGKVNFEEHLLDKELKLIDTFKFNDSYSNYASGKWKTCMLWNRSGQKDDHLSYEHDTYVKPTEYGKQLAYVNEIIANTFKKEHIKTVRLFMCINGLIIPHKDYLEFKKGFTRIHIPLKINEHALTSEEDVVYNMQKGEIWFIEGRKIHSAANFSKVKRINLVIDFAPDIPFEELFLNSENYQPNLIPKISQRTQLKEEELGYIKGLSKIINEMNFDDVLSILSKIHFYRNVSSELVFGWLDEIATASNNYNIQRKAQEVTDLLIRKGPINN

SEQ ID NO: 243 - DNA, 831 bp, Artificial Sequence
  gene sequence of E27K+S37N+I39K+I58Y+D173G mutant
atggaatccaagatcatcggtaaagtcaacttcgaggagcatctgctggataaagagctgaaactgatcgacactttcaaattcaacgacagctacagcaattacgcttctggtaaatggaagacttgcatgctgtggaaccgttctggtcagaaagatgaccatctgtcttatgaacatgatacctacgtgaaacctactgaatacggcaaacagctggcatacgtaaacgaaatcatcgctaacacctttaagaaagaacacatcaagacggtgcgtctgttcatgtgtatcaacggcctgatcatcccacacaaagactacctggaattcaagaaaggcttcacccgtatccacatcccgctgaaaatcaacgaacacgcactgacctctgaagaagatgttgtttacaacatgcagaaaggtgaaatttggttcatcgaaggccgtaaaatccacagcgctgccaatttcagcaaagtgaaacgtatcaacctggtcatcgacttcgcgccgtatattccgtttgaagaactgttcctgaattctgagaactatcaaccgaacctgatcccgaaaatctctcaacgtacccagctgaaagaagaagagctgggttatatcaaaggtctgtctaaaattatcaatgaaatgaactttgacgacatcctgtccattctgagcaaaattcacttctatcgcaacgtttcctccgaactggtttttggctggctggacgaaattgccacggcgtccaacaactataacattcagcgcaaagcgcaggaagtaaccgatctgctgattcgcaaaggcccgattaataactaa

SEQ ID NO: 244 - protein, 276 aa, Artificial Sequence
  amino acid sequence of E27K+S37N+I39K+I58Y+D173G mutant
MESKIIGKVNFEEHLLDKELKLIDTFKFNDSYSNYASGKWKTCMLWNRSGQKDDHLSYEHDTYVKPTEYGKQLAYVNEIIANTFKKEHIKTVRLFMCINGLIIPHKDYLEFKKGFTRIHIPLKINEHALTSEEDVVYNMQKGEIWFIEGRKIHSAANFSKVKRINLVIDFAPYIPFEELFLNSENYQPNLIPKISQRTQLKEEELGYIKGLSKIINEMNFDDILSILSKIHFYRNVSSELVFGWLDEIATASNNYNIQRKAQEVTDLLIRKGPINN

SEQ ID NO: 245 - DNA, 831 bp, Artificial Sequence
  gene sequence of E27K+S37F+I39K+I58Y+D173G mutant
atggaatccaagatcatcggtaaagtcaacttcgaggagcatctgctggataaagagctgaaactgatcgacactttcaaattcaacgacagctacagcttttacgcttctggtaaatggaagacttgcatgctgtggaaccgttctggtcagaaagatgaccatctgtcttatgaacatgatacctacgtgaaacctactgaatacggcaaacagctggcatacgtaaacgaaatcatcgctaacacctttaagaaagaacacatcaagacggtgcgtctgttcatgtgtatcaacggcctgatcatcccacacaaagactacctggaattcaagaaaggcttcacccgtatccacatcccgctgaaaatcaacgaacacgcactgacctctgaagaagatgttgtttacaacatgcagaaaggtgaaatttggttcatcgaaggccgtaaaatccacagcgctgccaatttcagcaaagtgaaacgtatcaacctggtcatcgacttcgcgccgtatattccgtttgaagaactgttcctgaattctgagaactatcaaccgaacctgatcccgaaaatctctcaacgtacccagctgaaagaagaagagctgggttatatcaaaggtctgtctaaaattatcaatgaaatgaactttgacgacatcctgtccattctgagcaaaattcacttctatcgcaacgtttcctccgaactggtttttggctggctggacgaaattgccacggcgtccaacaactataacattcagcgcaaagcgcaggaagtaaccgatctgctgattcgcaaaggcccgattaataactaa

SEQ ID NO: 246 - protein, 276 aa, Artificial Sequence
  amino acid sequence of E27K+S37F+I39K+I58Y+D173G mutant
MESKIIGKVNFEEHLLDKELKLIDTFKFNDSYSFYASGKWKTCMLWNRSGQKDDHLSYEHDTYVKPTEYGKQLAYVNEIIANTFKKEHIKTVRLFMCINGLIIPHKDYLEFKKGFTRIHIPLKINEHALTSEEDVVYNMQKGEIWFIEGRKIHSAANFSKVKRINLVIDFAPYIPFEELFLNSENYQPNLIPKISQRTQLKEEELGYIKGLSKIINEMNFDDILSILSKIHFYRNVSSELVFGWLDEIATASNNYNIQRKAQEVTDLLIRKGPINN

SEQ ID NO: 247 - DNA, 831 bp, Artificial Sequence
  gene sequence of E27K+I39K+S37N+I58A mutant
atggaatccaagatcatcggtaaagtcaacttcgaggagcatctgctggataaagagctgaaactgatcgacactttcaaattcaacgacagctacagcgaatacgctaatggtaaatggaagacttgcatgctgtggaaccgttctggtcagaaagatgaccatctgtctgcagaacatgatacctacgtgaaacctactgaatacggcaaacagctggcatacgtaaacgaaatcatcgctaacacctttaagaaagaacacatcaagacggtgcgtctgttcatgtgtatcaacggcctgatcatcccacacaaagactacctggaattcaagaaaggcttcacccgtatccacatcccgctgaaaatcaacgaacacgcactgacctctgaagaagatgttgtttacaacatgcagaaaggtgaaatttggttcatcgaaggccgtaaaatccacagcgctgccaatttcagcaaagtgaaacgtatcaacctggtcatcgacttcgcgccggatattccgtttgaagaactgttcctgaattctgagaactatcaaccgaacctgatcccgaaaatctctcaacgtacccagctgaaagaagaagagctgggttatatcaaaggtctgtctaaaattatcaatgaaatgaactttgacgacatcctgtccattctgagcaaaattcacttctatcgcaacgtttcctccgaactggtttttggctggctggacgaaattgccacggcgtccaacaactataacattcagcgcaaagcgcaggaagtaaccgatctgctgattcgcaaaggcccgattaataactaa

SEQ ID NO: 248 - protein, 276 aa, Artificial Sequence
  amino acid sequence of E27K+I39K+S37N+I58A mutant
MESKIIGKVNFEEHLLDKELKLIDTFKFNDSYSEYANGKWKTCMLWNRSGQKDDHLSAEHDTYVKPTEYGKQLAYVNEIIANTFKKEHIKTVRLFMCINGLIIPHKDYLEFKKGFTRIHIPLKINEHALTSEEDVVYNMQKGEIWFIEGRKIHSAANFSKVKRINLVIDFAPDIPFEELFLNSENYQPNLIPKISQRTQLKEEELGYIKGLSKIINEMNFDDILSILSKIHFYRNVSSELVFGWLDEIATASNNYNIQRKAQEVTDLLIRKGPINN

SEQ ID NO: 249 - DNA, 831 bp, Artificial Sequence
  gene sequence of E27K+I39K+S37N+I58R+K123Q mutant
atggaatccaagatcatcggtaaagtcaacttcgaggagcatctgctggataaagagctgaaactgatcgacactttcaaattcaacgacagctacagcgaatacgctaatggtaaatggaagacttgcatgctgtggaaccgttctggtcagaaagatgaccatctgtctcgtgaacatgatacctacgtgaaacctactgaatacggcaaacagctggcatacgtaaacgaaatcatcgctaacacctttaagaaagaacacatcaagacggtgcgtctgttcatgtgtatcaacggcctgatcatcccacacaaagactacctggaattcaagaaaggcttcacccgtatccacatcccgctgcagatcaacgaacacgcactgacctctgaagaagatgttgtttacaacatgcagaaaggtgaaatttggttcatcgaaggccgtaaaatccacagcgctgccaatttcagcaaagtgaaacgtatcaacctggtcatcgacttcgcgccggatattccgtttgaagaactgttcctgaattctgagaactatcaaccgaacctgatcccgaaaatctctcaacgtacccagctgaaagaagaagagctgggttatatcaaaggtctgtctaaaattatcaatgaaatgaactttgacgacatcctgtccattctgagcaaaattcacttctatcgcaacgtttcctccgaactggtttttggctggctggacgaaattgccacggcgtccaacaactataacattcagcgcaaagcgcaggaagtaaccgatctgctgattcgcaaaggcccgattaataactaa

SEQ ID NO: 250 - protein, 276 aa, Artificial Sequence
  amino acid sequence of E27K+I39K+S37N+I58R+K123Q mutant
MESKIIGKVNFEEHLLDKELKLIDTFKFNDSYSEYANGKWKTCMLWNRSGQKDDHLSREHDTYVKPTEYGKQLAYVNEIIANTFKKEHIKTVRLFMCINGLIIPHKDYLEFKKGFTRIHIPLQINEHALTSEEDVVYNMQKGEIWFIEGRKIHSAANFSKVKRINLVIDFAPDIPFEELFLNSENYQPNLIPKISQRTQLKEEELGYIKGLSKIINEMNFDDILSILSKIHFYRNVSSELVFGWLDEIATASNNYNIQRKAQEVTDLLIRKGPINN

SEQ ID NO: 251 - DNA, 831 bp, Artificial Sequence
  sequence of E27K+S37F+I39K+I58Y+D173G+I118R mutant
atggaatccaagatcatcggtaaagtcaacttcgaggagcatctgctggataaagagctgaaactgatcgacactttcaaattcaacgacagctacagcttttacgcttctggtaaatggaagacttgcatgctgtggaaccgttctggtcagaaagatgaccatctgtcttatgaacatgatacctacgtgaaacctactgaatacggcaaacagctggcatacgtaaacgaaatcatcgctaacacctttaagaaagaacacatcaagacggtgcgtctgttcatgtgtatcaacggcctgatcatcccacacaaagactacctggaattcaagaaaggcttcacccgtcgtcacatcccgctgaaaatcaacgaacacgcactgacctctgaagaagatgttgtttacaacatgcagaaaggtgaaatttggttcatcgaaggccgtaaaatccacagcgctgccaatttcagcaaagtgaaacgtatcaacctggtcatcgacttcgcgccgtatattccgtttgaagaactgttcctgaattctgagaactatcaaccgaacctgatcccgaaaatctctcaacgtacccagctgaaagaagaagagctgggttatatcaaaggtctgtctaaaattatcaatgaaatgaactttgacgacatcctgtccattctgagcaaaattcacttctatcgcaacgtttcctccgaactggtttttggctggctggacgaaattgccacggcgtccaacaactataacattcagcgcaaagcgcaggaagtaaccgatctgctgattcgcaaaggcccgattaataactaa

SEQ ID NO: 252 - protein, 276 aa, Artificial Sequence
  amino acid sequence of E27K+S37F+I39K+I58Y+D173G+I118R mutant
MESKIIGKVNFEEHLLDKELKLIDTFKFNDSYSFYASGKWKTCMLWNRSGQKDDHLSYEHDTYVKPTEYGKQLAYVNEIIANTFKKEHIKTVRLFMCINGLIIPHKDYLEFKKGFTRRHIPLKINEHALTSEEDVVYNMQKGEIWFIEGRKIHSAANFSKVKRINLVIDFAPYIPFEELFLNSENYQPNLIPKISQRTQLKEEELGYIKGLSKIINEMNFDDILSILSKIHFYRNVSSELVFGWLDEIATASNNYNIQRKAQEVTDLLIRKGPINN

SEQ ID NO: 253 - DNA, 831 bp, Artificial Sequence
  gene sequence of E27K+E34L+S37N+I39K+I58R mutant
atggaatccaagatcatcggtaaagtcaacttcgaggagcatctgctggataaagagctgaaactgatcgacactttcaaattcaacgacagctacagcctgtacgctaatggtaaatggaagacttgcatgctgtggaaccgttctggtcagaaagatgaccatctgtctcgtgaacatgatacctacgtgaaacctactgaatacggcaaacagctggcatacgtaaacgaaatcatcgctaacacctttaagaaagaacacatcaagacggtgcgtctgttcatgtgtatcaacggcctgatcatcccacacaaagactacctggaattcaagaaaggcttcacccgtatccacatcccgctgaaaatcaacgaacacgcactgacctctgaagaagatgttgtttacaacatgcagaaaggtgaaatttggttcatcgaaggccgtaaaatccacagcgctgccaatttcagcaaagtgaaacgtatcaacctggtcatcgacttcgcgccggatattccgtttgaagaactgttcctgaattctgagaactatcaaccgaacctgatcccgaaaatctctcaacgtacccagctgaaagaagaagagctgggttatatcaaaggtctgtctaaaattatcaatgaaatgaactttgacgacatcctgtccattctgagcaaaattcacttctatcgcaacgtttcctccgaactggtttttggctggctggacgaaattgccacggcgtccaacaactataacattcagcgcaaagcgcaggaagtaaccgatctgctgattcgcaaaggcccgattaataactaa

SEQ ID NO: 254 - protein, 276 aa, Artificial Sequence
  amino acid sequence of E27K+E34L+S37N+I39K+I58R mutant
MESKIIGKVNFEEHLLDKELKLIDTFKFNDSYSLYANGKWKTCMLWNRSGQKDDHLSREHDTYVKPTEYGKQLAYVNEIIANTFKKEHIKTVRLFMCINGLIIPHKDYLEFKKGFTRIHIPLKINEHALTSEEDVVYNMQKGEIWFIEGRKIHSAANFSKVKRINLVIDFAPDIPFEELFLNSENYQPNLIPKISQRTQLKEEELGYIKGLSKIINEMNFDDILSILSKIHFYRNVSSELVFGWLDEIATASNNYNIQRKAQEVTDLLIRKGPINN

SEQ ID NO: 255 - DNA, 831 bp, Artificial Sequence
  gene sequence of E27K+E34L+S37N+I39K+I58Y+D173G mutant
atggaatccaagatcatcggtaaagtcaacttcgaggagcatctgctggataaagagctgaaactgatcgacactttcaaattcaacgacagctacagcctgtacgctaatggtaaatggaagacttgcatgctgtggaaccgttctggtcagaaagatgaccatctgtcttatgaacatgatacctacgtgaaacctactgaatacggcaaacagctggcatacgtaaacgaaatcatcgctaacacctttaagaaagaacacatcaagacggtgcgtctgttcatgtgtatcaacggcctgatcatcccacacaaagactacctggaattcaagaaaggcttcacccgtcgtcacatcccgctgaaaatcaacgaacacgcactgacctctgaagaagatgttgtttacaacatgcagaaaggtgaaatttggttcatcgaaggccgtaaaatccacagcgctgccaatttcagcaaagtgaaacgtatcaacctggtcatcgacttcgcgccggatattccgtttgaagaactgttcctgaattctgagaactatcaaccgaacctgatcccgaaaatctctcaacgtacccagctgaaagaagaagagctgggttatatcaaaggtctgtctaaaattatcaatgaaatgaactttgacgacatcctgtccattctgagcaaaattcacttctatcgcaacgtttcctccgaactggtttttggctggctggacgaaattgccacggcgtccaacaactataacattcagcgcaaagcgcaggaagtaaccgatctgctgattcgcaaaggcccgattaataactaa

SEQ ID NO: 256 - protein, 276 aa, Artificial Sequence
  amino acid sequence of E27K+E34L+S37N+I39K+I58Y+D173G mutant
MESKIIGKVNFEEHLLDKELKLIDTFKFNDSYSLYANGKWKTCMLWNRSGQKDDHLSYEHDTYVKPTEYGKQLAYVNEIIANTFKKEHIKTVRLFMCINGLIIPHKDYLEFKKGFTRRHIPLKINEHALTSEEDVVYNMQKGEIWFIEGRKIHSAANFSKVKRINLVIDFAPDIPFEELFLNSENYQPNLIPKISQRTQLKEEELGYIKGLSKIINEMNFDDILSILSKIHFYRNVSSELVFGWLDEIATASNNYNIQRKAQEVTDLLIRKGPINN

SEQ ID NO: 257 - DNA, 831 bp, Artificial Sequence
  gene sequence of E27K+E34L+S37N+I39K+I58Y+D173G+K123Q mutant
atggaatccaagatcatcggtaaagtcaacttcgaggagcatctgctggataaagagctgaaactgatcgacactttcaaattcaacgacagctacagcctgtacgctaatggtaaatggaagacttgcatgctgtggaaccgttctggtcagaaagatgaccatctgtcttatgaacatgatacctacgtgaaacctactgaatacggcaaacagctggcatacgtaaacgaaatcatcgctaacacctttaagaaagaacacatcaagacggtgcgtctgttcatgtgtatcaacggcctgatcatcccacacaaagactacctggaattcaagaaaggcttcacccgtcgtcacatcccgctgcagatcaacgaacacgcactgacctctgaagaagatgttgtttacaacatgcagaaaggtgaaatttggttcatcgaaggccgtaaaatccacagcgctgccaatttcagcaaagtgaaacgtatcaacctggtcatcgacttcgcgccggatattccgtttgaagaactgttcctgaattctgagaactatcaaccgaacctgatcccgaaaatctctcaacgtacccagctgaaagaagaagagctgggttatatcaaaggtctgtctaaaattatcaatgaaatgaactttgacgacatcctgtccattctgagcaaaattcacttctatcgcaacgtttcctccgaactggtttttggctggctggacgaaattgccacggcgtccaacaactataacattcagcgcaaagcgcaggaagtaaccgatctgctgattcgcaaaggcccgattaataactaa

SEQ ID NO: 258 - protein, 276 aa, Artificial Sequence
  sequence of E27K+E34L+S37N+I39K+I58Y+D173G+K123Q mutant
MESKIIGKVNFEEHLLDKELKLIDTFKFNDSYSLYANGKWKTCMLWNRSGQKDDHLSYEHDTYVKPTEYGKQLAYVNEIIANTFKKEHIKTVRLFMCINGLIIPHKDYLEFKKGFTRRHIPLQINEHALTSEEDVVYNMQKGEIWFIEGRKIHSAANFSKVKRINLVIDFAPDIPFEELFLNSENYQPNLIPKISQRTQLKEEELGYIKGLSKIINEMNFDDILSILSKIHFYRNVSSELVFGWLDEIATASNNYNIQRKAQEVTDLLIRKGPINN

SEQ ID NO: 259 - DNA, 831 bp, Artificial Sequence
  H14R+E27K+D30S+E34G+I39K+I98V+K106Q+K112E+I223V mutant
atggaatccaagatcatcggtaaagtcaacttcgaggagcgtctgctggataaagagctgaaactgatcgacactttcaaattcaacagcagctacagcggttacgcttctggtaaatggaagacttgcatgctgtggaaccgttctggtcagaaagatgaccatctgtctattgaacatgatacctacgtgaaacctactgaatacggcaaacagctggcatacgtaaacgaaatcatcgctaacacctttaagaaagaacacatcaagacggtgcgtctgttcatgtgtgttaacggcctgatcatcccacaccaggactacctggaattcgaaaaaggcttcacccgtatccacatcccgctgaaaatcaacgaacacgcactgacctctgaagaagatgttgtttacaacatgcagaaaggtgaaatttggttcatcgaaggccgtaaaatccacagcgctgccaatttcagcaaagtgaaacgtatcaacctggtcatcgacttcgcgccggatattccgtttgaagaactgttcctgaattctgagaactatcaaccgaacctgatcccgaaaatctctcaacgtacccagctgaaagaagaagagctgggttatatcaaaggtctgtctaaaattatcaatgaaatgaactttgacgacgttctgtccattctgagcaaaattcacttctatcgcaacgtttcctccgaactggtttttggctggctggacgaaattgccacggcgtccaacaactataacattcagcgcaaagcgcaggaagtaaccgatctgctgattcgcaaaggcccgattaataactaa

SEQ ID NO: 260 - protein, 276 aa, Artificial Sequence
  H14R+E27K+D30S+E34G+I39K+I98V+K106Q+K112E+I223V mutant
MESKIIGKVNFEERLLDKELKLIDTFKFNSSYSGYASGKWKTCMLWNRSGQKDDHLSIEHDTYVKPTEYGKQLAYVNEIIANTFKKEHIKTVRLFMCVNGLIIPHQDYLEFEKGFTRIHIPLKINEHALTSEEDVVYNMQKGEIWFIEGRKIHSAANFSKVKRINLVIDFAPDIPFEELFLNSENYQPNLIPKISQRTQLKEEELGYIKGLSKIINEMNFDDVLSILSKIHFYRNVSSELVFGWLDEIATASNNYNIQRKAQEVTDLLIRKGPINN

SEQ ID NO: 261 - DNA, 831 bp, Artificial Sequence
  H14R+E27K+E34N+I39K+I98V+K106Q+K112E+I223V mutant
atggaatccaagatcatcggtaaagtcaacttcgaggagcgtctgctggataaagagctgaaactgatcgacactttcaaattcaacgacagctacagcaattacgcttctggtaaatggaagacttgcatgctgtggaaccgttctggtcagaaagatgaccatctgtctattgaacatgatacctacgtgaaacctactgaatacggcaaacagctggcatacgtaaacgaaatcatcgctaacacctttaagaaagaacacatcaagacggtgcgtctgttcatgtgtgttaacggcctgatcatcccacaccaggactacctggaattcgaaaaaggcttcacccgtatccacatcccgctgaaaatcaacgaacacgcactgacctctgaagaagatgttgtttacaacatgcagaaaggtgaaatttggttcatcgaaggccgtaaaatccacagcgctgccaatttcagcaaagtgaaacgtatcaacctggtcatcgacttcgcgccggatattccgtttgaagaactgttcctgaattctgagaactatcaaccgaacctgatcccgaaaatctctcaacgtacccagctgaaagaagaagagctgggttatatcaaaggtctgtctaaaattatcaatgaaatgaactttgacgacgttctgtccattctgagcaaaattcacttctatcgcaacgtttcctccgaactggtttttggctggctggacgaaattgccacggcgtccaacaactataacattcagcgcaaagcgcaggaagtaaccgatctgctgattcgcaaaggcccgattaataactaa

SEQ ID NO: 262 - protein, 276 aa, Artificial Sequence
  H14R+E27K+E34N+I39K+I98V+K106Q+K112E+I223V mutant
MESKIIGKVNFEERLLDKELKLIDTFKFNDSYSNYASGKWKTCMLWNRSGQKDDHLSIEHDTYVKPTEYGKQLAYVNEIIANTFKKEHIKTVRLFMCVNGLIIPHQDYLEFEKGFTRIHIPLKINEHALTSEEDVVYNMQKGEIWFIEGRKIHSAANFSKVKRINLVIDFAPDIPFEELFLNSENYQPNLIPKISQRTQLKEEELGYIKGLSKIINEMNFDDVLSILSKIHFYRNVSSELVFGWLDEIATASNNYNIQRKAQEVTDLLIRKGPINN

SEQ ID NO: 263 - DNA, 831 bp, Artificial Sequence
  H14R+E27K+E34G+I39K+I98V+K106Q+K112E+I223V mutant
atggaatccaagatcatcggtaaagtcaacttcgaggagcgtctgctggataaagagctgaaactgatcgacactttcaaattcaacgacagctacagcggttacgcttctggtaaatggaagacttgcatgctgtggaaccgttctggtcagaaagatgaccatctgtctattgaacatgatacctacgtgaaacctactgaatacggcaaacagctggcatacgtaaacgaaatcatcgctaacacctttaagaaagaacacatcaagacggtgcgtctgttcatgtgtgttaacggcctgatcatcccacaccaggactacctggaattcgaaaaaggcttcacccgtatccacatcccgctgaaaatcaacgaacacgcactgacctctgaagaagatgttgtttacaacatgcagaaaggtgaaatttggttcatcgaaggccgtaaaatccacagcgctgccaatttcagcaaagtgaaacgtatcaacctggtcatcgacttcgcgccggatattccgtttgaagaactgttcctgaattctgagaactatcaaccgaacctgatcccgaaaatctctcaacgtacccagctgaaagaagaagagctgggttatatcaaaggtctgtctaaaattatcaatgaaatgaactttgacgacgttctgtccattctgagcaaaattcacttctatcgcaacgtttcctccgaactggtttttggctggctggacgaaattgccacggcgtccaacaactataacattcagcgcaaagcgcaggaagtaaccgatctgctgattcgcaaaggcccgattaataactaa

SEQ ID NO: 264 - protein, 276 aa, Artificial Sequence
  H14R+E27K+E34G+I39K+I98V+K106Q+K112E+I223V mutant
MESKIIGKVNFEERLLDKELKLIDTFKFNDSYSGYASGKWKTCMLWNRSGQKDDHLSIEHDTYVKPTEYGKQLAYVNEIIANTFKKEHIKTVRLFMCVNGLIIPHQDYLEFEKGFTRIHIPLKINEHALTSEEDVVYNMQKGEIWFIEGRKIHSAANFSKVKRINLVIDFAPDIPFEELFLNSENYQPNLIPKISQRTQLKEEELGYIKGLSKIINEMNFDDVLSILSKIHFYRNVSSELVFGWLDEIATASNNYNIQRKAQEVTDLLIRKGPINN

SEQ ID NO: 265 - DNA, 831 bp, Artificial Sequence
  H14R+E27K+E34G+S37W+I39K+I98V+K106Q+K112E+I223V mutant
atggaatccaagatcatcggtaaagtcaacttcgaggagcgtctgctggataaagagctgaaactgatcgacactttcaaattcaacgacagctacagcggttacgcttggggtaaatggaagacttgcatgctgtggaaccgttctggtcagaaagatgaccatctgtctattgaacatgatacctacgtgaaacctactgaatacggcaaacagctggcatacgtaaacgaaatcatcgctaacacctttaagaaagaacacatcaagacggtgcgtctgttcatgtgtgttaacggcctgatcatcccacaccaggactacctggaattcgaaaaaggcttcacccgtatccacatcccgctgaaaatcaacgaacacgcactgacctctgaagaagatgttgtttacaacatgcagaaaggtgaaatttggttcatcgaaggccgtaaaatccacagcgctgccaatttcagcaaagtgaaacgtatcaacctggtcatcgacttcgcgccggatattccgtttgaagaactgttcctgaattctgagaactatcaaccgaacctgatcccgaaaatctctcaacgtacccagctgaaagaagaagagctgggttatatcaaaggtctgtctaaaattatcaatgaaatgaactttgacgacgttctgtccattctgagcaaaattcacttctatcgcaacgtttcctccgaactggtttttggctggctggacgaaattgccacggcgtccaacaactataacattcagcgcaaagcgcaggaagtaaccgatctgctgattcgcaaaggcccgattaataactaa

SEQ ID NO: 266 - protein, 276 aa, Artificial Sequence
  H14R+E27K+E34G+S37W+I39K+I98V+K106Q+K112E+I223V mutant
MESKIIGKVNFEERLLDKELKLIDTFKFNDSYSGYAWGKWKTCMLWNRSGQKDDHLSIEHDTYVKPTEYGKQLAYVNEIIANTFKKEHIKTVRLFMCVNGLIIPHQDYLEFEKGFTRIHIPLKINEHALTSEEDVVYNMQKGEIWFIEGRKIHSAANFSKVKRINLVIDFAPDIPFEELFLNSENYQPNLIPKISQRTQLKEEELGYIKGLSKIINEMNFDDVLSILSKIHFYRNVSSELVFGWLDEIATASNNYNIQRKAQEVTDLLIRKGPINN

SEQ ID NO: 267 - DNA, 831 bp, Artificial Sequence
  H14R+E27K+E34G+S37F+I39K+I98V+K106Q+K112E+I223V mutant
atggaatccaagatcatcggtaaagtcaacttcgaggagcgtctgctggataaagagctgaaactgatcgacactttcaaattcaacgacagctacagcggttacgcttttggtaaatggaagacttgcatgctgtggaaccgttctggtcagaaagatgaccatctgtctattgaacatgatacctacgtgaaacctactgaatacggcaaacagctggcatacgtaaacgaaatcatcgctaacacctttaagaaagaacacatcaagacggtgcgtctgttcatgtgtgttaacggcctgatcatcccacaccaggactacctggaattcgaaaaaggcttcacccgtatccacatcccgctgaaaatcaacgaacacgcactgacctctgaagaagatgttgtttacaacatgcagaaaggtgaaatttggttcatcgaaggccgtaaaatccacagcgctgccaatttcagcaaagtgaaacgtatcaacctggtcatcgacttcgcgccggatattccgtttgaagaactgttcctgaattctgagaactatcaaccgaacctgatcccgaaaatctctcaacgtacccagctgaaagaagaagagctgggttatatcaaaggtctgtctaaaattatcaatgaaatgaactttgacgacgttctgtccattctgagcaaaattcacttctatcgcaacgtttcctccgaactggtttttggctggctggacgaaattgccacggcgtccaacaactataacattcagcgcaaagcgcaggaagtaaccgatctgctgattcgcaaaggcccgattaataactaa

SEQ ID NO: 268 - protein, 276 aa, Artificial Sequence
  H14R+E27K+E34G+S37F+I39K+I98V+K106Q+K112E+I223V mutant
MESKIIGKVNFEERLLDKELKLIDTFKFNDSYSGYAFGKWKTCMLWNRSGQKDDHLSIEHDTYVKPTEYGKQLAYVNEIIANTFKKEHIKTVRLFMCVNGLIIPHQDYLEFEKGFTRIHIPLKINEHALTSEEDVVYNMQKGEIWFIEGRKIHSAANFSKVKRINLVIDFAPDIPFEELFLNSENYQPNLIPKISQRTQLKEEELGYIKGLSKIINEMNFDDVLSILSKIHFYRNVSSELVFGWLDEIATASNNYNIQRKAQEVTDLLIRKGPINN

SEQ ID NO: 269 - DNA, 831 bp, Artificial Sequence
  H14R+E27K+E34G+S37E+I39K+I98V+K106Q+K112E+I223V mutant
atggaatccaagatcatcggtaaagtcaacttcgaggagcgtctgctggataaagagctgaaactgatcgacactttcaaattcaacgacagctacagcggttacgctgaaggtaaatggaagacttgcatgctgtggaaccgttctggtcagaaagatgaccatctgtctattgaacatgatacctacgtgaaacctactgaatacggcaaacagctggcatacgtaaacgaaatcatcgctaacacctttaagaaagaacacatcaagacggtgcgtctgttcatgtgtgttaacggcctgatcatcccacaccaggactacctggaattcgaaaaaggcttcacccgtatccacatcccgctgaaaatcaacgaacacgcactgacctctgaagaagatgttgtttacaacatgcagaaaggtgaaatttggttcatcgaaggccgtaaaatccacagcgctgccaatttcagcaaagtgaaacgtatcaacctggtcatcgacttcgcgccggatattccgtttgaagaactgttcctgaattctgagaactatcaaccgaacctgatcccgaaaatctctcaacgtacccagctgaaagaagaagagctgggttatatcaaaggtctgtctaaaattatcaatgaaatgaactttgacgacgttctgtccattctgagcaaaattcacttctatcgcaacgtttcctccgaactggtttttggctggctggacgaaattgccacggcgtccaacaactataacattcagcgcaaagcgcaggaagtaaccgatctgctgattcgcaaaggcccgattaataactaa

SEQ ID NO: 270 - protein, 276 aa, Artificial Sequence
  H14R+E27K+E34G+S37E+I39K+I98V+K106Q+K112E+I223V mutant
MESKIIGKVNFEERLLDKELKLIDTFKFNDSYSGYAEGKWKTCMLWNRSGQKDDHLSIEHDTYVKPTEYGKQLAYVNEIIANTFKKEHIKTVRLFMCVNGLIIPHQDYLEFEKGFTRIHIPLKINEHALTSEEDVVYNMQKGEIWFIEGRKIHSAANFSKVKRINLVIDFAPDIPFEELFLNSENYQPNLIPKISQRTQLKEEELGYIKGLSKIINEMNFDDVLSILSKIHFYRNVSSELVFGWLDEIATASNNYNIQRKAQEVTDLLIRKGPINN

SEQ ID NO: 271 - DNA, 831 bp, Artificial Sequence
  H14R+E27K+E34G+Y35K+I39K+I98V+K106Q+K112E+I223V mutant
atggaatccaagatcatcggtaaagtcaacttcgaggagcgtctgctggataaagagctgaaactgatcgacactttcaaattcaacgacagctacagcggtaaagcttctggtaaatggaagacttgcatgctgtggaaccgttctggtcagaaagatgaccatctgtctattgaacatgatacctacgtgaaacctactgaatacggcaaacagctggcatacgtaaacgaaatcatcgctaacacctttaagaaagaacacatcaagacggtgcgtctgttcatgtgtgttaacggcctgatcatcccacaccaggactacctggaattcgaaaaaggcttcacccgtatccacatcccgctgaaaatcaacgaacacgcactgacctctgaagaagatgttgtttacaacatgcagaaaggtgaaatttggttcatcgaaggccgtaaaatccacagcgctgccaatttcagcaaagtgaaacgtatcaacctggtcatcgacttcgcgccggatattccgtttgaagaactgttcctgaattctgagaactatcaaccgaacctgatcccgaaaatctctcaacgtacccagctgaaagaagaagagctgggttatatcaaaggtctgtctaaaattatcaatgaaatgaactttgacgacgttctgtccattctgagcaaaattcacttctatcgcaacgtttcctccgaactggtttttggctggctggacgaaattgccacggcgtccaacaactataacattcagcgcaaagcgcaggaagtaaccgatctgctgattcgcaaaggcccgattaataactaa

SEQ ID NO: 272 - protein, 276 aa, Artificial Sequence
  H14R+E27K+E34G+Y35K+I39K+I98V+K106Q+K112E+I223V mutant
MESKIIGKVNFEERLLDKELKLIDTFKFNDSYSGKASGKWKTCMLWNRSGQKDDHLSIEHDTYVKPTEYGKQLAYVNEIIANTFKKEHIKTVRLFMCVNGLIIPHQDYLEFEKGFTRIHIPLKINEHALTSEEDVVYNMQKGEIWFIEGRKIHSAANFSKVKRINLVIDFAPDIPFEELFLNSENYQPNLIPKISQRTQLKEEELGYIKGLSKIINEMNFDDVLSILSKIHFYRNVSSELVFGWLDEIATASNNYNIQRKAQEVTDLLIRKGPINN

SEQ ID NO: 273 - DNA, 831 bp, Artificial Sequence
  H14R+E27K+E34G+S37N+I39K+I98V+K106Q+K112E+I223V mutant
atggaatccaagatcatcggtaaagtcaacttcgaggagcgtctgctggataaagagctgaaactgatcgacactttcaaattcaacgacagctacagcggttacgctaatggtaaatggaagacttgcatgctgtggaaccgttctggtcagaaagatgaccatctgtctattgaacatgatacctacgtgaaacctactgaatacggcaaacagctggcatacgtaaacgaaatcatcgctaacacctttaagaaagaacacatcaagacggtgcgtctgttcatgtgtgttaacggcctgatcatcccacaccaggactacctggaattcgaaaaaggcttcacccgtatccacatcccgctgaaaatcaacgaacacgcactgacctctgaagaagatgttgtttacaacatgcagaaaggtgaaatttggttcatcgaaggccgtaaaatccacagcgctgccaatttcagcaaagtgaaacgtatcaacctggtcatcgacttcgcgccggatattccgtttgaagaactgttcctgaattctgagaactatcaaccgaacctgatcccgaaaatctctcaacgtacccagctgaaagaagaagagctgggttatatcaaaggtctgtctaaaattatcaatgaaatgaactttgacgacgttctgtccattctgagcaaaattcacttctatcgcaacgtttcctccgaactggtttttggctggctggacgaaattgccacggcgtccaacaactataacattcagcgcaaagcgcaggaagtaaccgatctgctgattcgcaaaggcccgattaataactaa

SEQ ID NO: 274 - protein, 276 aa, Artificial Sequence
  H14R+E27K+E34G+S37N+I39K+I98V+K106Q+K112E+I223V mutant
MESKIIGKVNFEERLLDKELKLIDTFKFNDSYSGYANGKWKTCMLWNRSGQKDDHLSIEHDTYVKPTEYGKQLAYVNEIIANTFKKEHIKTVRLFMCVNGLIIPHQDYLEFEKGFTRIHIPLKINEHALTSEEDVVYNMQKGEIWFIEGRKIHSAANFSKVKRINLVIDFAPDIPFEELFLNSENYQPNLIPKISQRTQLKEEELGYIKGLSKIINEMNFDDVLSILSKIHFYRNVSSELVFGWLDEIATASNNYNIQRKAQEVTDLLIRKGPINN

SEQ ID NO: 275 - DNA, 831 bp, Artificial Sequence
  H14R+E27K+E34G+I39K+I98V+K106Q+K112E+K123Q+I223V mutant
atggaatccaagatcatcggtaaagtcaacttcgaggagcgtctgctggataaagagctgaaactgatcgacactttcaaattcaacgacagctacagcggttacgcttctggtaaatggaagacttgcatgctgtggaaccgttctggtcagaaagatgaccatctgtctattgaacatgatacctacgtgaaacctactgaatacggcaaacagctggcatacgtaaacgaaatcatcgctaacacctttaagaaagaacacatcaagacggtgcgtctgttcatgtgtgttaacggcctgatcatcccacaccaggactacctggaattcgaaaaaggcttcacccgtatccacatcccgctgcaaatcaacgaacacgcactgacctctgaagaagatgttgtttacaacatgcagaaaggtgaaatttggttcatcgaaggccgtaaaatccacagcgctgccaatttcagcaaagtgaaacgtatcaacctggtcatcgacttcgcgccggatattccgtttgaagaactgttcctgaattctgagaactatcaaccgaacctgatcccgaaaatctctcaacgtacccagctgaaagaagaagagctgggttatatcaaaggtctgtctaaaattatcaatgaaatgaactttgacgacgttctgtccattctgagcaaaattcacttctatcgcaacgtttcctccgaactggtttttggctggctggacgaaattgccacggcgtccaacaactataacattcagcgcaaagcgcaggaagtaaccgatctgctgattcgcaaaggcccgattaataactaa

SEQ ID NO: 276 - protein, 276 aa, Artificial Sequence
  H14R+E27K+E34G+I39K+I98V+K106Q+K112E+K123Q+I223V mutant
MESKIIGKVNFEERLLDKELKLIDTFKFNDSYSGYASGKWKTCMLWNRSGQKDDHLSIEHDTYVKPTEYGKQLAYVNEIIANTFKKEHIKTVRLFMCVNGLIIPHQDYLEFEKGFTRIHIPLQINEHALTSEEDVVYNMQKGEIWFIEGRKIHSAANFSKVKRINLVIDFAPDIPFEELFLNSENYQPNLIPKISQRTQLKEEELGYIKGLSKIINEMNFDDVLSILSKIHFYRNVSSELVFGWLDEIATASNNYNIQRKAQEVTDLLIRKGPINN

SEQ ID NO: 277 - DNA, 831 bp, Artificial Sequence
  H14R+E27K+E34G+I39K+I98V+K106Q+K112E+K123S+I223V mutant
atggaatccaagatcatcggtaaagtcaacttcgaggagcgtctgctggataaagagctgaaactgatcgacactttcaaattcaacgacagctacagcggttacgcttctggtaaatggaagacttgcatgctgtggaaccgttctggtcagaaagatgaccatctgtctattgaacatgatacctacgtgaaacctactgaatacggcaaacagctggcatacgtaaacgaaatcatcgctaacacctttaagaaagaacacatcaagacggtgcgtctgttcatgtgtgttaacggcctgatcatcccacaccaggactacctggaattcgaaaaaggcttcacccgtatccacatcccgctgagcatcaacgaacacgcactgacctctgaagaagatgttgtttacaacatgcagaaaggtgaaatttggttcatcgaaggccgtaaaatccacagcgctgccaatttcagcaaagtgaaacgtatcaacctggtcatcgacttcgcgccggatattccgtttgaagaactgttcctgaattctgagaactatcaaccgaacctgatcccgaaaatctctcaacgtacccagctgaaagaagaagagctgggttatatcaaaggtctgtctaaaattatcaatgaaatgaactttgacgacgttctgtccattctgagcaaaattcacttctatcgcaacgtttcctccgaactggtttttggctggctggacgaaattgccacggcgtccaacaactataacattcagcgcaaagcgcaggaagtaaccgatctgctgattcgcaaaggcccgattaataactaa

SEQ ID NO: 278 - protein, 276 aa, Artificial Sequence
  H14R+E27K+E34G+I39K+I98V+K106Q+K112E+K123S+I223V mutant
MESKIIGKVNFEERLLDKELKLIDTFKFNDSYSGYASGKWKTCMLWNRSGQKDDHLSIEHDTYVKPTEYGKQLAYVNEIIANTFKKEHIKTVRLFMCVNGLIIPHQDYLEFEKGFTRIHIPLSINEHALTSEEDVVYNMQKGEIWFIEGRKIHSAANFSKVKRINLVIDFAPDIPFEELFLNSENYQPNLIPKISQRTQLKEEELGYIKGLSKIINEMNFDDVLSILSKIHFYRNVSSELVFGWLDEIATASNNYNIQRKAQEVTDLLIRKGPINN

SEQ ID NO: 279 - DNA, 831 bp, Artificial Sequence
  H14R+E27K+E34G+I39K+I58A+I98V+K106Q+K112E+I223V mutant
atggaatccaagatcatcggtaaagtcaacttcgaggagcgtctgctggataaagagctgaaactgatcgacactttcaaattcaacgacagctacagcggttacgcttctggtaaatggaagacttgcatgctgtggaaccgttctggtcagaaagatgaccatctgtctgcagaacatgatacctacgtgaaacctactgaatacggcaaacagctggcatacgtaaacgaaatcatcgctaacacctttaagaaagaacacatcaagacggtgcgtctgttcatgtgtgttaacggcctgatcatcccacaccaggactacctggaattcgaaaaaggcttcacccgtatccacatcccgctgaaaatcaacgaacacgcactgacctctgaagaagatgttgtttacaacatgcagaaaggtgaaatttggttcatcgaaggccgtaaaatccacagcgctgccaatttcagcaaagtgaaacgtatcaacctggtcatcgacttcgcgccggatattccgtttgaagaactgttcctgaattctgagaactatcaaccgaacctgatcccgaaaatctctcaacgtacccagctgaaagaagaagagctgggttatatcaaaggtctgtctaaaattatcaatgaaatgaactttgacgacgttctgtccattctgagcaaaattcacttctatcgcaacgtttcctccgaactggtttttggctggctggacgaaattgccacggcgtccaacaactataacattcagcgcaaagcgcaggaagtaaccgatctgctgattcgcaaaggcccgattaataactaa

SEQ ID NO: 280 - protein, 276 aa, Artificial Sequence
  H14R+E27K+E34G+I39K+I58A+I98V+K106Q+K112E+I223V mutant
MESKIIGKVNFEERLLDKELKLIDTFKFNDSYSGYASGKWKTCMLWNRSGQKDDHLSAEHDTYVKPTEYGKQLAYVNEIIANTFKKEHIKTVRLFMCVNGLIIPHQDYLEFEKGFTRIHIPLKINEHALTSEEDVVYNMQKGEIWFIEGRKIHSAANFSKVKRINLVIDFAPDIPFEELFLNSENYQPNLIPKISQRTQLKEEELGYIKGLSKIINEMNFDDVLSILSKIHFYRNVSSELVFGWLDEIATASNNYNIQRKAQEVTDLLIRKGPINN

SEQ ID NO: 281 - DNA, 831 bp, Artificial Sequence
  H14R+E27K+E34G+I39K+I98V+K106Q+K112E+I118F+I223V mutant
atggaatccaagatcatcggtaaagtcaacttcgaggagcgtctgctggataaagagctgaaactgatcgacactttcaaattcaacgacagctacagcggttacgcttctggtaaatggaagacttgcatgctgtggaaccgttctggtcagaaagatgaccatctgtctattgaacatgatacctacgtgaaacctactgaatacggcaaacagctggcatacgtaaacgaaatcatcgctaacacctttaagaaagaacacatcaagacggtgcgtctgttcatgtgtgttaacggcctgatcatcccacaccaggactacctggaattcgaaaaaggcttcacccgtttccacatcccgctgaaaatcaacgaacacgcactgacctctgaagaagatgttgtttacaacatgcagaaaggtgaaatttggttcatcgaaggccgtaaaatccacagcgctgccaatttcagcaaagtgaaacgtatcaacctggtcatcgacttcgcgccggatattccgtttgaagaactgttcctgaattctgagaactatcaaccgaacctgatcccgaaaatctctcaacgtacccagctgaaagaagaagagctgggttatatcaaaggtctgtctaaaattatcaatgaaatgaactttgacgacgttctgtccattctgagcaaaattcacttctatcgcaacgtttcctccgaactggtttttggctggctggacgaaattgccacggcgtccaacaactataacattcagcgcaaagcgcaggaagtaaccgatctgctgattcgcaaaggcccgattaataactaa

SEQ ID NO: 282 - protein, 276 aa, Artificial Sequence
  H14R+E27K+E34G+I39K+I98V+K106Q+K112E+I118F+I223V mutant
MESKIIGKVNFEERLLDKELKLIDTFKFNDSYSGYASGKWKTCMLWNRSGQKDDHLSIEHDTYVKPTEYGKQLAYVNEIIANTFKKEHIKTVRLFMCVNGLIIPHQDYLEFEKGFTRFHIPLKINEHALTSEEDVVYNMQKGEIWFIEGRKIHSAANFSKVKRINLVIDFAPDIPFEELFLNSENYQPNLIPKISQRTQLKEEELGYIKGLSKIINEMNFDDVLSILSKIHFYRNVSSELVFGWLDEIATASNNYNIQRKAQEVTDLLIRKGPINN

SEQ ID NO: 283 - DNA, 831 bp, Artificial Sequence
  H14R+E27K+E34G+S37T+I39K+I98V+K106Q+K112E+I223V mutant
atggaatccaagatcatcggtaaagtcaacttcgaggagcgtctgctggataaagagctgaaactgatcgacactttcaaattcaacgacagctacagcggttacgctaccggtaaatggaagacttgcatgctgtggaaccgttctggtcagaaagatgaccatctgtctattgaacatgatacctacgtgaaacctactgaatacggcaaacagctggcatacgtaaacgaaatcatcgctaacacctttaagaaagaacacatcaagacggtgcgtctgttcatgtgtgttaacggcctgatcatcccacaccaggactacctggaattcgaaaaaggcttcacccgtatccacatcccgctgaaaatcaacgaacacgcactgacctctgaagaagatgttgtttacaacatgcagaaaggtgaaatttggttcatcgaaggccgtaaaatccacagcgctgccaatttcagcaaagtgaaacgtatcaacctggtcatcgacttcgcgccggatattccgtttgaagaactgttcctgaattctgagaactatcaaccgaacctgatcccgaaaatctctcaacgtacccagctgaaagaagaagagctgggttatatcaaaggtctgtctaaaattatcaatgaaatgaactttgacgacgttctgtccattctgagcaaaattcacttctatcgcaacgtttcctccgaactggtttttggctggctggacgaaattgccacggcgtccaacaactataacattcagcgcaaagcgcaggaagtaaccgatctgctgattcgcaaaggcccgattaataactaa

SEQ ID NO: 284 - protein, 276 aa, Artificial Sequence
  H14R+E27K+E34G+S37T+I39K+I98V+K106Q+K112E+I223V mutant
MESKIIGKVNFEERLLDKELKLIDTFKFNDSYSGYATGKWKTCMLWNRSGQKDDHLSIEHDTYVKPTEYGKQLAYVNEIIANTFKKEHIKTVRLFMCVNGLIIPHQDYLEFEKGFTRIHIPLKINEHALTSEEDVVYNMQKGEIWFIEGRKIHSAANFSKVKRINLVIDFAPDIPFEELFLNSENYQPNLIPKISQRTQLKEEELGYIKGLSKIINEMNFDDVLSILSKIHFYRNVSSELVFGWLDEIATASNNYNIQRKAQEVTDLLIRKGPINN

SEQ ID NO: 285 - DNA, 831 bp, Artificial Sequence
  H14R+E27K+E34G+I39K+I58V+I98V+K106Q+K112E+I223V mutant
atggaatccaagatcatcggtaaagtcaacttcgaggagcgtctgctggataaagagctgaaactgatcgacactttcaaattcaacgacagctacagcggttacgcttctggtaaatggaagacttgcatgctgtggaaccgttctggtcagaaagatgaccatctgtctgttgaacatgatacctacgtgaaacctactgaatacggcaaacagctggcatacgtaaacgaaatcatcgctaacacctttaagaaagaacacatcaagacggtgcgtctgttcatgtgtgttaacggcctgatcatcccacaccaggactacctggaattcgaaaaaggcttcacccgtatccacatcccgctgaaaatcaacgaacacgcactgacctctgaagaagatgttgtttacaacatgcagaaaggtgaaatttggttcatcgaaggccgtaaaatccacagcgctgccaatttcagcaaagtgaaacgtatcaacctggtcatcgacttcgcgccggatattccgtttgaagaactgttcctgaattctgagaactatcaaccgaacctgatcccgaaaatctctcaacgtacccagctgaaagaagaagagctgggttatatcaaaggtctgtctaaaattatcaatgaaatgaactttgacgacgttctgtccattctgagcaaaattcacttctatcgcaacgtttcctccgaactggtttttggctggctggacgaaattgccacggcgtccaacaactataacattcagcgcaaagcgcaggaagtaaccgatctgctgattcgcaaaggcccgattaataactaa

SEQ ID NO: 286 - protein, 276 aa, Artificial Sequence
  H14R+E27K+E34G+I39K+I58V+I98V+K106Q+K112E+I223V mutant
MESKIIGKVNFEERLLDKELKLIDTFKFNDSYSGYASGKWKTCMLWNRSGQKDDHLSVEHDTYVKPTEYGKQLAYVNEIIANTFKKEHIKTVRLFMCVNGLIIPHQDYLEFEKGFTRIHIPLKINEHALTSEEDVVYNMQKGEIWFIEGRKIHSAANFSKVKRINLVIDFAPDIPFEELFLNSENYQPNLIPKISQRTQLKEEELGYIKGLSKIINEMNFDDVLSILSKIHFYRNVSSELVFGWLDEIATASNNYNIQRKAQEVTDLLIRKGPINN

SEQ ID NO: 287 - DNA, 831 bp, Artificial Sequence
  H14R+E27K+E34G+I39K+I98V+K106Q+K112E+K123I+I223V mutant
atggaatccaagatcatcggtaaagtcaacttcgaggagcgtctgctggataaagagctgaaactgatcgacactttcaaattcaacgacagctacagcggttacgcttctggtaaatggaagacttgcatgctgtggaaccgttctggtcagaaagatgaccatctgtctattgaacatgatacctacgtgaaacctactgaatacggcaaacagctggcatacgtaaacgaaatcatcgctaacacctttaagaaagaacacatcaagacggtgcgtctgttcatgtgtgttaacggcctgatcatcccacaccaggactacctggaattcgaaaaaggcttcacccgtatccacatcccgctgattatcaacgaacacgcactgacctctgaagaagatgttgtttacaacatgcagaaaggtgaaatttggttcatcgaaggccgtaaaatccacagcgctgccaatttcagcaaagtgaaacgtatcaacctggtcatcgacttcgcgccggatattccgtttgaagaactgttcctgaattctgagaactatcaaccgaacctgatcccgaaaatctctcaacgtacccagctgaaagaagaagagctgggttatatcaaaggtctgtctaaaattatcaatgaaatgaactttgacgacgttctgtccattctgagcaaaattcacttctatcgcaacgtttcctccgaactggtttttggctggctggacgaaattgccacggcgtccaacaactataacattcagcgcaaagcgcaggaagtaaccgatctgctgattcgcaaaggcccgattaataactaa

SEQ ID NO: 288 - protein, 276 aa, Artificial Sequence
  H14R+E27K+E34G+I39K+I98V+K106Q+K112E+K123I+I223V mutant
MESKIIGKVNFEERLLDKELKLIDTFKFNDSYSGYASGKWKTCMLWNRSGQKDDHLSIEHDTYVKPTEYGKQLAYVNEIIANTFKKEHIKTVRLFMCVNGLIIPHQDYLEFEKGFTRIHIPLIINEHALTSEEDVVYNMQKGEIWFIEGRKIHSAANFSKVKRINLVIDFAPDIPFEELFLNSENYQPNLIPKISQRTQLKEEELGYIKGLSKIINEMNFDDVLSILSKIHFYRNVSSELVFGWLDEIATASNNYNIQRKAQEVTDLLIRKGPINN

SEQ ID NO: 289 - protein, 280 aa, Artificial Sequence
  amino acid sequence of PH1
MESKIIGKVNFEEHLLDKELKLIDTFEFNDSYSEYASGIWKTCMLWNRSGQKDDHLSIEHDTYVKPTEYGKQLAYVNEIIANTFKKEHIKTVRLFMCINGLIIPHKDYLEFKKGFTRIHIPLKINEHALTSEEDVVYNMQKGEIWFIEGRKIHSAANFSKVKRINLVIDFAPDIPFEELFLNSENYQPNLIPKISQRKELTDEVIEGILGFSIIISEANYREIVSILAKLHFFYKADCRSMYDWLKEICKRRGDPALIEKTASLERFFLGHRERGEVMTY

SEQ ID NO: 290 - protein, 276 aa, Artificial Sequence
  amino acid sequence of I39K+S33N
MESKIIGKVNFEEHLLDKELKLIDTFEFNDSYNEYASGKWKTCMLWNRSGQKDDHLSIEHDTYVKPTEYGKQLAYVNEIIANTFKKEHIKTVRLFMCINGLIIPHKDYLEFKKGFTRIHIPLKINEHALTSEEDVVYNMQKGEIWFIEGRKIHSAANFSKVKRINLVIDFAPDIPFEELFLNSENYQPNLIPKISQRTQLKEEELGYIKGLSKIINEMNFDDILSILSKIHFYRNVSSELVFGWLDEIATASNNYNIQRKAQEVTDLLIRKGPINN

SEQ ID NO: 291 - protein, 276 aa, Artificial Sequence
  amino acid sequence of E27K+I39K+F28L+S31A
MESKIIGKVNFEEHLLDKELKLIDTFKLNDAYSEYASGRWKTCMLWNRSGQKDDHLSIEHDTYVKPTEYGKQLAYVNEIIANTFKKEHIKTVRLFMCINGLIIPHKDYLEFKKGFTRIHIPLKINEHALTSEEDVVYNMQKGEIWFIEGRKIHSAANFSKVKRINLVIDFAPDIPFEELFLNSENYQPNLIPKISQRTQLKEEELGYIKGLSKIINEMNFDDILSILSKIHFYRNVSSELVFGWLDEIATASNNYNIQRKAQEVTDLLIRKGPINN

SEQ ID NO: 292 - protein, 280 aa, Artificial Sequence
  amino acid sequence of PH1 mutant with E27K mutation
MESKIIGKVNFEEHLLDKELKLIDTFKFNDSYSEYASGIWKTCMLWNRSGQKDDHLSIEHDTYVKPTEYGKQLAYVNEIIANTFKKEHIKTVRLFMCINGLIIPHKDYLEFKKGFTRIHIPLKINEHALTSEEDVVYNMQKGEIWFIEGRKIHSAANFSKVKRINLVIDFAPDIPFEELFLNSENYQPNLIPKISQRKELTDEVIEGILGFSIIISEANYREIVSILAKLHFFYKADCRSMYDWLKEICKRRGDPALIEKTASLERFFLGHRERGEVMTY